European Patent Specification EP 3 536 797 B1, published January 4, 2023. Title: PRODUCTS AND METHODS FOR ENHANCED TRANSGENE EXPRESSION AND PROCESSING. Applicant: SELEXIS S.A. The sequence listing filed with the application follows.

SEQUENCE LISTING (116 sequences)

SEQ ID NO: 1 - DNA, 3616 bp, Homo sapiens
  MISC_BINDING (1)..(320): MAR 1_68 OF CHROMOSOME 1
gactctagattataccaacctcataaaataagagcatatataaaagcaaatgctcttatcttgcagatccctgaactgaggaggcaagatcagtttggcagttgaagcagctggaatctgcaattcagagaatctaagaaaagacaaccctgaagagagagacccagaaacctagcaggagtttctccaaacattcaaggctgagggataaatgttacatgcacagggtgagcctccagaggcttgtccattagcaactgctacagtttcattatctcagggatcacagattgtgctacctattgcctaccatctgaaaacagttgcttcctatatttcatccagtttaatatttatttaaaccaagaaggttaatctggcaccagctattccgttgtgagtggatgtgaaagtaccaattccattctgttttactattaactatcctttgccttaatatgtatcagtaggtggcttgttgctaggaaatattaaatgaatggcatgtttcataggttgtgtttaaagttgttttttgagttaaatctttctttaataatactttctgatgtcaaaaacacttagaagtcatggtgttgaacatctatatagggttggatctaaaatagcttcttaacctttcctaaccactgtttttgtttgtttgtttttaactaagcatccagtttgggaaattctgaattaggggaatcataaaaggtttcattttagctgggccacataaggaaagtaagatatcaaattgtaaaaatcgttaagaacttctatcccatctgaagtgtgggttaggtgcctcttctctgtgctcccttaacatcctattttatctgtatatatatatattcttccaaatatccatgcatgggaaaaaaaatctgatcataaaaatattttaggctgggagtggtggctcacgcctgtaatcccagcactttgggaggctgaggtgggcggatcatgaggtcaagagatcgagaccatcctgaccaatatggtgaaaccccatctctactaaagatacaaaactattagctggacgtggtggcacgtgcctgtagtcccagctactcgggaggctgaggcaggagaacggcttgaacccaggaggtggaggttgcagtgagctgagatcgcgccactgcactccagcctgggcgacagagcgagactctgtctcaaaaaaaaaatatatatatatatatatatacacatatatatataaaatatatatatatacacacatatatatataaaatatatatatatacacacatatatataaaatatatatatatacacacatatatataaaatatatatatacacacatatatataaaatatatatatacacacatatatataaaatatatatatacacacatatatataaaatatatatatacacacatatatataaaatatatatatacacacatatatataaaatatatatatacacacatatatataaaatatatatatacacacatatatataaaatatatatatacacacatatatataaaatatatatatacacacatatatataaaatatatatatacacacatatataaaatatatatatacacacatatataaaatatatatatacacatatatataaaatatatatatacacatatatataaaatatatatacacacatatatataaaatatatatatacacacatatatataaaatatatatatacacatatatataaaatatatatatacacatatatataaaatatatatatatacacatatatataaaatatatatacacacatatatataaagtatatatatacacacatatatataaaatatatatatacacatatatataaaatatatatatacacatatatataaaatatatatatacacatatatataaaaatatatatatatattttttaaaatattccaattgtctcactttgtggatgagaaaaagaagtagttagaggtcaagtaacttggcctacatcttttctcaagattgtaaactcctagtgagcaataaccacatcttcattttctttgtataaaacaagaaagtttagcatgaaaaaggtactcaattacaaatgtgttggattgaattgaagacccttggaaggggattttgtacctgaggatctctttcttttggccatattgttcaatggacaaaatttagccttcgaaggcaggccgatttgaggttaatactacctttaccacttgatagctatgtgaccttggccatgtggtttcaacagtctgaacctcattttctctgtgtatgtgtggtcctccttacaagtttgtgaaaaatgtgaagtccttagccatgatagcccaatataacaggctaaatgataataggtttatgttcttttcctttatattctcagataagcactgtccaagtttgaggtgttttgaggtctcgcctgatttggattgtttgagtttatgctattctttgaattctttgagctgttctgaagcagtgtatcatgaacaaaaacatccccagttcagtccaaacccctggttacatatcattcttatgccatgttataaccagtttgagagtgttccctctgttattgcatttaagtttcagcctcacacagaaattcagcagccaatttctaagccctaagcataaaatctggggtgggggggggggatggcctgaagagcagcattatgaatagcaccattataattaatgatctctcaggaagatttacaatcacaggtagcagataaaacaaatagtactgcttctgcacttcccctccttttattcgctatgaaattttatgggaaatcagtccagtgaaaaatgtaagctcttaatctttcccagaaatcctacctcatttgatgaatactttgagggaatgaattagagcatttttttcttttatagtctacttcgcatttacgaagtgaggacggtagcttaggctgcctggccaactgatgagaaggtcagaggcatttttagagacctctgttgtctttcattcatgttcattttccacaaggcaagtaatttccaacaaatcagtgtcttcattagtaataagattattaacaacaataatagtcatagtaactattcagtgagagtccattatatatcaggcattctacaaggtactttatatacatctgagtaaacctcacacaattctacagggaggtatttctatccccatttaacaaataaggaaacgaagtccaagtaaattaacttgcccaaggtcacacagatagtacctggcagaacaggaatttaaacctaaatttgtccaactccaaaagcagccttctatttgttataaatgctgcctctcattatcacatattttattattaacaacaacaaacataccaattagcttaagatacaatacaaccagataatcatgatgacaacagtaattgttatactattataataaaatagatgttttgtatgttactataatcttgaatttgaatagaaatttgcatttctgaaagcatgttcctgtcatctaatatgattctgtatctattaaaatagtactacatctagag

SEQ ID NO: 2 - DNA, 4624 bp, Homo sapiens
  MISC_BINDING (1)..(4624): MAR 1_6 OF CHROMOSOME 1
ggatcttaaatctattttatttatttatttttcatgtggccaataccctccacccccttcttctgtctctttcaacttattgtggttaccttgaggctacctgagacagtaggcttgggtggggaagtatgcattctaagtgtaaagtttgatgagctttgacaaatgtcaacccatgtaccagaacattttcatcacccataaaatctcccttgtgtcacttgccagtcagtgtctattctagtatccaactcctggctccaagaaaccattgaactgttttctgtcactataaattagatttgtcttttctagagtttcatgtaaatggaatcatacactaagtactctttgtgcctggcttctgctcagcataatgtttttgagaatcattcatgctgctgcatgttttcagtagttcatttttttaaataggtgaattgtaactcattctgtgaatataccatattctgtcttccatttatctgttagtggatctttaggtcgtttctagttttgggctattgcaaataaagctgctgtaaatattaatgcacaagttttccatgttcatatgtttcatttcacttaggaaaatacctaagagaggaattgcacatattaaaaaaattttaaaaactactaagctgttctccaaaatggttgtacaatttttattcccaagagcaatatgagtgtttaattgctccacattctcaccaacacttggtgcttgttagttttattttcattgttttcattgttatgtctgtgaggcagcattgatgtgcatgtctctgagtgtcatcttagcggtgatgctgagcatcagttcacgtccttataggccgtttgtatatctgctttgtgaaatgtctgttcaaatcttttgcctattttaaattgagttgtgttcgtcttcttaggattaagtaatgagttaaaaatatttctgatacaaatctttcattatatatttctaatgctttctcatctatagtttattttctcatattctttaactgtatcttttgaagagcaaattttacttttgattatgcccaatttatcaagtttttatatggctcttttgattatgcccataatcacattagactttgcctaacccaagtttgcagagattttttcttttatgcttttatctagaaattttgtagttttaggttttaaaaaagtttaatttatttatttgagacagggtattgctctttacatatactggagtgcagtgatgcaatcatggctcactgcagcctcaacctcttgggctcaagcggttctcccatctcagagtcctgagtagctggccaggtgcatgccagcttcaatgtgtttttcatttgcatttccctgataattattgacgttgagcatttttttcatatatcagttagctatttgtacgtcttcttttgagaaacatctattcgggtcttttgcccattttaaagtcagatggtttgtttgtcagctattgagttgtttgagttccttgtatattctggatattaccatcttgtcagatgcacagtttgcaaattttttttttctattttgtaggttgtctctttctctgttgtttcctccggtatgcagaagttttttagtgtgatgtaatttcatttgtctgtttttgcttttgttgcctgtactttcttattcttatccaaaaaatctttatctagatcaatgtcacgaagagtttctcctctgttttcttcgagtagttttttataattttgggtatacatttaagtctttaatctatttggaattgatttttgcatatggtgagagatcagagtctaatttcatacttttggatgtggaaagctagttttttcagcaccatttattgaagagactgtctcttctccaatgtgtgttctttgtgccttcgtcaaaaatcagttggctgtgcgtggatttatttctgtgttctctattttgttccattggtctagttttagccttaaatttaggtctgcaatttttttttttttgtatatggtgtgaagtaagagtcaaagttcattatttttcatatggatatgtaattactccagtaccatcatttagtttgaatggactgtcctttctccatggaattacatgggcatcttttgtctgaaaccaattatgtatgtttacgtatgtgtatgtttatgcatatgttataggtttaatatatattaatatatataatatataatatataaatattaatatgtattatataatatatattaatatattatattatattactatataaataatattaatatattatattaaaatattaataaatatatcatattaaatattatattaattaaatattaataaatatattatattaatatatttatatattaaacctataacatatgcatatacttatttatatataacatgcatgtacttatttatatatacaatatatatttatatattatataatatattatatgtatttatatattatatatcatatattatatgtatttatatattatatatcatataatatatatatttatattatatatattatatgatatataatattatataatgtattaatatatattaaacctatatttataattctggactcactattttgtttcattggtgtctgtgtgtatctaaccctatgccaataatgtactatcttaattaccatagctttatagtaagctttgaaatcagatagtgtattttttatcattgttttttaaaataatagtttatctttttatttgaatttgtaatcagctagtcagtttctgcaaaaagcttactgggattttgcttggaattatgttacatctgtagcatgtactatccaatattctagcctttatccacatgtggctattaaggtttaaattaattaaattaaaatttaattaattaaaattaaaacttaataattggttcctcattcacactaccatatgtcaagtgttcaatagccacatatggtcaatgtcttggaaaagtcaatacagtacatttccattattgcagtaagttctgtcaaacagcactatcgtagaccgattaggagagaactgacttaacagtattggatgctccagtcaatgaacatctttttttttttcatttatttcagtagtctctgcagtatattatagatttcagtttacatattttgcatatattttattaaatgtataacggtagaagtactattattggatgatgtgttctatagatgtattttaggtcaagtttgttgatagtgttgtttaaatctcgtatacctcttgatttttttatttacttgttctttgaattactgagacaggaatgttatatccttaactatatttgtgaatttattcacttcttccttcagttctgttaacttttgcttaggtgctttttaaaaatgaaactttcaatctctgccttttaattgtagcatttagaccatttacattcaatgtaattatcaatatcagtttatttaagtctgaagttgtgcaatttttcctctacctatattataaatctttctatatacaaaacacatgctatgttttctgcatatgttttaaatgacacccggaaagcattgacactatttttgctttaggttatctttcaaagatgttaaaaatgagaaagaaatattctgcatttatccatacacttattatttgcaaaggtttttttaaatacctttgtgtagatttcagttaccaacttgtatttccttcagcttgaagaacttacaatttcttgtaggacaggtctctgacaacaaattatctcagcttttctttgtctaaaaaagttattgcctttatttttaaaatatattttcactggatattgaattttaggtgataatctttttttttttgttagcactttaaatatgtcttctaatgtcctcttgctttcatagtttctgatgagaagtctactgttattagtatctctttgtgtgtgtctctcttttttccctctctgctattatggctatttttttttttttttttttttttggtcactggtgtcagcaatttaattatggtgtgccttggtatgttttgtgtgtgtgtgtgtgtgtgtgtgtgtgtgtgtgtgtgtgtagctgatgttctttgagctttagaatctgtgagtttgtagttttcatcaattattttttcttttcattccttttatttactcatgttcgtgttttattttatatttttaagaattttgtgcgtatttgtaataactgtttaaatgtcatttgtgaattccattgcttctaggtaggattctattgacagatattttttccctgacgagaggtcatactttccttattcttcatgtatctagtggtttttggttgaatactggatattttgaattttatgggagtgctgaattctacaatattccttaaaaatgtgttggattttgttttagcagatagctatcttacttgaagatcaatttcatattttttgatgttcattttttcatttattaaagaataggtccatggtagagtttactgatatcaacctttctggtgtctctaataaatgcaacatattcaataagatcc

SEQ ID NO: 3 - DNA, 3354 bp, Homo sapiens
  MISC_BINDING (1)..(3354): MAR X_S29 OF CHROMOSOME X
gatccctttataaaaccacaatataatggagtgctataatttcaaacagtgtttggtctgctggcagagtggtcattctaacagcagtcacagtagagtagaaataagactgcagtatatctaaggcaaaaagctgaggtttcaggagcttgaaggtaaagaggaagaaagaaatgggaatgggaattggaaagacaaatatcgttaagagaaaattgcttttaggagaggggaaagaatctatgtgtacttaagactatggaatcaatcccatttaagctgggaaactagtttcatatataactaataaattttatttacagaatatctatttacctgatctaggcttcaagccaaagggactgtgtgaaaaaccatcagttctgtcatattcctaaaaaaaaattaaaaagttaaaaataaataaataataaaacttcttttctttcaaaataatcaaggtgcttattcacatccattccaatttggggaaatacttattttcctatgattagcgaagagaaaagtaacttgcatttcaattcaagttgatacatgtcacttttaagaggtcaactaatatttgctagttgagctaaccatataggctttaaatactttcatagtagaaagaaaatgaaaatcattagtgaactgtataaaatagatcatactttttgaaagaatcagactgaagtttccgaaaaaaagaagtaagcttcaatgaaaaggtaagtgaatttagcatttactcagcatctactatggacttaacacctaacagtagataatctgaaggcaaacatatttgtatagggactgcagaatgatagatgataaatatcatctcttctatttgaatgaatattttttcaaatctttcacacacagtggtttgctatggaaagatttgtagtacattaaacaaatctgaagatggagttagaaagcttaggctatgttttgagcacaacatataatttctctgtgattgtttcttcatctttcaaatgaggttactgtgaagattaaatgagataactaaatgatgataaaataatgtaatcttagcagcaccttatttaatctgtgcaacaactctgtgaagtgagtagggctcagcttcagtcacttctctgccatttattaactaagatagtttggaaagttacccatctcttcagctgtaaaatgatgaggatcatacctattttatggggctgcttttaggtacaaatatacaggcaagcactttgttaatactaaagcattacaccaattagttttactcttttccattcacacatgaaattaatgtaatcagaattctgtagattacctaaatcttctgttaacacgtgatatgcagttcaggttaaatgtcagttgagttaccaaagcacatacatactcaccaccctatccaaatctacaagcctcccagtttgtcttcactattttggttaaattaatatgaattcctagatgaaaatttcactgatccaaatgaaataaaaaatatattacaaaactcacacctgtaatctcaacattttgggaggccaaggcaggtagatcacttgaggccaggagttcaagaccagcctgatcaacatggtgaaaccctgtctctactaaaaatacaaaaattagccaggtgtggtggcatgtgcctgtagtcctacctactcgggaggctgaggcacaagaatcgcttgaatgtgggaggtggaggttgcagtgacctgagatcgtgccactgcactccagcctaggcaacagagtgagatcatgtgtcatatatatatatatatatatatatatatatatatatatatacacacacacacacatatatatatacacatatatatacgtatatatatatatgtatatatatacatatatatacatatatatatatacgtatatatatacgtatatatatatcaatgtaaattatttgggaaatttggtatgaatagtcttccctgtgaacacagatcataaaatcatatatcaagcagacaaataagtagtagtcacttatatgcttatacttgtaacttaaagtaaaagaattacaaaagcatatgacaaagactaattttaagatatcctaatttaaattgttttctaaaagtgtgtataccattttacctatcatatgaataatttagaaacatgtttataaaattaatgtccaaatccattcaaaagttttgtaatgcagatcacccacaacaacaaagaatcctagcctattaaaaaagcaacaccacctacatataatgaaatattagcagcatctatgtaaccaaagttacacagtgaatttgggccatccaacactttgagcaaagtgttgaattcatcaaatgaatgtgtaatcatttacttactaatgccaatacactttaaggtaatcttaagtagaagagatagagtttagaattttttaaatttatctcttgttgtaaagcaatagacttgaataaataaattagaagaatcagtcattcaagccaccagagtatttgatcgagatttcacaaactctaactttctgatacccattctcccaaaaacgtgtaacctcctgtcgataggaacaacccactgcagggatgtttctcgtggaaaaaggaaatttcttttgcattggtttcagacctaactggttacaagaaaaaccaaaggccattgcacaatgctgaagtacttttttcaaatttaaaatttgaaagttgttcttaaaatctatcatttattttaaaatacggatgaatgagaaagcatagatttgataaagtgaattcttttctgcaatctacagacacttccaaaaatcactacagacactacagacactacagaaaatcataaataaacaagtgctagtatcaatatttttaccaaaaaatggcattcttagaattttttataggctagaaggtttgtacaaactaatctgccacggattttaaaatatgagtgaataaattatattgcaaaaaaaatcaggttacagagaactggcaaggaagactcttatgtaaaacacagaaaacatacaaaacgtatttttaagacaaataaaaacagaacttgtacctcagatgatactggagattgtgttgacatattagcattatcactgtcttgctaaaacataaaaataaaaagatggaagatgaaattacaatacaaatgatgatttaaacatataaaaggaaaataaaaattgttctgaccaactactaaaggaagacctactaaagatatgccatccagcacattgccactctacatgtggtctgtaaaccagcagcatagggatcctctagctagagt

SEQ ID NO: 4 - DNA, 5463 bp, Mus musculus
  MISC_FEATURE: S4_1-703_2328-5457 CONSTRUCT WITH FULL AVAI SITES
ctcgaggtctcaagataagaatgactgctgtaactcaaatccaccaaagctatttgtgttagaatgctttcctttggtaataacataataccacagagtgagtgaatgtatcaagcaaagtactcactcataatctctccacccaaatgactttgtcttctaaaattaaacccttcccagaggcctctccccttaataccatattgggctcttcacacttcttccaacatcgccttccatcctggcccttccaacctcccttctgtttgtgctaggaacagctcaaggcctcctatctaccacagagttacatggcttgccccttgccaaccccccagtaccacacagtgagtgcaaaatctcaccacattcagaacccagtcactattcaaatcatattttaacctttgcagtactgactacttttgattcatctaaacattactgaactttattctagaaaacatttaagaaatttgtagttaggttcatcctttgagaccttacatttaatttctttctatgtaaacggaaagcattgttcagtcccacgctcattatggcaacccacttccaagtacttcgtttactacgtgggctggaatcatacagttttctgttgtgcttgtgggagcagatccccctaacctctgctgatttttctcaccacttatcatacatttattacatgcatgcactgctgtgtgagtttctaaatacttgggtagcaattctctactattactttaattttcctacttgtctgcaaatacgaaaagtagcttgaaagaacttcagatctttgttgttatctgttgcaaacactccatttttctgttgtagcaaaaaaaaaaaaaaagacatccatagttgtcaatgagaatgcaagatacatacattctgcacctgtgtgctaacataagtggctgccctgtgactcagagattgcttgtccttctcctaagcctatccttttttgttactttggatacttttgttcaatgaatccagaaaaagtgtttttcagattcaccatgtgaccctcatttaaaacctgtaatccccctatggttaagttcctgcttttgtttctgttttctttctttcagtaaaaggaattgaacccagtccttccacttactatctgagcatatggctcttttagattatgatgttggtggtgttcattggtctcaccaaaatgctaaagaagccttcatcttctacttgtgggtagtctttacattcattactgcaagtttagtttatgtggtagtaccagatcctttgcttcttttgacttcatgcctacctaacagcagctctttcctttagttaagcttatgaaatagtgtttctctcatgtttcctctatattctctcttttgccttcctgtttcttcctgttgattccatcccattggagtgaaatcttatgatcttttggcatcaacaaagtgatctgcatccaaataattccacatctcattccatgttgactgtggatctatatatatatatatgtatatatgtatatatgtatatatgtatatatgtatatatgtatatatgtatatatgtatatatgtatatatgtatatatgtatatatgtatatatgtatatatgtatatatgtatatatgtatatatgtatatatgtatatatgtatatatgtatatatgtatatatgtatatatgtatatatgtatatatgtatatatgtatatatgtatatatgtatatatgtatatatgtatatatgtatatatgtatatatgtatatacgtatatatgcatatacgtatatatgtatatatgtatatatgtatatatgtatatatgtatatatgtatatatgtatatatgtatatatgtatgtatgtatgtatgtatgtatatatgtatatatgtatgtatgtatgtatgtatgtatgtatgtatatatgtatatatatatgtatgtatgtatgtatgtatgtatgtatatgtgtatatgtgtatatgtgtatatgtgtatatgtgtatatatgtatatatgtatatatgtatatatgtatatgtgtatatgtgtatatgtgtatatatgtatatatgtatatatgtatatatgtatatatataacatagtattaaattatatatacatatataagtgaaatgtcacaatcttctagaacttgctctgtatgtccacttaacatggtagagtgagctatgtcagcattttctatttcctgtgaatcattctgtgtgttgccaagaagaaatatgatatattctgaggttatgaaatgatattttggtcatcatgtttctcatcctattttcatattacctaaatacttttgcttttaaaattattattattaataataatataattatttatacaataatatttaaataatatatttatttaatataattattatatttcacataaaagcaatagttccagtgttacaaattgtaggcaactgggctgttctgattatctaagttgggcccaggatatgtgctgaatagttaaagcacatgcccagcatgtatgagggtaaaaggatgggtggatgtagtgacccatttgtaatttaagccttagcaggcagaggtgtgacccatagtgcaaagtacatagtcattataaggtcatctatatcacaatctctggattagattgattgaacctgctcagtgaccaatgtgttagcaatatacaggaggatgataacatcaacgtcagaagacacattgaagggcttacaaatagtgcccatttactttaatacagaaaaattcaatgtaccctctaggcaatttcaacttttagtctcttggtaggatagtctacatttagaatggctaattcataaattagaaagcttcttcaccccctacttttctggttatttctctatgaatgtggtaggcatgagttagtacacatgtttccatgtacatgtgtttctatgtgtctgcatgcatatggtagaatgtactcatattctatgtacagttagaacaatatttatattgtcaaagaaatcaaaaggagtattataagcttcagaaataaggataagtttgaaatattcattgttttattttttacagtattttttcctttgagaattctatgtaaagtactttgaacatatttgccttcaactcctccctcactttcaccctctcttcattcctccctttcctttccactcaaagttgagattcctttatttatttatttatccttcaaatatcactggtactatccacatgatctcaggattgaggtctgctctgacgtgtcatcctgctttcatgcaatggccttataggtggaacaacattatgaactaaccagtaccccggagctcttgactctagctgcatatatatcaaaagatggcctagtcggccatcactggaaagagaggctcattggacttgcaaactttatatgccccagtacaggggaacaccagggccaaaaagggggagtgggtgggcaggggagtgggggtgggtggatatgggggacttttggtatagcattggaaatgtaaatgagttaaatacctaataaaaaatggaaaaaaaaagtttctaatgtgtgtttctagaaacttcctctcttaaagcaacaacatgtccatgagcaatatagaattgaagatcaccatcaaatcctctttattcctcattgtttccatcatgtactaccagacctctttaaagtgtagtacagtgtgttaggaaatgagcagattatcctgggtatgtgctaaattagctactgagtcaaaatacattttttgctgaacattaagtgtttggtcatttctgggcaaaagaaagaaagaaagaaagaaaagaaagaaagaaaggaaggaaggaaggaaggaaggaaggaaggaaggaaagaaggaaggaaagaaaaaatggatgtaaattgttctgacagcatctgtctgagtcaggcagtggaatgaaggaggaatcctagagaatgcacaggaaagcagcccaaggagagtgtgggctgaaaggcatcatgttagaaacatgcactcgatgacagaaccttgagaaaaaggaactcaagcaaaagcacttatttaaaattgtaaaacgcactttattcatagccatgggggatgtcaatattccaagcataagaatgatcagtttccaatcactgtgaacccccaaaacacaaagtgaaaacccactactttatttgatgagatttggggttgctctattaatttataaaatcagagtaagacacgatataaatgaaacgattgtagttctaaagcagcggcacttccctgaacagtgtcattttgacaagtaactgctaacatcttcaggtcacagcgactgaagaaaaagtagggaaagaaggctggctgtgctgtttgacattttcttttcttatctggtgacatgaagagaagctctgggtccccctactcttgttcatatatctgttgcttttatgctgcatcctgaggtttgaagaaatgcatttggcactgagaaaagatgaggagagaatgccttggacatggtcctaacatgctttggtactgagaaaagagagcagaggagatgacatagaataggagagataatttggcctattttggccttcatctgagtgatagattttacttaacaaatagaaacaaagttttacttataaacagaaccaatgacctgtgtcatctctgatatattgagctttgaattcagtgaaattatgaactaaatatatcactccataattttctaagagggctatttgtatagtttcagtgatagtgtgacaaagtgtaatctaaatttctaaaaagtaaaataagtagataaaatagtaggtagaatagtataataatagaataagtataggtatggactagaataaatagacaaaatagtagataaaatgctaatgattttgttgacagggtaatcatgaatatttttattatttagctaaagaaccaatgttcatgtactcaagaagtgtattgaggaacttaggaaattagtctgaacaggtgagagggtgcgccagagaacctgacagcttctggaacaggcggaagcacagaggcactgaggcagcaccctgtgtgggccggggacagccggccaccttccggaccggaggacaggtgcccgcccggctggggaggcgacctaagccacagcagcagcggtcgccatcttggtccgggacccgccgaacttaggaaattagtctgaacaggtgagagggtgcgccagagaacctgacagcttctggaacaggcagaagcacagaggcgctgaggcagcaccctgtgtgggccggggacagccggccaccttccggaccggaggacaggtgcccacccggctggggaggcggcctaagccacagcagcagcggtcgccatcttggtcccggg

SEQ ID NO: 5 - DNA, 2957 bp, Chicken Lysozyme
tctagaaaacaatatatttccaaatgaaaaaaaaatctgataaaaagttgactttaaaaaagtatcaataaatgtatgcatttctcactagccttaaactctgcatgaagtgtttgatgagcagatgaagacaacatcatttctagtttcagaaataataacagcatcaaaaccgcagctgtaactccactgagctcacgttaagttttgatgtgtgaatatctgacagaactgacataatgagcactgcaaggatatcagacaagtcaaaatgaagacagacaaaagtattttttaatataaaaatggtctttatttcttcaatacaaggtaaactactattgcagtttaagaccaacacaaaagttggacagcaaattgcttaacagtctcctaaaggctgaaaaaaaggaacccatgaaagctaaaagttatgcagtatttcaagtataacatctaaaaatgatgaaacgatccctaaaggtagagattaactaagtacttctgctgaaaatgtattaaaatccgcagttgctaggataccatcttaccttgttgagaaatacaggtctccggcaacgcaacattcagcagactctttggcctgctggaatcaggaaactgcttactatatacacatataaatcctttggagttgggcattctgagagacatccatttcctgacattttgcagtgcaactctgcattccaactcagacaagctcccatgctgtatttcaaagccatttcttgaatagtttacccagacatccttgtgcaaattgggaatgaggaaatgcaatggtacaggaagacaatacagccttatgtttagaaagtcagcagcgctggtaatcttcataaaaatgtaactgttttccaaataggaatgtatttcacttgtaaaacacctggtcctttttatattacttttttttttttttaaggacacctgcactaatttgcaatcacttgtatttataaaagcacacgcactcctcattttcttacatttgaagatcagcagaatgtctctttcataatgtaataatcatatgcacagtttaaaatattttctattacaaaatacagtacacaagagggtgaggccaaagtctattacttgaatatattccaaagtgtcagcactgggggtgtaaaattacattacatggtatgaataggcggaattcttttacaactgaaatgctcgatttcattgggatcaaaggtaagtactgtttactatcttcaagagacttcaatcaagtcggtgtatttccaaagaagcttaaaagattgaagcacagacacaggccacaccagagcctacacctgctgcaataagtggtgctatagaaaggattcaggaactaacaagtgcataatttacaaatagagatgctttatcatactttgcccaacatgggaaaaaagacatcccatgagaatatccaactgaggaacttctctgtttcatagtaactcatctactactgctaagatggtttgaaaagtacccagcaggtgagatatgttcgggaggtggctgtgtggcagcgtgtcccaacacgacacaaagcaccccacccctatctgcaatgctcactgcaaggcagtgccgtaaacagctgcaacaggcatcacttctgcataaatgctgtgactcgttagcatgctgcaactgtgtttaaaacctatgcactccgttaccaaaataatttaagtcccaaataaatccatgcagcttgcttcctatgccaacatattttagaaagtattcattcttctttaagaatatgcacgtggatctacacttcctgggatctgaagcgatttatacctcagttgcagaagcagtttagtgtcctggatctgggaaggcagcagcaaacgtgcccgttttacatttgaacccatgtgacaacccgccttactgagcatcgctctaggaaatttaaggctgtatccttacaacacaagaaccaacgacagactgcatataaaattctataaataaaaataggagtgaagtctgtttgacctgtacacacagagcatagagataaaaaaaaaaggaaatcaggaattacgtatttctataaatgccatatatttttactagaaacacagatgacaagtatatacaacatgtaaatccgaagttatcaacatgttaactaggaaaacatttacaagcatttgggtatgcaactagatcatcaggtaaaaaatcccattagaaaaatctaagcctcgccagtttcaaaggaaaaaaaccagagaacgctcactacttcaaaggaaaaaaaataaagcatcaagctggcctaaacttaataaggtatctcatgtaacaacagctatccaagctttcaagccacactataaataaaaacctcaagttccgatcaacgttttccataatgcaatcagaaccaaaggcattggcacagaaagcaaaaagggaatgaaagaaaagggctgtacagtttccaaaaggttcttcttttgaagaaatgtttctgacctgtcaaaacatacagtccagtagaaattttactaagaaaaaagaacaccttacttaaaaaaaaaaaacaacaaaaaaaacaggcaaaaaaacctctcctgtcactgagctgccaccacccaaccaccacctgctgtgggctttgtctcccaagacaaaggacacacagccttatccaatattcaacattacttataaaaacgctgatcagaagaaataccaagtatttcctcagagactgttatatcctttcatcggcaacaagagatgaaatacaacagagtgaatatcaaagaaggcggcaggagccaccgtggcaccatcaccgggcagtgcagtgcccaactgccgttttctgagcacgcataggaagccgtcagtcacatgtaataaaccaaaacctggtacagttatattatggatcc

SEQ ID NO: 6 - DNA, 3659 bp, Homo sapiens
  MISC_FEATURE: 1_68R(NcoI+XbaI filled)
gtacccccaaaagaaagagatcctcaggtacaaaatccccttccaagggtcttcaattcaatccaacacatttgtaattgagtacctttttcatgctaaactttcttgttttatacaaagaaaatgaagatgtggttattgctcactaggagtttacaatcttgagaaaagatgtaggccaagttacttgacctctaactacttctttttctcatccacaaagtgagacaattggaatattttaaaaaatatatatatatatttttatatatatgtgtatatatatattttatatatatgtgtatatatatattttatatatatgtgtatatatatattttatatatatgtgtgtatatatatactttatatatatgtgtgtatatatattttatatatatgtgtatatatatatattttatatatatgtgtatatatatattttatatatatgtgtatatatatattttatatatatgtgtgtatatatatattttatatatatgtgtgtatatatattttatatatatgtgtatatatatattttatatatatgtgtatatatatattttatatatgtgtgtatatatatattttatatatgtgtgtatatatatattttatatatatgtgtgtatatatatattttatatatatgtgtgtatatatatattttatatatatgtgtgtatatatatattttatatatatgtgtgtatatatatattttatatatatgtgtgtatatatatattttatatatatgtgtgtatatatatattttatatatatgtgtgtatatatatattttatatatatgtgtgtatatatatattttatatatatgtgtgtatatatatattttatatatatgtgtgtatatatatatattttatatatatgtgtgtatatatatatattttatatatatatgtgtgtatatatatatattttatatatatatgtgtatatatatatatatatatattttttttttgagacagagtctcgctctgtcgcccaggctggagtgcagtggcgcgatctcagctcactgcaacctccacctcctgggttcaagccgttctcctgcctcagcctcccgagtagctgggactacaggcacgtgccaccacgtccagctaatagttttgtatctttagtagagatggggtttcaccatattggtcaggatggtctcgatctcttgacctcatgatccgcccacctcagcctcccaaagtgctgggattacaggcgtgagccaccactcccagcctaaaatatttttatgatcagattttttttcccatgcatggatatttggaagaatatatatatatacagataaaataggatgttaagggagcacagagaagaggcacctaacccacacttcagatgggatagaagttcttaacgatttttacaatttgatatcttactttccttatgtggcccagctaaaatgaaaccttttatgattcccctaattcagaatttcccaaactggatgcttagttaaaaacaaacaaacaaaaacagtggttaggaaaggttaagaagctattttagatccaaccctatatagatgttcaacaccatgacttctaagtgtttttgacatcagaaagtattattaaagaaagatttaactcaaaaaacaactttaaacacaacctatgaaacatgccattcatttaatatttcctagcaacaagccacctactgatacatattaaggcaaaggatagttaatagtaaaacagaatggaattggtactttcacatccactcacaacggaatagctggtgccagattaaccttcttggtttaaataaatattaaactggatgaaatataggaagcaactgttttcagatggtaggcaataggtagcacaatctgtgatccctgagataatgaaactgtagcagttgctaatggacaagcctctggaggctcaccctgtgcatgtaacatttatccctcagccttgaatgtttggagaaactcctgctaggtttctgggtctctctcttcagggttgtcttttcttagattctctgaattgcagattccagctgcttcaactgccaaactgatcttgcctcctcagttcagggatctgcaagataagagcatttgcttttatatatgctcttattttatgaggttggtataatctagctagagtcgagatctttggccatattgttcaatggacaaaatttagccttcgaaggcaggccgatttgaggttaatactacctttaccacttgatagctatgtgaccttggccatgtggtttcaacagtctgaacctcattttctctgtgtatgtgtggtcctccttacaagtttgtgaaaaatgtgaagtccttagccatgatagcccaatataacaggctaaatgataataggtttatgttcttttcctttatattctcagataagcactgtccaagtttgaggtgttttgaggtctcgcctgatttggattgtttgagtttatgctattctttgaattctttgagctgttctgaagcagtgtatcatgaacaaaaacatccccagttcagtccaaacccctggttacatatcattcttatgccatgttataaccagtttgagagtgttccctctgttattgcatttaagtttcagcctcacacagaaattcagcagccaatttctaagccctaagcataaaatctggggtgggggggggggatggcctgaagagcagcattatgaatagcaccattataattaatgatctctcaggaagatttacaatcacaggtagcagataaaacaaatagtactgcttctgcacttcccctccttttattcgctatgaaattttatgggaaatcagtccagtgaaaaatgtaagctcttaatctttcccagaaatcctacctcatttgatgaatactttgagggaatgaattagagcatttttttcttttatagtctacttcgcatttacgaagtgaggacggtagcttaggctgcctggccaactgatgagaaggtcagaggcatttttagagacctctgttgtctttcattcatgttcattttccacaaggcaagtaatttccaacaaatcagtgtcttcattagtaataagattattaacaacaataatagtcatagtaactattcagtgagagtccattatatatcaggcattctacaaggtactttatatacatctgagtaaacctcacacaattctacagggaggtatttctatccccatttaacaaataaggaaacgaagtccaagtaaattaacttgcccaaggtcacacagatagtacctggcagaacaggaatttaaacctaaatttgtccaactccaaaagcagccttctatttgttataaatgctgcctctcattatcacatattttattattaacaacaacaaacataccaattagcttaagatacaatacaaccagataatcatgatgacaacagtaattgttatactattataataaaatagatgttttgtatgttactataatcttgaatttgaatagaaatttgcatttctgaaagcatgttcctgtcatctaatatgattctgtatctattaaaatagtactacatctagcccgggctcgacattgattattga

SEQ ID NO: 7 - DNA, 2751 bp, Homo sapiens
  MISC_FEATURE: 1_68R2 (NcoI + XbaI filled)
gtacccccaaaagaaagagatcctcaggtacaaaatccccttccaagggtcttcaattcaatccaacacatttgtaattgagtacctttttcatgctaaactttcttgttttatacaaagaaaatgaagatgtggttattgctcactaggagtttacaatcttgagaaaagatgtaggccaagttacttgacctctaactacttctttttctcatccacaaagtgagacaattggaatattttaaaaaatatatatatatatttttatatatatgtgtatatatatattttatatatatgtgtatatatatattttatatatatgtgtatatatatattttatatatatgtgtgtatatatatactttatatatatgtgtgtatatatattttatatatatgtgtatatatatatattttatatatatgtgtatatatatattttatatatatgtgtatatatatattttatatatatgtgtgtatatatatattttatatatatgtgtgtatatatattttatatatatgtgtatatatatattttatatatatgtgtatatatatattttatatatgtgtgtatatatatattttatatatgtgtgtatatatatattttatatatatgtgtgtatatatatattttatatatatgtgtgtatatatatattttatatatatgtgtgtatatatatattttatatatatgtgtgtatatatatattttatatatatgtgtgtatatatatattttatatatatgtgtgtatatatatattttatatatatgtgtgtatatatatattttatatatatgtgtgtatatatatattttatatatatgtgtgtatatatatattttatatatatgtgtgtatatatatatattttatatatatgtgtgtatatatatatattttatatatatatgtgtgtatatatatatattttatatatatatgtgtatatatatatatatatatattttttttttgagacagagtctcgctctgtcgcccaggctggagtgcagtggcgcgatctcagctcactgcaacctccacctcctgggttcaagccgttctcctgcctcagcctcccgagtagctgggactacaggcacgtgccaccacgtccagctaatagttttgtatctttagtagagatggggtttcaccatattggtcaggatggtctcgatctcttgacctcatgatccgcccacctcagcctcccaaagtgctgggattacaggcgtgagccaccactcccagcctaaaatatttttatgatctttggccatattgttcaatggacaaaatttagccttcgaaggcaggccgatttgaggttaatactacctttaccacttgatagctatgtgaccttggccatgtggtttcaacagtctgaacctcattttctctgtgtatgtgtggtcctccttacaagtttgtgaaaaatgtgaagtccttagccatgatagcccaatataacaggctaaatgataataggtttatgttcttttcctttatattctcagataagcactgtccaagtttgaggtgttttgaggtctcgcctgatttggattgtttgagtttatgctattctttgaattctttgagctgttctgaagcagtgtatcatgaacaaaaacatccccagttcagtccaaacccctggttacatatcattcttatgccatgttataaccagtttgagagtgttccctctgttattgcatttaagtttcagcctcacacagaaattcagcagccaatttctaagccctaagcataaaatctggggtgggggggggggatggcctgaagagcagcattatgaatagcaccattataattaatgatctctcaggaagatttacaatcacaggtagcagataaaacaaatagtactgcttctgcacttcccctccttttattcgctatgaaattttatgggaaatcagtccagtgaaaaatgtaagctcttaatctttcccagaaatcctacctcatttgatgaatactttgagggaatgaattagagcatttttttcttttatagtctacttcgcatttacgaagtgaggacggtagcttaggctgcctggccaactgatgagaaggtcagaggcatttttagagacctctgttgtctttcattcatgttcattttccacaaggcaagtaatttccaacaaatcagtgtcttcattagtaataagattattaacaacaataatagtcatagtaactattcagtgagagtccattatatatcaggcattctacaaggtactttatatacatctgagtaaacctcacacaattctacagggaggtatttctatccccatttaacaaataaggaaacgaagtccaagtaaattaacttgcccaaggtcacacagatagtacctggcagaacaggaatttaaacctaaatttgtccaactccaaaagcagccttctatttgttataaatgctgcctctcattatcacatattttattattaacaacaacaaacataccaattagcttaagatacaatacaaccagataatcatgatgacaacagtaattgttatactattataataaaatagatgttttgtatgttactataatcttgaatttgaatagaaatttgcatttctgaaagcatgttcctgtcatctaatatgattctgtatctattaaaatagtactacatctagcccgggctcgacattgattattga

SEQ ID NO: 8 - DNA, 2082 bp, Homo sapiens
  MISC_FEATURE: 1_6R2(HindIII filled)
tcgacatggaattacatgggcatcttttgtctgaaaccaattatgtatgtttacgtatgtgtatgtttatgcatatgttataggtttaatatatattaatatatataatatataatatataaatattaatatgtattatataatatatattaatatattatattatattactatataaataatattaatatattatattaaaatattaataaatatatcatattaaatattatattaattaaatattaataaatatattatattaatatatttatatattaaacctataacatatgcatatacttatttatatataacatgcatgtacttatttatatatacaatatatatttatatattatataatatattatatgtatttatatattatatatcatatattatatgtatttatatattatatatcatataatatatatatttatattatatatattatatgatatataatattatataatgtattaatatatattaaacctatatttataattctggactcactattttgtttcattggtgtctgtgtgtatctaaccctatgccaataatgtactatcttaattaccatagctttatagtaagctagcttgatatcgaattcctgcagcccgggggatccactagatttggccatattgttcaatggacaaaatttagccttcgaaggcaggccgatttgaggttaatactacctttaccacttgatagctatgtgaccttggccatgtggtttcaacagtctgaacctcattttctctgtgtatgtgtggtcctccttacaagtttgtgaaaaatgtgaagtccttagccatgatagcccaatataacaggctaaatgataataggtttatgttcttttcctttatattctcagataagcactgtccaagtttgaggtgttttgaggtctcgcctgatttggattgtttgagtttatgctattctttgaattctttgagctgttctgaagcagtgtatcatgaacaaaaacatccccagttcagtccaaacccctggttacatatcattcttatgccatgttataaccagtttgagagtgttccctctgttattgcatttaagtttcagcctcacacagaaattcagcagccaatttctaagccctaagcataaaatctggggtgggggggggggatggcctgaagagcagcattatgaatagcaccattataattaatgatctctcaggaagatttacaatcacaggtagcagataaaacaaatagtactgcttctgcacttcccctccttttattcgctatgaaattttatgggaaatcagtccagtgaaaaatgtaagctcttaatctttcccagaaatcctacctcatttgatgaatactttgagggaatgaattagagcatttttttcttttatagtctacttcgcatttacgaagtgaggacggtagcttaggctgcctggccaactgatgagaaggtcagaggcatttttagagacctctgttgtctttcattcatgttcattttccacaaggcaagtaatttccaacaaatcagtgtcttcattagtaataagattattaacaacaataatagtcatagtaactattcagtgagagtccattatatatcaggcattctacaaggtactttatatacatctgagtaaacctcacacaattctacagggaggtatttctatccccatttaacaaataaggaaacgaagtccaagtaaattaacttgcccaaggtcacacagatagtacctggcagaacaggaatttaaacctaaatttgtccaactccaaaagcagccttctatttgttataaatgctgcctctcattatcacatattttattattaacaacaacaaacataccaattagcttaagatacaatacaaccagataatcatgatgacaacagtaattgttatactattataataaaatagatgttttgtatgttactataatcttgaatttgaatagaaatttgcatttctgaaagcatgttcctgtcatctaatatgattctgtatctattaaaatagtactacatctagccc

SEQ ID NO: 9 - DNA, 3345 bp, Homo sapiens
  X_S29(2*HindIII, SalI filled) (1)..(3345)
  misc_feature (1)..(3345)
gatccctttataaaaccacaatataatggagtgctataatttcaaacagtgtttggtctgctggcagagtggtcattctaacagcagtcacagtagagtagaaataagactgcagtatatctaaggcaaaaagctgaggtttcaggagcttgaaggtaaagaggaagaaagaaatgggaatgggaattggaaagacaaatatcgttaagagaaaattgcttttaggagaggggaaagaatctatgtgtacttaagactatggaatcaatcccatttaagctgggaaactagtttcatatataactaataaattttatttacagaatatctatttacctgatctaggcttcaagccaaagggactgtgtgaaaaaccatcagttctgtcatattcctaaaaaaaaattaaaaagttaaaaataaataaataataaaacttcttttctttcaaaataatcaaggtgcttattcacatccattccaatttggggaaatacttattttcctatgattagcgaagagaaaagtaacttgcatttcaattcaagttgatacatgtcacttttaagaggtcaactaatatttgctagttgagctaaccatataggctttaaatactttcatagtagaaagaaaatgaaaatcattagtgaactgtataaaatagatcatactttttgaaagaatcagactgaagtttccgaaaaaaagaagtaagctagcttcaatgaaaaggtaagtgaatttagcatttactcagcatctactatggacttaacacctaacagtagataatctgaaggcaaacatatttgtatagggactgcagaatgatagatgataaatatcatctcttctatttgaatgaatattttttcaaatctttcacacacagtggtttgctatggaaagatttgtagtacattaaacaaatctgaagatggagttagaaagctagcttaggctatgttttgagcacaacatataatttctctgtgattgtttcttcatctttcaaatgaggttactgtgaagattaaatgagataactaaatgatgataaaataatgtaatcttagcagcaccttatttaatctgtgcaacaactctgtgaagtgagtagggctcagcttcagtcacttctctgccatttattaactaagatagtttggaaagttacccatctcttcagctgtaaaatgatgaggatcatacctattttatggggctgcttttaggtacaaatatacaggcaagcactttgttaatactaaagcattacaccaattagttttactcttttccattcacacatgaaattaatgtaatcagaattctgtagattacctaaatcttctgttaacacgtgatatgcagttcaggttaaatgtcagttgagttaccaaagcacatacatactcaccaccctatccaaatctacaagcctcccagtttgtcttcactattttggttaaattaatatgaattcctagatgaaaatttcactgatccaaatgaaataaaaaatatattacaaaactcacacctgtaatctcaacattttgggaggccaaggcaggtagatcacttgaggccaggagttcaagaccagcctgatcaacatggtgaaaccctgtctctactaaaaatacaaaaattagccaggtgtggtggcatgtgcctgtagtcctacctactcgggaggctgaggcacaagaatcgcttgaatgtgggaggtggaggttgcagtgacctgagatcgtgccactgcactccagcctaggcaacagagtgagatcatgtgtcatatatatatatatatatatatatatatatatatatatatacacacacacacacatatatatatacacatatatatacgtatatatatatatgtatatatatacatatatatacatatatatatatacgtatatatatacgtatatatatatcaatgtaaattatttgggaaatttggtatgaatagtcttccctgtgaacacagatcataaaatcatatatcaagcagacaaataagtagtagtcacttatatgcttatacttgtaacttaaagtaaaagaattacaaaagcatatgacaaagactaattttaagatatcctaatttaaattgttttctaaaagtgtgtataccattttacctatcatatgaataatttagaaacatgtttataaaattaatgtccaaatccattcaaaagttttgtaatgcagatcacccacaacaacaaagaatcctagcctattaaaaaagcaacaccacctacatataatgaaatattagcagcatctatgtaaccaaagttacacagtgaatttgggccatccaacactttgagcaaagtgttgaattcatcaaatgaatgtgtaatcatttacttactaatgccaatacactttaaggtaatcttaagtagaagagatagagtttagaattttttaaatttatctcttgttgtaaagcaatagacttgaataaataaattagaagaatcagtcattcaagccaccagagtatttgatcgagatttcacaaactctaactttctgatacccattctcccaaaaacgtgtaacctcctgtcgataggaacaacccactgcagggatgtttctcgtggaaaaaggaaatttcttttgcattggtttcagacctaactggttacaagaaaaaccaaaggccattgcacaatgctgaagtacttttttcaaatttaaaatttgaaagttgttcttaaaatctatcatttattttaaaatacggatgaatgagaaagcatagatttgataaagtgaattcttttctgcaatctacagacacttccaaaaatcactacagacactacagacactacagaaaatcataaataaacaagtgctagtatcaatatttttaccaaaaaatggcattcttagaattttttataggctagaaggtttgtacaaactaatctgccacggattttaaaatatgagtgaataaattatattgcaaaaaaaatcaggttacagagaactggcaaggaagactcttatgtaaaacacagaaaacatacaaaacgtatttttaagacaaataaaaacagaacttgtacctcagatgatactggagattgtgttgacatattagcattatcactgtcttgctaaaacataaaaataaaaagatggaagatgaaattacaatacaaatgatgatttaaacatataaaaggaaaataaaaattgttctgaccaactactaaaggaagacctactaaagatatgccatccagcacattgccactctacatgtggtctgtaaaccagcagcatagg

SEQ ID NO: 10 - DNA, 892 bp, Homo sapiens
  misc_feature (1)..(892): X_S29R3
aattcaacactttgctcaaagtgttggatggcccaaattcactgtgtaactttggttacatagatgctgctaatatttcattatatgtaggtggtgttgcttttttaataggctaggattctttgttgttgtgggtgatctgcattacaaaacttttgaatggatttggacattaattttataaacatgtttctaaattattcatatgataggtaaaatggtatacacacttttagaaaacaatttaaattaggatatcttaaaattagtctttgtcatatgcttttgtaattcttttactttaagttacaagtataagcatataagtgactactacttatttgtctgcttgatatatgattttatgatctgtgttcacagggaagactattcataccaaatttcccaaataatttacattgatatatatatacgtatatatatacgtatatatatatatgtatatatatgtatatatatacatatatatatatacgtatatatatgtgtatatatatatgtgtgtgtgtgtgtatatatatatatatatatatatatatatatatatatatatgacacatgatctcactctgttgcctaggctggagtgcagtggcacgatctcaggtcactgcaacctccacctcccacattcaagcgattcttgtgcctcagcctcccgagtaggtaggactacaggcacatgccaccacacctggctaatttttgtatttttagtagagacagggtttcaccatgttgatcaggctggtcttgaactcctggcctcaagtgatctacctgccttggcctcccaaaatgttgagattacaggtgtgagttttgtaatatattttttatttcatttggatcagtgaaattttcatctagg

SEQ ID NO: 11 - DNA, 1173 bp, Homo sapiens
  C_GAPDH promoter (1)..(363): Human CMV IE gene enhancer
ctagttattaatagtaatcaattacggggtcattagttcatagcccatatatggagttccgcgttacataacttacggtaaatggcccgcctggctgaccgcccaacgacccccgcccattgacgtcaataatgacgtatgttcccatagtaacgccaatagggactttccattgacgtcaatgggtggactatttacggtaaactgcccacttggcagtacatcaagtgtatcatatgccaagtacgccccctattgacgtcaatgacggtaaatggcccgcctggcattatgcccagtacatgaccttatgggactttcctacttggcagtacatctacgtattagtcatcgctattaccatgacctcgaggagaagttccccaactttcccgcctctcagcctttgaaagaaagaaaggggagggggcaggccgcgtgcagccgcgagcggtgctgggctccggctccaattccccatctcagtcgttcccaaagtcctcctgtttcatccaagcgtgtaagggtccccgtccttgactccctagtgtcctgctgcccacagtccagtcctgggaaccagcaccgatcacctcccatcgggccaatctcagtcccttcccccctacgtcggggcccacacgctcggtgcgtgcccagttgaaccaggcggctgcggaaaaaaaaaagcggggagaaagtagggcccggctactagcggttttacgggcgcacgtagctcaggcctcaagaccttgggctgggactggctgagcctggcgggaggcggggtccgagtcaccgcctgccgccgcgcccccggtttctataaattgagcccgcagcctcccgcttcgctctctgctcctcctgttcgacagtcagccgcatcttcttttgcgtcgccaggtgaagacgggcggagagaaacccgggaggctagggacggcctgaaggcggcaggggcgggcgcaggccggatgtgttcgcgccgctgcggggtgggcccgggcggcctccgcattgcaggggcgggcggaggacgtgatgcggcgcgggctgggcatggaggcctggtgggggaggggaggggaggcgtgtgtgtcggccggggccactaggcgctcactgttctctccctccgcgcagccgagccacatcgctcagacacca

SEQ ID NO: 12 - DNA, 411 bp, Homo sapiens
  misc_feature: hSRP14
atggtgttgttggagagcgagcagttcctgacggagctgaccagacttttccagaagtgccggacgtcgggcagcgtctatatcaccttgaagaagtatgacggtcgaaccaaacccattccaaagaagggtactgtggagggctttgagcccgcagacaacaagtgtctgttaagagctaccgatgggaagaagaagatcagcactgtggtgagctccaaggaagtgaataagtttcagatggcttattcaaacctccttagagctaacatggatgggctgaagaagagagacaaaaagaacaaaactaagaagaccaaagcagcagcagcagcagcagcagcagcacctgccgcagcagcaacagcaccaacaacagcagcaacaacagcagcaacagcagcacagtaa

SEQ ID NO: 13 - protein, 136 aa, Homo sapiens
  MISC_FEATURE: hSRP14
MVLLESEQFLTELTRLFQKCRTSGSVYITLKKYDGRTKPIPKKGTVEGFEPADNKCLLRATDGKKKISTVVSSKEVNKFQMAYSNLLRANMDGLKKRDKKNKTKKTKAAAAAAAAAPAAAATAPTTAATTAATAAQ

SEQ ID NO: 14 - DNA, 1431 bp, Homo sapiens
  misc_feature: hSEC61A1
atggcaatcaaatttctggaagtcatcaagcccttctgtgtcatcctgccggaaattcagaagccagagaggaagattcagtttaaggagaaagtgctgtggaccgctatcaccctctttatcttcttagtgtgctgccagattcccctgtttgggatcatgtcttcagattcagctgaccctttctattggatgagagtgattctagcctctaacagaggcacattgatggagctagggatctctcctattgtcacgtctggccttataatgcaactcttggctggcgccaagataattgaagttggtgacaccccaaaagaccgagctctcttcaacggagcccaaaagttatttggcatgatcattactatcggccagtctatcgtgtatgtgatgaccgggatgtatggggacccttctgaaatgggtgctggaatttgcctgctaatcaccattcagctctttgttgctggcttaattgtcctacttttggatgaactcctgcaaaaaggatatggccttggctctggtatttctctcttcattgcaactaacatctgtgaaaccatcgtatggaaggcattcagccccactactgtcaacactggccgaggaatggaatttgaaggtgctatcatcgcacttttccatctgctggccacacgcacagacaaggtccgagcccttcgggaggcgttctaccgccagaatcttcccaacctcatgaatctcatcgccaccatctttgtctttgcagtggtcatctatttccagggcttccgagtggacctgccaatcaagtcggcccgctaccgtggccagtacaacacctatcccatcaagctcttctatacgtccaacatccccatcatcctgcagtctgccctggtgtccaacctttatgtcatctcccaaatgctctcagctcgcttcagtggcaacttgctggtcagcctgctgggcacctggtcggacacgtcttctgggggcccagcacgtgcttatccagttggtggcctttgctattacctgtcccctccagaatcttttggctccgtgttagaagacccggtccatgcagttgtatacatagtgttcatgctgggctcctgtgcattcttctccaaaacgtggattgaggtctcaggttcctctgccaaagatgttgcaaagcagctgaaggagcagcagatggtgatgagaggccaccgagagacctccatggtccatgaactcaaccggtacatccccacagccgcggcctttggtgggctgtgcatcggggccctctcggtcctggctgacttcctaggcgccattgggtctggaaccgggatcctgctcgcagtcacaatcatctaccagtactttgagatcttcgttaaggagcaaagcgaggttggcagcatgggggccctgctcttctga

SEQ ID NO: 15 - protein, 476 aa, Homo sapiens
  MISC_FEATURE: hSEC61A1
MAIKFLEVIKPFCVILPEIQKPERKIQFKEKVLWTAITLFIFLVCCQIPLFGIMSSDSADPFYWMRVILASNRGTLMELGISPIVTSGLIMQLLAGAKIIEVGDTPKDRALFNGAQKLFGMIITIGQSIVYVMTGMYGDPSEMGAGICLLITIQLFVAGLIVLLLDELLQKGYGLGSGISLFIATNICETIVWKAFSPTTVNTGRGMEFEGAIIALFHLLATRTDKVRALREAFYRQNLPNLMNLIATIFVFAVVIYFQGFRVDLPIKSARYRGQYNTYPIKLFYTSNIPIILQSALVSNLYVISQMLSARFSGNLLVSLLGTWSDTSSGGPARAYPVGGLCYYLSPPESFGSVLEDPVHAVVYIVFMLGSCAFFSKTWIEVSGSSAKDVAKQLKEQQMVMRGHRETSMVHELNRYIPTAAAFGGLCIGALSVLADFLGAIGSGTGILLAVTIIYQYFEIFVKEQSEVGSMGALLF

SEQ ID NO: 16 - DNA, 291 bp, Homo sapiens
  misc_feature: hSEC61B
atgcctggtccgacccccagtggcactaacgtgggatcctcagggcgctctcccagcaaagcagtggccgcccgggcggcgggatccactgtccggcagaggaaaaatgccagctgtgggacaaggagtgcaggccgcacaacctcggcaggcaccggggggatgtggcgattctacacagaagattcacctgggctcaaagttggccctgttccagtattggttatgagtcttctgttcatcgcttctgtatttatgttgcacatttggggcaagtacactcgttcgtag

SEQ ID NO: 17 - protein, 96 aa, Homo sapiens
  MISC_FEATURE: hSEC61B
MPGPTPSGTNVGSSGRSPSKAVAARAAGSTVRQRKNASCGTRSAGRTTSAGTGGMWRFYTEDSPGLKVGPVPVLVMSLLFIASVFMLHIWGKYTRS

SEQ ID NO: 18 - DNA, 207 bp, Homo sapiens
  misc_feature: hSEC61G
atggatcaggtaatgcagtttgttgagccaagtcggcagtttgtaaaggactccattcggctggttaaaagatgcactaaacctgatagaaaagaattccagaagattgccatggcaacagcaataggatttgctataatgggattcattggcttctttgtgaaattgatccatattcctattaataacatcattgttggtggctga

SEQ ID NO: 19 - protein, 68 aa, Homo sapiens
  MISC_FEATURE: hSEC61G
MDQVMQFVEPSRQFVKDSIRLVKRCTKPDRKEFQKIAMATAIGFAIMGFIGFFVKLIHIPINNIIVGG

SEQ ID NO: 20 - DNA, 1515 bp, Homo sapiens
  misc_feature: hSRP54
atggttctagcagaccttggaagaaaaataacatcagcattacgctcgttgagcaatgccaccattatcaatgaagaggtattgaatgctatgctaaaagaagtctgtaccgctttgttggaagcagatgttaatattaaactagtgaagcaactaagagaaaatgttaagtctgctattgatcttgaagagatggcatctggtcttaacaaaagaaaaatgattcagcatgctgtatttaaagaacttgtgaagcttgtagaccctggagttaaggcatggacacccactaaaggaaaacaaaatgtgattatgtttgttggattgcaagggagtggtaaaacaacaacatgttcaaagctagcatattattaccagaggaaaggttggaagacctgtttaatatgtgcagacacattcagagcaggggcttttgaccaactaaaacagaatgctaccaaagcaagaattccattttatggaagctatacagaaatggatcctgtcatcattgcttctgaaggagtagagaaatttaaaaatgaaaattttgaaattattattgttgatacaagtggccgccacaaacaagaagactctttgtttgaagaaatgcttcaagttgctaatgctatacaacctgataacattgtttatgtgatggatgcctccattgggcaggcttgtgaagcccaggctaaggcttttaaagataaagtagatgtagcctcagtaatagtgacaaaacttgatggccatgcaaaaggaggtggtgcactcagtgcagtcgctgccacaaaaagtccgattattttcattggtacaggggaacatatagatgactttgaacctttcaaaacacagccttttattagcaaacttcttggtatgggcgacattgaaggactgatagataaagtcaacgagttgaagttggatgacaatgaagcacttatagagaagttgaaacatggtcagtttacgttgcgagacatgtatgagcaatttcaaaatatcatgaaaatgggccccttcagtcagatcttggggatgatccctggttttgggacagattttatgagcaaaggaaatgaacaggagtcaatggcaaggctaaagaaattaatgacaataatggatagtatgaatgatcaagaactagacagtacggatggtgccaaagtttttagtaaacaaccaggaagaatccaaagagtagcaagaggatcgggtgtatcaacaagagatgttcaagaacttttgacacaatataccaagtttgcacagatggtaaaaaagatgggaggtatcaaaggacttttcaaaggtggcgacatgtctaagaatgtgagccagtcacagatggcaaaattgaaccaacaaatggccaaaatgatggatcctagggttcttcatcacatgggtggtatggcaggacttcagtcaatgatgaggcagtttcaacagggtgctgctggcaacatgaaaggcatgatgggattcaataatatgtaa

SEQ ID NO: 21 - protein, 504 aa, Homo sapiens
  MISC_FEATURE: hSRP54
MVLADLGRKITSALRSLSNATIINEEVLNAMLKEVCTALLEADVNIKLVKQLRENVKSAIDLEEMASGLNKRKMIQHAVFKELVKLVDPGVKAWTPTKGKQNVIMFVGLQGSGKTTTCSKLAYYYQRKGWKTCLICADTFRAGAFDQLKQNATKARIPFYGSYTEMDPVIIASEGVEKFKNENFEIIIVDTSGRHKQEDSLFEEMLQVANAIQPDNIVYVMDASIGQACEAQAKAFKDKVDVASVIVTKLDGHAKGGGALSAVAATKSPIIFIGTGEHIDDFEPFKTQPFISKLLGMGDIEGLIDKVNELKLDDNEALIEKLKHGQFTLRDMYEQFQNIMKMGPFSQILGMIPGFGTDFMSKGNEQESMARLKKLMTIMDSMNDQELDSTDGAKVFSKQPGRIQRVARGSGVSTRDVQELLTQYTKFAQMVKKMGGIKGLFKGGDMSKNVSQSQMAKLNQQMAKMMDPRVLHHMGGMAGLQSMMRQFQQGAAGNMKGMMGFNNM

SEQ ID NO: 22 - DNA, 249 bp, Homo sapiens
  misc_feature: hSRP9
atgccgcagtaccagacctgggaggagttcagccgcgctgccgagaagctttacctcgctgaccctatgaaggcacgtgtggttctcaaatataggcattctgatgggaacttgtgtgttaaagtaacagatgatttagttagacagtgtcttgctctattgctcaggctgcagtgcagtggcatgatcatagctcactgcatcctcgacctcctgggctcaagcggtcctcttgcttcagcctcctga

SEQ ID NO: 23 - protein, 82 aa, Homo sapiens
  MISC_FEATURE: hSRP9
MPQYQTWEEFSRAAEKLYLADPMKARVVLKYRHSDGNLCVKVTDDLVRQCLALLLRLQCSGMIIAHCILDLLGSSGPLASAS

SEQ ID NO: 24 - DNA, 1917 bp, Homo sapiens
  misc_feature: hSRPRalpha
atgctcgacttcttcaccattttctccaagggcgggcttgtgctctggtgcttccagggcgttagcgactcatgcaccggacccgttaacgcgttgattcgttccgtgctgctgcaggaacggggaggtaacaactccttcacccatgaggcactcacactcaagtataaactggacaaccagtttgagctggtgtttgtggttggttttcagaagatcctgacactgacatatgtagacaaattgatagatgacgtgcatcggctgtttcgggacaagtaccgcacagagatccaacagcaaagtgctttaagtttattaaatggcacttttgatttccaaaatgacttcctgcggctccttcgtgaagcagaggagagcagtaagatccgtgctcccactaccatgaagaaatttgaagattctgaaaaggccaagaaacctgtgaggtccatgattgagacacggggggaaaagcccaaggaaaaagcaaagaatagcaaaaaaaagggggccaagaaggaaggttctgatggtcctttggctaccagcaaaccagtccctgcagaaaagtcaggtcttccagtgggtcctgagaacggagtagaactttccaaagaggagctgatccgcaggaagcgcgaggagttcattcagaagcatgggaggggtatggagaagtccaacaagtccacgaagtcagatgctccaaaggagaagggcaaaaaagcaccccgggtgtgggaactgggtggctgtgctaacaaagaagtgttggattacagtactcccaccaccaatggaacccctgaggctgccttgtctgaggacatcaacctgattcgagggactgggtctggggggcagcttcaggatctggactgcagcagctctgatgacgaaggggctgctcaaaactctaccaaacctagtgcgaccaagggaacactgggtggcatgtttggtatgctgaagggccttgtgggttcaaagagcttgagtcgtgaagacatggaatctgtgctggacaagatgcgtgatcatctcattgctaagaacgtggctgcagacattgccgtccagctctgtgaatctgttgccaacaagttggaagggaaggtgatggggacgttcagcacggtgacttccacagtaaagcaagccctacaggagtccctggtgcagattctgcagccacagcgtcgtgtagacatgctccgggacatcatggatgcccagcgtcgccagcgcccttatgtcgtcaccttctgcggcgttaatggagtggggaaatctactaatcttgccaagatttccttctggttgttagagaatggcttcagtgtcctcattgctgcctgtgatacatttcgtgctggggccgtggagcagctgcgtacacacacccggcgtttgagtgccctacaccctccagagaagcatggtggccgcaccatggtgcagttgtttgaaaagggctatggcaaggatgctgctggcattgccatggaagccattgcttttgcacgtaaccaaggctttgacgtggtgctggtggacacggcaggccgcatgcaagacaatgcccctctgatgactgccctggccaaactcattactgtcaatacacctgatttggtgctgtttgtaggagaagccttagtaggcaatgaagccgtggaccagctggtcaagttcaacagagccttggctgaccattctatggctcagacacctcggctcattgatggcattgttcttaccaaatttgataccattgatgacaaggtgggagctgctatttctatgacgtacatcacaagcaaacccatcgtctttgtgggcaccggccagacctactgtgacctacgcagcctcaatgccaaggctgtggtggctgccctcatgaaggcttaa

SEQ ID NO: 25 - protein, 638 aa, Homo sapiens
  MISC_FEATURE: hSRPRalpha
MLDFFTIFSKGGLVLWCFQGVSDSCTGPVNALIRSVLLQERGGNNSFTHEALTLKYKLDNQFELVFVVGFQKILTLTYVDKLIDDVHRLFRDKYRTEIQQQSALSLLNGTFDFQNDFLRLLREAEESSKIRAPTTMKKFEDSEKAKKPVRSMIETRGEKPKEKAKNSKKKGAKKEGSDGPLATSKPVPAEKSGLPVGPENGVELSKEELIRRKREEFIQKHGRGMEKSNKSTKSDAPKEKGKKAPRVWELGGCANKEVLDYSTPTTNGTPEAALSEDINLIRGTGSGGQLQDLDCSSSDDEGAAQNSTKPSATKGTLGGMFGMLKGLVGSKSLSREDMESVLDKMRDHLIAKNVAADIAVQLCESVANKLEGKVMGTFSTVTSTVKQALQESLVQILQPQRRVDMLRDIMDAQRRQRPYVVTFCGVNGVGKSTNLAKISFWLLENGFSVLIAACDTFRAGAVEQLRTHTRRLSALHPPEKHGGRTMVQLFEKGYGKDAAGIAMEAIAFARNQGFDVVLVDTAGRMQDNAPLMTALAKLITVNTPDLVLFVGEALVGNEAVDQLVKFNRALADHSMAQTPRLIDGIVLTKFDTIDDKVGAAISMTYITSKPIVFVGTGQTYCDLRSLNAKAVVAALMKA

SEQ ID NO: 26 - DNA, 816 bp, Homo sapiens
  misc_feature: hSRPRbeta
atggcttccgcggactcgcgccgggtggcagatggcggcggtgccgggggcaccttccagccctacctagacaccttgcggcaggagctgcagcagacggacccaacgctgttgtcagtagtggtggcggttcttgcggtgctgctgacgctagtcttctggaagttaatccggagcagaaggagcagtcagagagctgttcttcttgttggcctttgtgattccgggaaaacgttgctctttgtcaggttgttaacaggcctttatagagacactcagacgtccattactgacagctgtgctgtatacagagtcaacaataacaggggcaatagtctgaccttgattgaccttcccggccatgagagtttgaggcttcagttcttagagcggtttaagtcttcagccagggctattgtgtttgttgtggatagtgcagcattccagcgagaggtgaaagatgtggctgagtttctgtatcaagtcctcattgacagtatgggtctgaagaatacaccatcattcttaatagcctgcaataagcaagatattgcaatggcaaaatcagcaaagttaattcaacagcagctggagaaagaactcaacaccttacgagttacccgttctgctgcccccagcacactggacagttccagcactgcccctgctcagctggggaagaaaggcaaagagtttgaattctcacagttgcccctcaaagtggagttcctggagtgcagtgccaagggtggaagaggggacgtgggctctgctgacatccaggacttggagaaatggctggctaaaattgcctga

SEQ ID NO: 27 - protein, 271 aa, Homo sapiens
  MISC_FEATURE: hSRPRbeta
MASADSRRVADGGGAGGTFQPYLDTLRQELQQTDPTLLSVVVAVLAVLLTLVFWKLIRSRRSSQRAVLLVGLCDSGKTLLFVRLLTGLYRDTQTSITDSCAVYRVNNNRGNSLTLIDLPGHESLRLQFLERFKSSARAIVFVVDSAAFQREVKDVAEFLYQVLIDSMGLKNTPSFLIACNKQDIAMAKSAKLIQQQLEKELNTLRVTRSAAPSTLDSSSTAPAQLGKKGKEFEFSQLPLKVEFLECSAKGGRGDVGSADIQDLEKWLAKIA

SEQ ID NO: 28 - DNA, 1779 bp, Homo sapiens
  misc_feature: hCANX
atggaagggaagtggttgctgtgtatgttactggtgcttggaactgctattgttgaggctcatgatggacatgatgatgatgtgattgatattgaggatgaccttgacgatgtcattgaagaggtagaagactcaaaaccagataccactgctcctccttcatctcccaaggttacttacaaagctccagttccaacaggggaagtatattttgctgattcttttgacagaggaactctgtcagggtggattttatccaaagccaagaaagacgataccgatgatgaaattgccaaatatgatggaaagtgggaggtagaggaaatgaaggagtcaaagcttccaggtgataaaggacttgtgttgatgtctcgggccaagcatcatgccatctctgctaaactgaacaagcccttcctgtttgacaccaagcctctcattgttcagtatgaggttaatttccaaaatggaatagaatgtggtggtgcctatgtgaaactgctttctaaaacaccagaactcaacctggatcagttccatgacaagaccccttatacgattatgtttggtccagataaatgtggagaggactataaactgcacttcatcttccgacacaaaaaccccaaaacgggtatctatgaagaaaaacatgctaagaggccagatgcagatctgaagacctattttactgataagaaaacacatctttacacactaatcttgaatccagataatagttttgaaatactggttgaccaatctgtggtgaatagtggaaatctgctcaatgacatgactcctcctgtaaatccttcacgtgaaattgaggacccagaagaccggaagcccgaggattgggatgaaagaccaaaaatcccagatccagaagctgtcaagccagatgactgggatgaagatgcccctgctaagattccagatgaagaggccacaaaacccgaaggctggttagatgatgagcctgagtacgtacctgatccagacgcagagaaacctgaggattgggatgaagacatggatggagaatgggaggctcctcagattgccaaccctagatgtgagtcagctcctggatgtggtgtctggcagcgacctgtgattgacaaccccaattataaaggcaaatggaagcctcctatgattgacaatcccagttaccagggaatctggaaacccaggaaaataccaaatccagatttctttgaagatctggaacctttcagaatgactccttttagtgctattggtttggagctgtggtccatgacctctgacattttttttgacaactttatcatttgtgctgatcgaagaatagttgatgattgggccaatgatggatggggcctgaagaaagctgctgatggggctgctgagccaggcgttgtggggcagatgatcgaggcagctgaagagcgcccgtggctgtgggtagtctatattctaactgtagcccttcctgtgttcctggttatcctcttctgctgttctggaaagaaacagaccagtggtatggagtataagaaaactgatgcacctcaaccggatgtgaaggaagaggaagaagagaaggaagaggaaaaggacaagggagatgaggaggaggaaggagaagagaaacttgaagagaaacagaaaagtgatgctgaagaagatggtggcactgtcagtcaagaggaggaagacagaaaacctaaagcagaggaggatgaaattttgaacagatcaccaagaaacagaaagccacgaagagagtga

SEQ ID NO: 29 - protein, 592 aa, Homo sapiens
  MISC_FEATURE: hCANX
MEGKWLLCMLLVLGTAIVEAHDGHDDDVIDIEDDLDDVIEEVEDSKPDTTAPPSSPKVTYKAPVPTGEVYFADSFDRGTLSGWILSKAKKDDTDDEIAKYDGKWEVEEMKESKLPGDKGLVLMSRAKHHAISAKLNKPFLFDTKPLIVQYEVNFQNGIECGGAYVKLLSKTPELNLDQFHDKTPYTIMFGPDKCGEDYKLHFIFRHKNPKTGIYEEKHAKRPDADLKTYFTDKKTHLYTLILNPDNSFEILVDQSVVNSGNLLNDMTPPVNPSREIEDPEDRKPEDWDERPKIPDPEAVKPDDWDEDAPAKIPDEEATKPEGWLDDEPEYVPDPDAEKPEDWDEDMDGEWEAPQIANPRCESAPGCGVWQRPVIDNPNYKGKWKPPMIDNPSYQGIWKPRKIPNPDFFEDLEPFRMTPFSAIGLELWSMTSDIFFDNFIICADRRIVDDWANDGWGLKKAADGAAEPGVVGQMIEAAEERPWLWVVYILTVALPVFLVILFCCSGKKQTSGMEYKKTDAPQPDVKEEEEEKEEEKDKGDEEEEGEEKLEEKQKSDAEEDGGTVSQEEEDRKPKAEEDEILNRSPRNRKPRRE

SEQ ID NO: 30 - DNA, 972 bp, Homo sapiens
  misc_feature: hUCP4
atgtccgtcccggaggaggaggagaggcttttgccgctgacccagagatggccccgagcgagcaaattcctactgtccggctgcgcggctaccgtggccgagctagcaacctttcccctggatctcacaaaaactcgactccaaatgcaaggagaagcagctcttgctcggttgggagacggtgcaagagaatctgccccctataggggaatggtgcgcacagccctagggatcattgaagaggaaggctttctaaagctttggcaaggagtgacacccgccatttacagacacgtagtgtattctggaggtcgaatggtcacatatgaacatctccgagaggttgtgtttggcaaaagtgaagatgagcattatcccctttggaaatcagtcattggagggatgatggctggtgttattggccagtttttagccaatccaactgacctagtgaaggttcagatgcaaatggaaggaaaaaggaaactggaaggaaaaccattgcgatttcgtggtgtacatcatgcatttgcaaaaatcttagctgaaggaggaatacgagggctttgggcaggctgggtacccaatatacaaagagcagcactggtgaatatgggagatttaaccacttatgatacagtgaaacactacttggtattgaatacaccacttgaggacaatatcatgactcacggtttatcaagtttatgttctggactggtagcttctattctgggaacaccagccgatgtcatcaaaagcagaataatgaatcaaccacgagataaacaaggaaggggacttttgtataaatcatcgactgactgcttgattcaggctgttcaaggtgaaggattcatgagtctatataaaggctttttaccatcttggctgagaatgaccccttggtcaatggtgttctggcttacttatgaaaaaatcagagagatgagtggagtcagtccattttaa

SEQ ID NO: 31 - protein, 323 aa, Homo sapiens
  MISC_FEATURE: hUCP4
MSVPEEEERLLPLTQRWPRASKFLLSGCAATVAELATFPLDLTKTRLQMQGEAALARLGDGARESAPYRGMVRTALGIIEEEGFLKLWQGVTPAIYRHVVYSGGRMVTYEHLREVVFGKSEDEHYPLWKSVIGGMMAGVIGQFLANPTDLVKVQMQMEGKRKLEGKPLRFRGVHHAFAKILAEGGIRGLWAGWVPNIQRAALVNMGDLTTYDTVKHYLVLNTPLEDNIMTHGLSSLCSGLVASILGTPADVIKSRIMNQPRDKQGRGLLYKSSTDCLIQAVQGEGFMSLYKGFLPSWLRMTPWSMVFWLTYEKIREMSGVSPF

SEQ ID NO: 32 - DNA, 1014 bp, Homo sapiens
  misc_feature: hCMPSAT
atggctgccccgagagacaatgtcactttattattcaagttatactgcttggcagtgatgaccctgatggctgcagtctataccatagctttaagatacacaaggacatcagacaaagaactctacttttcaaccacagccgtgtgtatcacagaagttataaagttattgctaagtgtgggaattttagctaaagaaactggtagtctgggtagattcaaagcatctttaagagaaaatgtcttggggagccccaaggaactgttgaagttaagtgtgccatcgttagtgtatgctgttcagaacaacatggctttcctagctcttagcaatctggatgcagcagtgtaccaggtgacctaccagttgaagattccgtgtactgctttatgcactgttttaatgttaaaccggacactcagcaaattacagtgggtttcagtttttatgctgtgtgctggagttacgcttgtacagtggaaaccagcccaagctacaaaagtggtggtggaacaaaatccattattagggtttggcgctatagctattgctgtattgtgctcaggatttgcaggagtatattttgaaaaagttttaaagagttcagatacttctctttgggtgagaaacattcaaatgtatctatcagggattattgtgacattagctggcgtctacttgtcagatggagctgaaattaaagaaaaaggatttttctatggttacacatattatgtctggtttgtcatctttcttgcaagtgttggtggcctctacacttctgttgtggttaagtacacagacaacatcatgaaaggcttttctgcagcagcggccattgtcctttccaccattgcttcagtaatgctgtttggattacagataacactcacctttgccctgggtactcttcttgtatgtgtttccatatatctctatggattacccagacaagacactacatccatccaacaaggagaaacagcttcaaaggagagagttattggtgtgtga

SEQ ID NO: 33 - protein, 337 aa, Homo sapiens
  MISC_FEATURE: hCMPSAT
MAAPRDNVTLLFKLYCLAVMTLMAAVYTIALRYTRTSDKELYFSTTAVCITEVIKLLLSVGILAKETGSLGRFKASLRENVLGSPKELLKLSVPSLVYAVQNNMAFLALSNLDAAVYQVTYQLKIPCTALCTVLMLNRTLSKLQWVSVFMLCAGVTLVQWKPAQATKVVVEQNPLLGFGAIAIAVLCSGFAGVYFEKVLKSSDTSLWVRNIQMYLSGIIVTLAGVYLSDGAEIKEKGFFYGYTYYVWFVIFLASVGGLYTSVVVKYTDNIMKGFSAAAAIVLSTIASVMLFGLQITLTFALGTLLVCVSIYLYGLPRQDTTSIQQGETASKERVIGV

SEQ ID NO: 34 - DNA, 1212 bp, Artificial Sequence
  Optimized Sequence
  misc_feature: rST6Gal1
atgatccacaccaacctgaagaagaagttctccctgttcatcctggtgtttctgctgttcgccgtgatctgcgtgtggaagaagggctccgactacgaggctctgaccctgcaggccaaagaattccagatgcccaagtcccaagaaaaggtggcaatgggctccgccagccaggtggtgttctccaactccaagcaggaccctaaagaggacatccctatcctgtcctaccacagagtgaccgccaaagtgaagcctcagcctagcttccaggtctgggacaaggactccacctacagcaagctgaaccctcggctgctgaagatctggcggaactacctgaacatgaacaagtacaaggtgtcctacaagggccctggccctggcgtgaagttctccgtggaggccctgaggtgccacctgagggaccacgtgaacgtgtccatgatcgaggccaccgacttcccattcaacaccaccgagtgggagggctacctgcctaaagagaacttccggaccaaagtgggcccttggcagagatgcgccgtggtgtcctccgccggctccctgaagaactctcagctgggccgggagatcgacaaccacgacgccgtgctgaggttcaacggcgctcctaccgacaacttccagcaggacgtgggctccaagaccaccatcagactgatgaacagccagctggtgaccaccgagaagcggtttctgaaggactccctgtacaccgagggcatcctgatcgtgtgggacccttccgtgtaccacgccgacatccctaagtggtatcagaagcccgactacaacttcttcgagacatacaagtcctaccggcggctgaacccttcccagcctttctacatcctgaagccccagatgccttgggagctgtgggacatcatccaggaaatctccgccgacctgatccagcctaaccctccttcctccggcatgctgggcatcatcatcatgatgaccctgtgcgaccaggtggacatctacgagtttctgccttccaagagaaagaccgacgtgtgctactaccaccagaagttcttcgactccgcctgcacaatgggcgcctaccaccccctgctgttcgagaagaacatggtgaagcacctgaacgagggcaccgacgaggacatctacctgttcggcaaggccaccctgtccggcttccggaacatccggtgctga

SEQ ID NO: 35 - protein, 403 aa, Rattus norvegicus
  MISC_FEATURE: rST6Gal1
MIHTNLKKKFSLFILVFLLFAVICVWKKGSDYEALTLQAKEFQMPKSQEKVAMGSASQVVFSNSKQDPKEDIPILSYHRVTAKVKPQPSFQVWDKDSTYSKLNPRLLKIWRNYLNMNKYKVSYKGPGPGVKFSVEALRCHLRDHVNVSMIEATDFPFNTTEWEGYLPKENFRTKVGPWQRCAVVSSAGSLKNSQLGREIDNHDAVLRFNGAPTDNFQQDVGSKTTIRLMNSQLVTTEKRFLKDSLYTEGILIVWDPSVYHADIPKWYQKPDYNFFETYKSYRRLNPSQPFYILKPQMPWELWDIIQEISADLIQPNPPSSGMLGIIIMMTLCDQVDIYEFLPSKRKTDVCYYHQKFFDSACTMGAYHPLLFEKNMVKHLNEGTDEDIYLFGKATLSGFRNIRC

SEQ ID NO: 36 - DNA, 957 bp, Homo sapiens
  misc_feature: hCOMSC
atgctttctgaaagcagctcctttttgaagggtgtgatgcttggaagcattttctgtgctttgatcactatgctaggacacattaggattggtcatggaaatagaatgcaccaccatgagcatcatcacctacaagctcctaacaaagaagatatcttgaaaatttcagaggatgagcgcatggagctcagtaagagctttcgagtatactgtattatccttgtaaaacccaaagatgtgagtctttgggctgcagtaaaggagacttggaccaaacactgtgacaaagcagagttcttcagttctgaaaatgttaaagtgtttgagtcaattaatatggacacaaatgacatgtggttaatgatgagaaaagcttacaaatacgcctttgataagtatagagaccaatacaactggttcttccttgcacgccccactacgtttgctatcattgaaaacctaaagtattttttgttaaaaaaggatccatcacagcctttctatctaggccacactataaaatctggagaccttgaatatgtgggtatggaaggaggaattgtcttaagtgtagaatcaatgaaaagacttaacagccttctcaatatcccagaaaagtgtcctgaacagggagggatgatttggaagatatctgaagataaacagctagcagtttgcctgaaatatgctggagtatttgcagaaaatgcagaagatgctgatggaaaagatgtatttaataccaaatctgttgggctttctattaaagaggcaatgacttatcaccccaaccaggtagtagaaggctgttgttcagatatggctgttacttttaatggactgactccaaatcagatgcatgtgatgatgtatggggtataccgccttagggcatttgggcatattttcaatgatgcattggttttcttacctccaaatggttctgacaatgactga

SEQ ID NO: 37 - protein, 318 aa, Homo sapiens
  MISC_FEATURE: hCOMSC
MLSESSSFLKGVMLGSIFCALITMLGHIRIGHGNRMHHHEHHHLQAPNKEDILKISEDERMELSKSFRVYCIILVKPKDVSLWAAVKETWTKHCDKAEFFSSENVKVFESINMDTNDMWLMMRKAYKYAFDKYRDQYNWFFLARPTTFAIIENLKYFLLKKDPSQPFYLGHTIKSGDLEYVGMEGGIVLSVESMKRLNSLLNIPEKCPEQGGMIWKISEDKQLAVCLKYAGVFAENAEDADGKDVFNTKSVGLSIKEAMTYHPNQVVEGCCSDMAVTFNGLTPNQMHVMMYGVYRLRAFGHIFNDALVFLPPNGSDND

SEQ ID NO: 38 - DNA, 1092 bp, Homo sapiens
  misc_feature: hT-Synthase
atggcctctaaatcctggctgaattttttaaccttcctctgtggatcagcaataggatttcttttatgttctcagctatttagtattttgttgggagaaaaggttgacacccagcctaatgttcttcataatgatcctcatgcaaggcattcagatgataatggacagaatcatctagaaggacaaatgaacttcaatgcagattctagccaacataaagatgagaacacagacattgctgaaaacctctatcagaaagttagaattctttgctgggttatgaccggccctcaaaacctagagaaaaaggccaaacacgtcaaagctacttgggcccagcgttgtaacaaagtgttgtttatgagttcagaagaaaataaagacttccctgctgtgggactgaaaaccaaagaaggcagagatcaactatactggaaaacaattaaagcttttcagtatgttcatgaacattatttagaagatgctgattggtttttgaaagcagatgatgacacgtatgtcatactagacaatttgaggtggcttctttcaaaatacgaccctgaagaacccatttactttgggagaagatttaagccttatgtaaagcagggctacatgagtggaggagcaggatatgtactaagcaaagaagccttgaaaagatttgttgatgcatttaaaacagacaagtgtacacatagttcctccattgaagacttagcactggggagatgcatggaaattatgaatgtagaagcaggagattccagagataccattggaaaagaaacttttcatccctttgtgccagaacaccatttaattaaaggttatctacctagaacgttttggtactggaattacaactattatcctcctgtagagggtcctggttgctgctctgatcttgcagtttcttttcactatgttgattctacaaccatgtatgagttagaatacctcgtttatcatcttcgtccatatggttatttatacagatatcaacctaccttacctgaacgtatactaaaggaaattagtcaagcaaacaaaaatgaagatacaaaagtgaagttaggaaatccttga

SEQ ID NO: 39 - protein, 363 aa, Homo sapiens
  MISC_FEATURE: hT-Synthase
MASKSWLNFLTFLCGSAIGFLLCSQLFSILLGEKVDTQPNVLHNDPHARHSDDNGQNHLEGQMNFNADSSQHKDENTDIAENLYQKVRILCWVMTGPQNLEKKAKHVKATWAQRCNKVLFMSSEENKDFPAVGLKTKEGRDQLYWKTIKAFQYVHEHYLEDADWFLKADDDTYVILDNLRWLLSKYDPEEPIYFGRRFKPYVKQGYMSGGAGYVLSKEALKRFVDAFKTDKCTHSSSIEDLALGRCMEIMNVEAGDSRDTIGKETFHPFVPEHHLIKGYLPRTFWYWNYNYYPPVEGPGCCSDLAVSFHYVDSTTMYELEYLVYHLRPYGYLYRYQPTLPERILKEISQANKNEDTKVKLGNP

SEQ ID NO: 40 - DNA, 1605 bp, Homo sapiens
  misc_feature: hP4HA1
atgatctggtatatattaattataggaattctgcttccccagtctttggctcatccaggcttttttacttcaattggtcagatgactgatttgatccatactgagaaagatctggtgacttctctgaaagattatattaaggcagaagaggacaagttagaacaaataaaaaaatgggcagagaagttagatcggctaactagtacagcgacaaaagatccagaaggatttgttgggcatccagtaaatgcattcaaattaatgaaacgtctgaatactgagtggagtgagttggagaatctggtccttaaggatatgtcagatggctttatctctaacctaaccattcagagacagtactttcctaatgatgaagatcaggttggggcagccaaagctctgttacgtctccaggatacctacaatttggatacagataccatctcaaagggtaatcttccaggagtgaaacacaaatcttttctaacggctgaggactgctttgagttgggcaaagtggcctatacagaagcagattattaccatacggaactgtggatggaacaagccctaaggcaactggatgaaggcgagatttctaccatagataaagtctctgttctagattatttgagctatgcggtatatcagcagggagacctggataaggcacttttgctcacaaagaagcttcttgaactagatcctgaacatcagagagctaatggtaacttaaaatattttgagtatataatggctaaagaaaaagatgtcaataagtctgcttcagatgaccaatctgatcagaaaactacaccaaagaaaaaaggggttgctgtggattacctgccagagagacagaagtacgaaatgctgtgccgtggggagggtatcaaaatgacccctcggagacagaaaaaactcttttgccgctaccatgatggaaaccgtaatcctaaatttattctggctccagctaaacaggaggatgaatgggacaagcctcgtattattcgcttccatgatattatttctgatgcagaaattgaaatcgtcaaagacctagcaaaaccaaggctgagccgagctacagtacatgaccctgagactggaaaattgaccacagcacagtacagagtatctaagagtgcctggctctctggctatgaaaatcctgtggtgtctcgaattaatatgagaatacaagatctaacaggactagatgtttccacagcagaggaattacaggtagcaaattatggagttggaggacagtatgaaccccattttgactttgcacggaaagatgagccagatgctttcaaagagctggggacaggaaatagaattgctacatggctgttttatatgagtgatgtgtctgcaggaggagccactgtttttcctgaagttggagctagtgtttggcccaaaaaaggaactgctgttttctggtataatctgtttgccagtggagaaggagattatagtacacggcatgcagcctgtccagtgctagttggcaacaaatgggtatccaataaatggctccatgaacgtggacaagaatttcgaagaccttgtacgttgtcagaattggaatga

SEQ ID NO: 41 - protein, 534 aa, Homo sapiens
  MISC_FEATURE: hP4HA1
MIWYILIIGILLPQSLAHPGFFTSIGQMTDLIHTEKDLVTSLKDYIKAEEDKLEQIKKWAEKLDRLTSTATKDPEGFVGHPVNAFKLMKRLNTEWSELENLVLKDMSDGFISNLTIQRQYFPNDEDQVGAAKALLRLQDTYNLDTDTISKGNLPGVKHKSFLTAEDCFELGKVAYTEADYYHTELWMEQALRQLDEGEISTIDKVSVLDYLSYAVYQQGDLDKALLLTKKLLELDPEHQRANGNLKYFEYIMAKEKDVNKSASDDQSDQKTTPKKKGVAVDYLPERQKYEMLCRGEGIKMTPRRQKKLFCRYHDGNRNPKFILAPAKQEDEWDKPRIIRFHDIISDAEIEIVKDLAKPRLSRATVHDPETGKLTTAQYRVSKSAWLSGYENPVVSRINMRIQDLTGLDVSTAEELQVANYGVGGQYEPHFDFARKDEPDAFKELGTGNRIATWLFYMSDVSAGGATVFPEVGASVWPKKGTAVFWYNLFASGEGDYSTRHAACPVLVGNKWVSNKWLHERGQEFRRPCTLSELE

SEQ ID NO: 42 - DNA, 1527 bp, Homo sapiens
  misc_feature: hP4HB
atgctgcgccgcgctctgctgtgcctggccgtggccgccctggtgcgcgccgacgcccccgaggaggaggaccacgtcctggtgctgcggaaaagcaacttcgcggaggcgctggcggcccacaagtacctgctggtggagttctatgccccttggtgtggccactgcaaggctctggcccctgagtatgccaaagccgctgggaagctgaaggcagaaggttccgagatcaggttggccaaggtggacgccacggaggagtctgacctggcccagcagtacggcgtgcgcggctatcccaccatcaagttcttcaggaatggagacacggcttcccccaaggaatatacagctggcagagaggctgatgacatcgtgaactggctgaagaagcgcacgggcccggctgccaccaccctgcctgacggcgcagctgcagagtccttggtggagtccagcgaggtggctgtcatcggcttcttcaaggacgtggagtcggactctgccaagcagtttttgcaggcagcagaggccatcgatgacataccatttgggatcacttccaacagtgacgtgttctccaaataccagctcgacaaagatggggttgtcctctttaagaagtttgatgaaggccggaacaactttgaaggggaggtcaccaaggagaacctgctggactttatcaaacacaaccagctgccccttgtcatcgagttcaccgagcagacagccccgaagatttttggaggtgaaatcaagactcacatcctgctgttcttgcccaagagtgtgtctgactatgacggcaaactgagcaacttcaaaacagcagccgagagcttcaagggcaagatcctgttcatcttcatcgacagcgaccacaccgacaaccagcgcatcctcgagttctttggcctgaagaaggaagagtgcccggccgtgcgcctcatcaccctggaggaggagatgaccaagtacaagcccgaatcggaggagctgacggcagagaggatcacagagttctgccaccgcttcctggagggcaaaatcaagccccacctgatgagccaggagctgccggaggactgggacaagcagcctgtcaaggtgcttgttgggaagaactttgaagacgtggcttttgatgagaaaaaaaacgtctttgtggagttctatgccccatggtgtggtcactgcaaacagttggctcccatttgggataaactgggagagacgtacaaggaccatgagaacatcgtcatcgccaagatggactcgactgccaacgaggtggaggccgtcaaagtgcacagcttccccacactcaagttctttcctgccagtgccgacaggacggtcattgattacaacggggaacgcacgctggatggttttaagaaattcctggagagcggtggccaggatggggcaggggatgatgacgatctcgaggacctggaagaagcagaggagccagacatggaggaagacgatgatcagaaagctgtgaaagatgaactgtaa

SEQ ID NO: 43 - protein, 508 aa, Homo sapiens
  MISC_FEATURE: hP4HB
MLRRALLCLAVAALVRADAPEEEDHVLVLRKSNFAEALAAHKYLLVEFYAPWCGHCKALAPEYAKAAGKLKAEGSEIRLAKVDATEESDLAQQYGVRGYPTIKFFRNGDTASPKEYTAGREADDIVNWLKKRTGPAATTLPDGAAAESLVESSEVAVIGFFKDVESDSAKQFLQAAEAIDDIPFGITSNSDVFSKYQLDKDGVVLFKKFDEGRNNFEGEVTKENLLDFIKHNQLPLVIEFTEQTAPKIFGGEIKTHILLFLPKSVSDYDGKLSNFKTAAESFKGKILFIFIDSDHTDNQRILEFFGLKKEECPAVRLITLEEEMTKYKPESEELTAERITEFCHRFLEGKIKPHLMSQELPEDWDKQPVKVLVGKNFEDVAFDEKKNVFVEFYAPWCGHCKQLAPIWDKLGETYKDHENIVIAKMDSTANEVEAVKVHSFPTLKFFPASADRTVIDYNGERTLDGFKKFLESGGQDGAGDDDDLEDLEEAEEPDMEEDDDQKAVKDEL

SEQ ID NO: 44 - DNA, 603 bp, Homo sapiens
  misc_feature: hGILZ
atggcccagtccaagctcgattgccgctcacctgtcggcctcgactgctgcaactgctgcctggacctggcccatcggagtgggctccagcgaggcagcagcggggagaacaacaacccgggcagccctacagtgagcaactttcggcagctgcaggaaaagctggtctttgagaacctcaataccgacaagctcaacagcataatgcggcaggattcgctagagccggtgctgcgggacccctgctacctgatcaacgagggcatctgcaaccgcaacatcgaccagaccatgctctccatcctgctcttcttccacagtgcctccggagccagcgtggtggccatagacaacaagatcgaacaggccatggatctggtgaagaatcatctgatgtatgctgtgagagaggaggtggagatcctgaaggagcagatccgagagctggtggagaagaactcccagctagagcgtgagaacaccctgttgaagaccctggcaagcccagagcagctggagaagttccagtcctgtctgagccctgaagagccagctcccgaatccccacaagtgcccgaggcccctggtggttctgcggtgtaa

SEQ ID NO: 45 - protein, 200 aa, Homo sapiens
  MISC_FEATURE: hGILZ
MAQSKLDCRSPVGLDCCNCCLDLAHRSGLQRGSSGENNNPGSPTVSNFRQLQEKLVFENLNTDKLNSIMRQDSLEPVLRDPCYLINEGICNRNIDQTMLSILLFFHSASGASVVAIDNKIEQAMDLVKNHLMYAVREEVEILKEQIRELVEKNSQLERENTLLKTLASPEQLEKFQSCLSPEEPAPESPQVPEAPGGSAV

SEQ ID NO: 46 - DNA, 651 bp, Homo sapiens
  misc_feature: hCyPB
atgctgcgcctctccgaacgcaacatgaaggtgctccttgccgccgccctcatcgcggggtccgtcttcttcctgctgctgccgggaccttctgcggccgatgagaagaagaaggggcccaaagtcaccgtcaaggtgtattttgacctacgaattggagatgaagatgtaggccgggtgatctttggtctcttcggaaagactgttccaaaaacagtggataattttgtggccttagctacaggagagaaaggatttggctacaaaaacagcaaattccatcgtgtaatcaaggacttcatgatccagggcggagacttcaccaggggagatggcacaggaggaaagagcatctacggtgagcgcttccccgatgagaacttcaaactgaagcactacgggcctggctgggtgagcatggccaacgcaggcaaagacaccaacggctcccagttcttcatcacgacagtcaagacagcctggctagatggcaagcatgtggtgtttggcaaagttctagagggcatggaggtggtgcggaaggtggagagcaccaagacagacagccgggataaacccctgaaggatgtgatcatcgcagactgcggcaagatcgaggtggagaagccctttgccatcgccaaggagtag

SEQ ID NO: 47 - protein, 216 aa, Homo sapiens
  MISC_FEATURE: hCyPB
MLRLSERNMKVLLAAALIAGSVFFLLLPGPSAADEKKKGPKVTVKVYFDLRIGDEDVGRVIFGLFGKTVPKTVDNFVALATGEKGFGYKNSKFHRVIKDFMIQGGDFTRGDGTGGKSIYGERFPDENFKLKHYGPGWVSMANAGKDTNGSQFFITTVKTAWLDGKHVVFGKVLEGMEVVRKVESTKTDSRDKPLKDVIIADCGKIEVEKPFAIAKE

SEQ ID NO: 48 - DNA, 1818 bp, Homo sapiens
  misc_feature: hNRF2
atgatggacttggagctgccgccgccgggactcccgtcccagcaggacatggatttgattgacatactttggaggcaagatatagatcttggagtaagtcgagaagtatttgacttcagtcagcgacggaaagagtatgagctggaaaaacagaaaaaacttgaaaaggaaagacaagaacaactccaaaaggagcaagagaaagcctttttcgctcagttacaactagatgaagagacaggtgaatttctcccaattcagccagcccagcacatccagtcagaaaccagtggatctgccaactactcccaggttgcccacattcccaaatcagatgctttgtactttgatgactgcatgcagcttttggcgcagacattcccgtttgtagatgacaatgaggtttcttcggctacgtttcagtcacttgttcctgatattcccggtcacatcgagagcccagtcttcattgctactaatcaggctcagtcacctgaaacttctgttgctcaggtagcccctgttgatttagacggtatgcaacaggacattgagcaagtttgggaggagctattatccattcctgagttacagtgtcttaatattgaaaatgacaagctggttgagactaccatggttccaagtccagaagccaaactgacagaagttgacaattatcatttttactcatctataccctcaatggaaaaagaagtaggtaactgtagtccacattttcttaatgcttttgaggattccttcagcagcatcctctccacagaagaccccaaccagttgacagtgaactcattaaattcagatgccacagtcaacacagattttggtgatgaattttattctgctttcatagctgagcccagtatcagcaacagcatgccctcacctgctactttaagccattcactctctgaacttctaaatgggcccattgatgtttctgatctatcactttgcaaagctttcaaccaaaaccaccctgaaagcacagcagaattcaatgattctgactccggcatttcactaaacacaagtcccagtgtggcatcaccagaacactcagtggaatcttccagctatggagacacactacttggcctcagtgattctgaagtggaagagctagatagtgcccctggaagtgtcaaacagaatggtcctaaaacaccagtacattcttctggggatatggtacaacccttgtcaccatctcaggggcagagcactcacgtgcatgatgcccaatgtgagaacacaccagagaaagaattgcctgtaagtcctggtcatcggaaaaccccattcacaaaagacaaacattcaagccgcttggaggctcatctcacaagagatgaacttagggcaaaagctctccatatcccattccctgtagaaaaaatcattaacctccctgttgttgacttcaacgaaatgatgtccaaagagcagttcaatgaagctcaacttgcattaattcgggatatacgtaggaggggtaagaataaagtggctgctcagaattgcagaaaaagaaaactggaaaatatagtagaactagagcaagatttagatcatttgaaagatgaaaaagaaaaattgctcaaagaaaaaggagaaaatgacaaaagccttcacctactgaaaaaacaactcagcaccttatatctcgaagttttcagcatgctacgtgatgaagatggaaaaccttattctcctagtgaatactccctgcagcaaacaagagatggcaatgttttccttgttcccaaaagtaagaagccagatgttaagaaaaactag

SEQ ID NO: 49 - protein, 605 aa, Homo sapiens
  MISC_FEATURE: hNRF2
MMDLELPPPGLPSQQDMDLIDILWRQDIDLGVSREVFDFSQRRKEYELEKQKKLEKERQEQLQKEQEKAFFAQLQLDEETGEFLPIQPAQHIQSETSGSANYSQVAHIPKSDALYFDDCMQLLAQTFPFVDDNEVSSATFQSLVPDIPGHIESPVFIATNQAQSPETSVAQVAPVDLDGMQQDIEQVWEELLSIPELQCLNIENDKLVETTMVPSPEAKLTEVDNYHFYSSIPSMEKEVGNCSPHFLNAFEDSFSSILSTEDPNQLTVNSLNSDATVNTDFGDEFYSAFIAEPSISNSMPSPATLSHSLSELLNGPIDVSDLSLCKAFNQNHPESTAEFNDSDSGISLNTSPSVASPEHSVESSSYGDTLLGLSDSEVEELDSAPGSVKQNGPKTPVHSSGDMVQPLSPSQGQSTHVHDAQCENTPEKELPVSPGHRKTPFTKDKHSSRLEAHLTRDELRAKALHIPFPVEKIINLPVVDFNEMMSKEQFNEAQLALIRDIRRRGKNKVAAQNCRKRKLENIVELEQDLDHLKDEKEKLLKEKGENDKSLHLLKKQLSTLYLEVFSMLRDEDGKPYSPSEYSLQQTRDGNVFLVPKSKKPDVKKN

SEQ ID NO: 50 - DNA, 2754 bp, Homo sapiens
  misc_feature: hHK1
atgatcgccgcgcagctcctggcctattacttcacggagctgaaggatgaccaggtcaaaaagattgacaagtatctctatgccatgcggctctccgatgaaactctcatagatatcatgactcgcttcaggaaggagatgaagaatggcctctcccgggattttaatccaacagccacagtcaagatgttgccaacattcgtaaggtccattcctgatggctctgaaaagggagatttcattgccctggatcttggtgggtcttcctttcgaattctgcgggtgcaagtgaatcatgagaaaaaccagaatgttcacatggagtccgaggtttatgacaccccagagaacatcgtgcacggcagtggaagccagctttttgatcatgttgctgagtgcctgggagatttcatggagaaaaggaagatcaaggacaagaagttacctgtgggattcacgttttcttttccttgccaacaatccaaaatagatgaggccatcctgatcacctggacaaagcgatttaaagcgagcggagtggaaggagcagatgtggtcaaactgcttaacaaagccatcaaaaagcgaggggactatgatgccaacatcgtagctgtggtgaatgacacagtgggcaccatgatgacctgtggctatgacgaccagcactgtgaagtcggcctgatcatcggcactggcaccaatgcttgctacatggaggaactgaggcacattgatctggtggaaggagacgaggggaggatgtgtatcaatacagaatggggagcctttggagacgatggatcattagaagacatccggacagagtttgacagggagatagaccggggatccctcaaccctggaaaacagctgtttgagaagatggtcagtggcatgtacttgggagagctggttcgactgatcctagtcaagatggccaaggagggcctcttatttgaagggcggatcaccccggagctgctcacccgagggaagtttaacaccagtgatgtgtcagccatcgaaaagaataaggaaggcctccacaatgccaaagaaatcctgacccgcctgggagtggagccgtccgatgatgactgtgtctcagtccagcacgtttgcaccattgtctcatttcgctcagccaacttggtggctgccacactgggcgccatcttgaaccgcctgcgtgataacaagggcacacccaggctgcggaccacggttggtgtcgacggatctctttacaagacgcacccacagtattcccggcgtttccacaagactctaaggcgcttggtgccagactccgatgtgcgcttcctcctctcggagagtggcagcggcaagggggctgccatggtgacggcggtggcctaccgcttggccgagcagcaccggcagatagaggagaccctggctcatttccacctcaccaaggacatgctgctggaggtgaagaagaggatgcgggccgagatggagctggggctgaggaagcagacgcacaacaatgccgtggttaagatgctgccctccttcgtccggagaactcccgacgggaccgagaatggtgacttcttggccctggatcttggaggaaccaatttccgtgtgctgctggtgaaaatccgtagtgggaaaaagagaacggtggaaatgcacaacaagatctacgccattcctattgaaatcatgcagggcactggggaagagctgtttgatcacattgtctcctgcatctctgacttcttggactacatggggatcaaaggccccaggatgcctctgggcttcacgttctcatttccctgccagcagacgagtctggacgcgggaatcttgatcacgtggacaaagggttttaaggcaacagactgcgtgggccacgatgtagtcaccttactaagggatgcgataaaaaggagagaggaatttgacctggacgtggtggctgtggtcaacgacacagtgggcaccatgatgacctgtgcttatgaggagcccacctgtgaggttggactcattgttgggaccggcagcaatgcctgctacatggaggagatgaagaacgtggagatggtggagggggaccaggggcagatgtgcatcaacatggagtggggggcctttggggacaacgggtgtctggatgatatcaggacacactacgacagactggtggacgaatattccctaaatgctgggaaacaaaggtatgagaagatgatcagtggtatgtacctgggtgaaatcgtccgcaacatcttaatcgacttcaccaagaagggattcctcttccgagggcagatctctgagacgctgaagacccggggcatctttgagaccaagtttctctctcagatcgagagtgaccgattagcactgctccaggtccgggctatcctccagcagctaggtctgaatagcacctgcgatgacagtatcctcgtcaagacagtgtgcggggtggtgtccaggagggccgcacagctgtgtggcgcaggcatggctgcggttgtggataagatccgcgagaacagaggactggaccgtctgaatgtgactgtgggagtggacgggacactctacaagcttcatccacacttctccagaatcatgcaccagacggtgaaggaactgtcaccaaaatgtaacgtgtccttcctcctgtctgaggatggcagcggcaagggggccgccctcatcacggccgtgggcgtgcggttacgcacagaggcaagcagctaa

SEQ ID NO: 51 - protein, 917 aa, Homo sapiens
  MISC_FEATURE: hHK1
MIAAQLLAYYFTELKDDQVKKIDKYLYAMRLSDETLIDIMTRFRKEMKNGLSRDFNPTATVKMLPTFVRSIPDGSEKGDFIALDLGGSSFRILRVQVNHEKNQNVHMESEVYDTPENIVHGSGSQLFDHVAECLGDFMEKRKIKDKKLPVGFTFSFPCQQSKIDEAILITWTKRFKASGVEGADVVKLLNKAIKKRGDYDANIVAVVNDTVGTMMTCGYDDQHCEVGLIIGTGTNACYMEELRHIDLVEGDEGRMCINTEWGAFGDDGSLEDIRTEFDREIDRGSLNPGKQLFEKMVSGMYLGELVRLILVKMAKEGLLFEGRITPELLTRGKFNTSDVSAIEKNKEGLHNAKEILTRLGVEPSDDDCVSVQHVCTIVSFRSANLVAATLGAILNRLRDNKGTPRLRTTVGVDGSLYKTHPQYSRRFHKTLRRLVPDSDVRFLLSESGSGKGAAMVTAVAYRLAEQHRQIEETLAHFHLTKDMLLEVKKRMRAEMELGLRKQTHNNAVVKMLPSFVRRTPDGTENGDFLALDLGGTNFRVLLVKIRSGKKRTVEMHNKIYAIPIEIMQGTGEELFDHIVSCISDFLDYMGIKGPRMPLGFTFSFPCQQTSLDAGILITWTKGFKATDCVGHDVVTLLRDAIKRREEFDLDVVAVVNDTVGTMMTCAYEEPTCEVGLIVGTGSNACYMEEMKNVEMVEGDQGQMCINMEWGAFGDNGCLDDIRTHYDRLVDEYSLNAGKQRYEKMISGMYLGEIVRNILIDFTKKGFLFRGQISETLKTRGIFETKFLSQIESDRLALLQVRAILQQLGLNSTCDDSILVKTVCGVVSRRAAQLCGAGMAAVVDKIRENRGLDRLNVTVGVDGTLYKLHPHFSRIMHQTVKELSPKCNVSFLLSEDGSGKGAALITAVGVRLRTEASS

SEQ ID NO: 52 - DNA, 1578 bp, Homo sapiens
  misc_feature: hPDI
atgagccgccagcttctgcctgtactgctgctgctgctgctcagggcttcgtgcccatggggtcaggaacagggagcgaggagcccctcggaggagcctccagaggaggaaatccccaaggaggatgggatcttggtgctgagccgccacaccctgggcctggccctgcgggagcaccctgccctgctggtggaattctatgccccgtggtgtgggcactgccaggccctggcccccgagtacagcaaggcagctgccgtgctcgcggccgagtcaatggtggtcacgctggccaaggtggatgggcccgcgcagcgcgagctggctgaggagtttggtgtgacggagtaccctacgctcaagttcttccgcaatgggaaccgcacgcacccggaggagtacacaggaccacgggacgctgagggcattgccgagtggctgcgacggcgggtggggcccagtgccatgcggctggaggacgaggcggccgcccaggcgctgatcggtggccgggacctagtggtcattggcttcttccaggacctgcaggacgaggacgtggccaccttcttggccttggcccaggacgccctggacatgacctttggcctcacagaccggccgcggctctttcagcagtttggcctcaccaaggacactgtggttctcttcaagaagtttgatgaggggcgggcagacttccccgtggacgaggagcttggcctggacctgggggatctgtcgcgcttcctggtcacacacagcatgcgcctggtcacggagttcaacagccagacgtctgccaagatcttcgcggccaggatcctcaaccacctgctgctgtttgtcaaccagacgctggctgcgcaccgggagctcctagcgggctttggggaggcagctccccgcttccgggggcaggtgctgttcgtggtggtggacgtggcggccgacaatgagcacgtgctgcagtactttggactcaaggctgaggcagcccccactctgcgcttggtcaaccttgaaaccactaagaagtatgcgcctgtggatgggggccctgtcaccgcagcgtccatcactgctttctgccatgcagtcctcaacggccaagtcaagccctatctcctgagccaggagataccccctgattgggatcagcggccagttaagaccctcgtgggcaagaattttgagcaggtggcttttgacgaaaccaagaatgtgtttgtcaagttctatgccccgtggtgcacccactgcaaggagatggcccctgcctgggaggcattggctgagaagtaccaagaccacgaggacatcatcattgctgagctggatgccacggccaacgagctggatgccttcgctgtgcacggcttccctactctcaagtacttcccagcagggccaggtcggaaggtgattgaatacaaaagcaccagggacctggagactttctccaagttcctggacaacgggggcgtgctgcccacggaggagcccccggaggagccagcagccccgttcccggagccaccggccaactccactatggggtccaaggaggaactgtag

SEQ ID NO: 53 - protein, 525 aa, Homo sapiens
  MISC_FEATURE: hPDI
MSRQLLPVLLLLLLRASCPWGQEQGARSPSEEPPEEEIPKEDGILVLSRHTLGLALREHPALLVEFYAPWCGHCQALAPEYSKAAAVLAAESMVVTLAKVDGPAQRELAEEFGVTEYPTLKFFRNGNRTHPEEYTGPRDAEGIAEWLRRRVGPSAMRLEDEAAAQALIGGRDLVVIGFFQDLQDEDVATFLALAQDALDMTFGLTDRPRLFQQFGLTKDTVVLFKKFDEGRADFPVDEELGLDLGDLSRFLVTHSMRLVTEFNSQTSAKIFAARILNHLLLFVNQTLAAHRELLAGFGEAAPRFRGQVLFVVVDVAADNEHVLQYFGLKAEAAPTLRLVNLETTKKYAPVDGGPVTAASITAFCHAVLNGQVKPYLLSQEIPPDWDQRPVKTLVGKNFEQVAFDETKNVFVKFYAPWCTHCKEMAPAWEALAEKYQDHEDIIIAELDATANELDAFAVHGFPTLKYFPAGPGRKVIEYKSTRDLETFSKFLDNGGVLPTEEPPEEPAAPFPEPPANSTMGSKEEL

SEQ ID NO: 54 - DNA, 492 bp, Homo sapiens
  misc_feature: hPIN1
atggcggacgaggagaagctgccgcccggctgggagaagcgcatgagccgcagctcaggccgagtgtactacttcaaccacatcactaacgccagccagtgggagcggcccagcggcaacagcagcagtggtggcaaaaacgggcagggggagcctgccagggtccgctgctcgcacctgctggtgaagcacagccagtcacggcggccctcgtcctggcggcaggagaagatcacccggaccaaggaggaggccctggagctgatcaacggctacatccagaagatcaagtcgggagaggaggactttgagtctctggcctcacagttcagcgactgcagctcagccaaggccaggggagacctgggtgccttcagcagaggtcagatgcagaagccatttgaagacgcctcgtttgcgctgcggacgggggagatgagcgggcccgtgttcacggattccggcatccacatcatcctccgcactgagtga

SEQ ID NO: 55 - protein, 163 aa, Homo sapiens
  MISC_FEATURE: hPIN1
MADEEKLPPGWEKRMSRSSGRVYYFNHITNASQWERPSGNSSSGGKNGQGEPARVRCSHLLVKHSQSRRPSSWRQEKITRTKEEALELINGYIQKIKSGEEDFESLASQFSDCSSAKARGDLGAFSRGQMQKPFEDASFALRTGEMSGPVFTDSGIHIILRTE

SEQ ID NO: 56 - DNA, 264 bp, Homo sapiens
  misc_feature: hSEPW1
atggctctcgccgtccgagtcgtttattgtggcgcttgaggctacaagtccaagtatcttcagctcaagaagaagttagaagatgagttccccggccgcctggacatctgcggcgagggaactccccaggccaccgggttctttgaagtgatggtagccgggaagttgattcactctaagaagaaaggcgatggctacgtggacacagaaagcaagtttctgaagttggtggccgccatcaaagccgccttggctcagggctaa

SEQ ID NO: 57 - protein, 87 aa, Homo sapiens
  MISC_FEATURE: hSEPW1
  MISC_FEATURE (13)..(13): Special amino acid selenocysteine (U)
MALAVRVVYCGAXGYKSKYLQLKKKLEDEFPGRLDICGEGTPQATGFFEVMVAGKLIHSKKKGDGYVDTESKFLKLVAAIKAALAQG

SEQ ID NO: 58 - DNA, 1254 bp, Homo sapiens
  misc_feature: hCALR
atgctgctatccgtgccgctgctgctcggcctcctcggcctggccgtcgccgagcctgccgtctacttcaaggagcagtttctggacggagacgggtggacttcccgctggatcgaatccaaacacaagtcagattttggcaaattcgttctcagttccggcaagttctacggtgacgaggagaaagataaaggtttgcagacaagccaggatgcacgcttttatgctctgtcggccagtttcgagcctttcagcaacaaaggccagacgctggtggtgcagttcacggtgaaacatgagcagaacatcgactgtgggggcggctatgtgaagctgtttcctaatagtttggaccagacagacatgcacggagactcagaatacaacatcatgtttggtcccgacatctgtggccctggcaccaagaaggttcatgtcatcttcaactacaagggcaagaacgtgctgatcaacaaggacatccgttgcaaggatgatgagtttacacacctgtacacactgattgtgcggccagacaacacctatgaggtgaagattgacaacagccaggtggagtccggctccttggaagacgattgggacttcctgccacccaagaagataaaggatcctgatgcttcaaaaccggaagactgggatgagcgggccaagatcgatgatcccacagactccaagcctgaggactgggacaagcccgagcatatccctgaccctgatgctaagaagcccgaggactgggatgaagagatggacggagagtgggaacccccagtgattcagaaccctgagtacaagggtgagtggaagccccggcagatcgacaacccagattacaagggcacttggatccacccagaaattgacaaccccgagtattctcccgatcccagtatctatgcctatgataactttggcgtgctgggcctggacctctggcaggtcaagtctggcaccatctttgacaacttcctcatcaccaacgatgaggcatacgctgaggagtttggcaacgagacgtggggcgtaacaaaggcagcagagaaacaaatgaaggacaaacaggacgaggagcagaggcttaaggaggaggaagaagacaagaaacgcaaagaggaggaggaggcagaggacaaggaggatgatgaggacaaagatgaggatgaggaggatgaggaggacaaggaggaagatgaggaggaagatgtccccggccaggccaaggacgagctgtag

SEQ ID NO: 59 - protein, 417 aa, Homo sapiens
  MISC_FEATURE: hCALR
MLLSVPLLLGLLGLAVAEPAVYFKEQFLDGDGWTSRWIESKHKSDFGKFVLSSGKFYGDEEKDKGLQTSQDARFYALSASFEPFSNKGQTLVVQFTVKHEQNIDCGGGYVKLFPNSLDQTDMHGDSEYNIMFGPDICGPGTKKVHVIFNYKGKNVLINKDIRCKDDEFTHLYTLIVRPDNTYEVKIDNSQVESGSLEDDWDFLPPKKIKDPDASKPEDWDERAKIDDPTDSKPEDWDKPEHIPDPDAKKPEDWDEEMDGEWEPPVIQNPEYKGEWKPRQIDNPDYKGTWIHPEIDNPEYSPDPSIYAYDNFGVLGLDLWQVKSGTIFDNFLITNDEAYAEEFGNETWGVTKAAEKQMKDKQDEEQRLKEEEEDKKRKEEEEAEDKEDDEDKDEDEEDEEDKEEDEEEDVPGQAKDEL

SEQ ID NO: 60 - protein, 656 aa, Homo sapiens
  MISC_FEATURE: DroBiP
MKFPMVAAALLLLCAVRAEEKKEKDKELGTVIGIDLGTTYSCVGVYKNGRVEIIANDQGNRITPSYVAFTADGERLIGDAAKNQLTTNPENTVFDAKRLIGREWSDTNVQHDIKFFPFKVVEKNSKPHISVDTSQGAKVFAPEEISAMVLGKMKETAEAYLGKKVTHAVVTVPAYFNDAQRQATKDAGVIAGLQVMRIINEPTAAAIAYGLDKKEGEKNVLVFDLGGGTFDVSLLTIDNGVFEVVATNGDTHLGGEDFDQRVMDHFIKLYKKKKGKDIRKDNRAVQKLRREVEKAKRALSGSHQVRIEIESFFEGDDFSETLTRAKFEELNLDLFRSTLKPVQKVLEDADMNKKDVHEIVLVGGSTRIPKVQQLVKDFFGGKEPSRGINPDEAVAYGAAVQAGVLSGEQDTDAIVLLDVNPLTMGIETVGGVMTKLIPRNTVIPTKKSQVFSTASDNQHTVTIQVYEGERPMTKDNHLLGKFDLTGIPPAPRGIPQIEVSFEIDANGILQVSAEDKGTGNKEKIVITNDQNRLTPEDIDRMIRDAEKFADEDKKLKERVESRNELESYAYSLKNQIGDKDKLGAKLSDDEKNKLESAIDESIKWLEQNPDADPEEYKKQKKDLEAIVQPVIAKLYQGAGGAPPPEGGDDADLKDEL

SEQ ID NO: 61 - DNA, 1371 bp, Homo sapiens
  misc_feature: hDDOST
atggggtacttccggtgtgcaggtgctgggtccttcggcaggaggaggaagatggagcccagcaccgcggcccgggcttgggccctcttttggttgctgctgcccttgcttggcgcggtttgcgccagcggaccccgcaccttagtgctgctggacaacctcaacgtgcgggagactcattcgcttttcttccggagcctgaaggaccggggctttgagctcacattcaagaccgctgatgaccccagcctgtctctcataaagtatggggaattcctctatgacaatctcatcattttctccccttcggtagaagattttggaggcaacatcaacgtggagaccatcagtgcctttattgacggcggaggcagtgtgctggtagctgccagctccgacattggtgaccctcttcgagagctgggcagtgagtgcgggattgagtttgacgaggagaaaacggctgtcattgaccatcacaactatgacatctcagaccttggccagcatacgctcatcgtggctgacactgagaacctgctgaaggccccaaccatcgttgggaaatcatctctaaatcccatcctctttcgaggtgttgggatggtggccgatcctgataaccctttggtgctggacatcctgacgggctcttccacctcttactccttcttcccggacaagcctatcacccagtatccacatgcggtggggaagaacaccctcctcattgctgggctccaggccaggaacaatgcccgcgtcatcttcagcggctccctcgacttcttcagcgactccttcttcaactcagcagtgcagaaggcggcgcccggctcccagaggtattcccagacaggcaactatgaactagctgtggccctctcccgctgggtgttcaaggaggagggtgtcctccgtgtggggcctgtgtcccatcatcgggtgggcgagacagccccacccaatgcctacactgtcactgacctagtggagtatagcatcgtgatccagcagctctcaaatggcaaatgggtcccctttgatggcgatgacattcagctggagtttgtccgcattgatccttttgtgaggaccttcctgaagaagaaaggtggcaaatacagtgttcagttcaagttgcccgacgtgtatggtgtattccagtttaaagtggattacaaccggctaggctacacacacctgtactcttccactcaggtatccgtgcggccactccagcacacgcagtatgagcgcttcatcccctcggcctacccctactacgccagcgccttctccatgatgctggggctcttcatcttcagcatcgtcttcttgcacatgaaggagaaggagaagtccgactga

SEQ ID NO: 62 - protein, 456 aa, Homo sapiens
  MISC_FEATURE: hDDOST
MGYFRCAGAGSFGRRRKMEPSTAARAWALFWLLLPLLGAVCASGPRTLVLLDNLNVRETHSLFFRSLKDRGFELTFKTADDPSLSLIKYGEFLYDNLIIFSPSVEDFGGNINVETISAFIDGGGSVLVAASSDIGDPLRELGSECGIEFDEEKTAVIDHHNYDISDLGQHTLIVADTENLLKAPTIVGKSSLNPILFRGVGMVADPDNPLVLDILTGSSTSYSFFPDKPITQYPHAVGKNTLLIAGLQARNNARVIFSGSLDFFSDSFFNSAVQKAAPGSQRYSQTGNYELAVALSRWVFKEEGVLRVGPVSHHRVGETAPPNAYTVTDLVEYSIVIQQLSNGKWVPFDGDDIQLEFVRIDPFVRTFLKKKGGKYSVQFKLPDVYGVFQFKVDYNRLGYTHLYSSTQVSVRPLQHTQYERFIPSAYPYYASAFSMMLGLFIFSIVFLHMKEKEKSD

SEQ ID NO: 63 - DNA, 1023 bp, Homo sapiens
  misc_feature: hHSP40
atgggtaaagactactaccagacgttgggcctggcccgcggcgcgtcggacgaggagatcaagcgggcctaccgccgccaggcgctgcgctaccacccggacaagaacaaggagcccggcgccgaggagaagttcaaggagatcgctgaggcctacgacgtgctcagcgacccgcgcaagcgcgagatcttcgaccgctacggggaggaaggcctaaaggggagtggccccagtggcggtagcggcggtggtgccaatggtacctctttcagctacacattccatggagaccctcatgccatgtttgctgagttcttcggtggcagaaatccctttgacaccttttttgggcagcggaacggggaggaaggcatggacattgatgacccattctctggcttccctatgggcatgggtggcttcaccaacgtgaactttggccgctcccgctctgcccaagagcccgcccgaaagaagcaagatcccccagtcacccacgaccttcgagtctcccttgaagagatctacagcggctgtaccaagaagatgaaaatctcccacaagcggctaaaccccgacggaaagagcattcgaaacgaagacaaaatattgaccatcgaagtgaagaaggggtggaaagaaggaaccaaaatcactttccccaaggaaggagaccagacctccaacaacattccagctgatatcgtctttgttttaaaggacaagccccacaatatctttaagagagatggctctgatgtcatttatcctgccaggatcagcctccgggaggctctgtgtggctgcacagtgaacgtccccactctggacggcaggacgatacccgtcgtattcaaagatgttatcaggcctggcatgcggcgaaaagttcctggagaaggcctccccctccccaaaacacccgagaaacgtggggacctcattattgagtttgaagtgatcttccccgaaaggattccccagacatcaagaaccgtacttgagcaggttcttccaatatag

SEQ ID NO: 64 - protein, 340 aa, Homo sapiens
  MISC_FEATURE: hHSP40
MGKDYYQTLGLARGASDEEIKRAYRRQALRYHPDKNKEPGAEEKFKEIAEAYDVLSDPRKREIFDRYGEEGLKGSGPSGGSGGGANGTSFSYTFHGDPHAMFAEFFGGRNPFDTFFGQRNGEEGMDIDDPFSGFPMGMGGFTNVNFGRSRSAQEPARKKQDPPVTHDLRVSLEEIYSGCTKKMKISHKRLNPDGKSIRNEDKILTIEVKKGWKEGTKITFPKEGDQTSNNIPADIVFVLKDKPHNIFKRDGSDVIYPARISLREALCGCTVNVPTLDGRTIPVVFKDVIRPGMRRKVPGEGLPLPKTPEKRGDLIIEFEVIFPERIPQTSRTVLEQVLPI

SEQ ID NO: 65 - DNA, 1662 bp, Homo sapiens
  misc_feature: hATP5A1
atgctgtccgtgcgcgttgctgcggccgtggtccgcgcccttcctcggcgggccggactggtctccagaaatgctttgggttcatctttcattgctgcaaggaacttccatgcctctaacactcatcttcaaaagactgggactgctgagatgtcctctattcttgaagagcgtattcttggagctgatacctctgttgatcttgaagaaactgggcgtgtcttaagtattggtgatggtattgcccgcgtacatgggctgaggaatgttcaagcagaagaaatggtagagttttcttcaggcttaaagggtatgtccttgaacttggaacctgacaatgttggtgttgtcgtgtttggaaatgataaactaattaaggaaggagatatagtgaagaggacaggagccattgtggacgttccagttggtgaggagctgttgggtcgtgtagttgatgcccttggtaatgctattgatggaaagggtccaattggttccaagacgcgtaggcgagttggtctgaaagcccccggtatcattcctcgaatttcagtgcgggaaccaatgcagactggcattaaggctgtggatagcttggtgccaattggtcgtggtcagcgtgaactgattattggtgaccgacagactgggaaaacctcaattgctattgacacaatcattaaccagaaacgtttcaatgatggatctgatgaaaagaagaagctgtactgtatttatgttgctattggtcaaaagagatccactgttgcccagttggtgaagagacttacagatgcagatgccatgaagtacaccattgtggtgtcggctacggcctcggatgctgccccacttcagtacctggctccttactctggctgttccatgggagagtattttagagacaatggcaaacatgctttgatcatctatgacgacttatccaaacaggctgttgcttaccgtcagatgtctctgttgctccgccgaccccctggtcgtgaggcctatcctggtgatgtgttctacctacactcccggttgctggagagagcagccaaaatgaacgatgcttttggtggtggctccttgactgctttgccagtcatagaaacacaggctggtgatgtgtctgcttacattccaacaaatgtcatttccatcactgacggacagatcttcttggaaacagaattgttctacaaaggtatccgccctgcaattaacgttggtctgtctgtatctcgtgtcggatccgctgcccaaaccagggctatgaagcaggtagcaggtaccatgaagctggaattggctcagtatcgtgaggttgctgcttttgcccagttcggttctgacctcgatgctgccactcaacaacttttgagtcgtggcgtgcgtctaactgagttgctgaagcaaggacagtattctcccatggctattgaagaacaagtggctgttatctatgcgggtgtaaggggatatcttgataaactggagcccagcaagattacaaagtttgagaatgctttcttgtctcatgtcgtcagccagcaccaagccttgttgggcactatcagggctgatggaaagatctcagaacaatcagatgcaaagctgaaagagattgtaacaaatttcttggctggatttgaagcttaa

SEQ ID NO: 66 - protein, 553 aa, Homo sapiens
  MISC_FEATURE: hATP5A1
MLSVRVAAAVVRALPRRAGLVSRNALGSSFIAARNFHASNTHLQKTGTAEMSSILEERILGADTSVDLEETGRVLSIGDGIARVHGLRNVQAEEMVEFSSGLKGMSLNLEPDNVGVVVFGNDKLIKEGDIVKRTGAIVDVPVGEELLGRVVDALGNAIDGKGPIGSKTRRRVGLKAPGIIPRISVREPMQTGIKAVDSLVPIGRGQRELIIGDRQTGKTSIAIDTIINQKRFNDGSDEKKKLYCIYVAIGQKRSTVAQLVKRLTDADAMKYTIVVSATASDAAPLQYLAPYSGCSMGEYFRDNGKHALIIYDDLSKQAVAYRQMSLLLRRPPGREAYPGDVFYLHSRLLERAAKMNDAFGGGSLTALPVIETQAGDVSAYIPTNVISITDGQIFLETELFYKGIRPAINVGLSVSRVGSAAQTRAMKQVAGTMKLELAQYREVAAFAQFGSDLDAATQQLLSRGVRLTELLKQGQYSPMAIEEQVAVIYAGVRGYLDKLEPSKITKFENAFLSHVVSQHQALLGTIRADGKISEQSDAKLKEIVTNFLAGFEA

SEQ ID NO: 67 - DNA, 3129 bp, Homo sapiens
  misc_feature: hSERCA2
atggagaacgcgcacaccaagacggtggaggaggtgctgggccacttcggcgtcaacgagagtacggggctgagcctggaacaggtcaagaagcttaaggagagatggggctccaacgagttaccggctgaagaaggaaaaaccttgctggaacttgtgattgagcagtttgaagacttgctagttaggattttattactggcagcatgtatatcttttgttttggcttggtttgaagaaggtgaagaaacaattacagcctttgtagaaccttttgtaattttactcatattagtagccaatgcaattgtgggtgtatggcaggaaagaaatgctgaaaatgccatcgaagcccttaaggaatatgagcctgaaatgggcaaagtgtatcgacaggacagaaagagtgtgcagcggattaaagctaaagacatagttcctggtgatattgtagaaattgctgttggtgacaaagttcctgctgatataaggttaacttccatcaaatctaccacactaagagttgaccagtcaattctcacaggtgaatctgtctctgtcatcaagcacactgatcccgtccctgacccacgagctgtcaaccaagataaaaagaacatgctgttttctggtacaaacattgctgctgggaaagctatgggagtggtggtagcaactggagttaacaccgaaattggcaagatccgggatgaaatggtggcaacagaacaggagagaacaccccttcagcaaaaactagatgaatttggggaacagctttccaaagtcatctcccttatttgcattgcagtctggatcataaatattgggcacttcaatgacccggttcatggagggtcctggatcagaggtgctatttactactttaaaattgcagtggccctggctgtagcagccattcctgaaggtctgcctgcagtcatcaccacctgcctggctcttggaactcgcagaatggcaaagaaaaatgccattgttcgaagcctcccgtctgtggaaacccttggttgtacttctgttatctgctcagacaagactggtacacttacaacaaaccagatgtcagtctgcaggatgttcattctggacagagtggaaggtgatacttgttcccttaatgagtttaccataactggatcaacttatgcacctattggagaagtgcataaagatgataaaccagtgaattgtcaccagtatgatggtctggtagaattagcaacaatttgtgctctttgtaatgactctgctttggattacaatgaggcaaagggtgtgtatgaaaaagttggagaagctacagagactgctctcacttgcctagtagagaagatgaatgtatttgataccgaattgaagggtctttctaaaatagaacgtgcaaatgcctgcaactcagtcattaaacagctgatgaaaaaggaattcactctagagttttcacgtgacagaaagtcaatgtcggtttactgtacaccaaataaaccaagcaggacatcaatgagcaagatgtttgtgaagggtgctcctgaaggtgtcattgacaggtgcacccacattcgagttggaagtactaaggttcctatgacctctggagtcaaacagaagatcatgtctgtcattcgagagtggggtagtggcagcgacacactgcgatgcctggccctggccactcatgacaacccactgagaagagaagaaatgcaccttgaggactctgccaactttattaaatatgagaccaatctgaccttcgttggctgcgtgggcatgctggatcctccgagaatcgaggtggcctcctccgtgaagctgtgccggcaagcaggcatccgggtcatcatgatcactggggacaacaagggcactgctgtggccatctgtcgccgcatcggcatcttcgggcaggatgaggacgtgacgtcaaaagctttcacaggccgggagtttgatgaactcaacccctccgcccagcgagacgcctgcctgaacgcccgctgttttgctcgagttgaaccctcccacaagtctaaaatcgtagaatttcttcagtcttttgatgagattacagctatgactggcgatggcgtgaacgatgctcctgctctgaagaaagccgagattggcattgctatgggctctggcactgcggtggctaaaaccgcctctgagatggtcctggcggatgacaacttctccaccattgtggctgccgttgaggaggggcgggcaatctacaacaacatgaaacagttcatccgctacctcatctcgtccaacgtcggggaagttgtctgtattttcctgacagcagcccttggatttcccgaggctttgattcctgttcagctgctctgggtcaatctggtgacagatggcctgcctgccactgcactggggttcaaccctcctgatctggacatcatgaataaacctccccggaacccaaaggaaccattgatcagcgggtggctctttttccgttacttggctattggctgttacgtcggcgctgctaccgtgggtgctgctgcatggtggttcattgctgctgacggtggtccaagagtgtccttctaccagctgagtcatttcctacagtgtaaagaggacaacccggactttgaaggcgtggattgtgcaatctttgaatccccatacccgatgacaatggcgctctctgttctagtaactatagaaatgtgtaacgccctcaacagcttgtccgaaaaccagtccttgctgaggatgcccccctgggagaacatctggctcgtgggctccatctgcctgtccatgtcactccacttcctgatcctctatgtcgaacccttgccactcatcttccagatcacaccgctgaacgtgacccagtggctgatggtgctgaaaatctccttgcccgtgattctcatggatgagacgctcaagtttgtggcccgcaactacctggaacctggtaaagagtgtgtgcagcctgccaccaaatcctgctcgttctcggcatgcaccgatgggatttcctggccgtttgtgctgctcataatgcccctggtgatctgggtctatagcacagacactaactttagcgatatgttctggtcttga

SEQ ID NO: 68 - protein, 1042 aa, Homo sapiens
  MISC_FEATURE: hSERCA2
MENAHTKTVEEVLGHFGVNESTGLSLEQVKKLKERWGSNELPAEEGKTLLELVIEQFEDLLVRILLLAACISFVLAWFEEGEETITAFVEPFVILLILVANAIVGVWQERNAENAIEALKEYEPEMGKVYRQDRKSVQRIKAKDIVPGDIVEIAVGDKVPADIRLTSIKSTTLRVDQSILTGESVSVIKHTDPVPDPRAVNQDKKNMLFSGTNIAAGKAMGVVVATGVNTEIGKIRDEMVATEQERTPLQQKLDEFGEQLSKVISLICIAVWIINIGHFNDPVHGGSWIRGAIYYFKIAVALAVAAIPEGLPAVITTCLALGTRRMAKKNAIVRSLPSVETLGCTSVICSDKTGTLTTNQMSVCRMFILDRVEGDTCSLNEFTITGSTYAPIGEVHKDDKPVNCHQYDGLVELATICALCNDSALDYNEAKGVYEKVGEATETALTCLVEKMNVFDTELKGLSKIERANACNSVIKQLMKKEFTLEFSRDRKSMSVYCTPNKPSRTSMSKMFVKGAPEGVIDRCTHIRVGSTKVPMTSGVKQKIMSVIREWGSGSDTLRCLALATHDNPLRREEMHLEDSANFIKYETNLTFVGCVGMLDPPRIEVASSVKLCRQAGIRVIMITGDNKGTAVAICRRIGIFGQDEDVTSKAFTGREFDELNPSAQRDACLNARCFARVEPSHKSKIVEFLQSFDEITAMTGDGVNDAPALKKAEIGIAMGSGTAVAKTASEMVLADDNFSTIVAAVEEGRAIYNNMKQFIRYLISSNVGEVVCIFLTAALGFPEALIPVQLLWVNLVTDGLPATALGFNPPDLDIMNKPPRNPKEPLISGWLFFRYLAIGCYVGAATVGAAAWWFIAADGGPRVSFYQLSHFLQCKEDNPDFEGVDCAIFESPYPMTMALSVLVTIEMCNALNSLSENQSLLRMPPWENIWLVGSICLSMSLHFLILYVEPLPLIFQITPLNVTQWLMVLKISLPVILMDETLKFVARNYLEPGKECVQPATKSCSFSACTDGISWPFVLLIMPLVIWVYSTDTNFSDMFWS

SEQ ID NO: 69 - DNA, 1938 bp, Homo sapiens
  misc_feature: hPDIA4
atgaggccccggaaagccttcctgctcctgctgctcttggggctggtgcagctgctggccgtggcgggtgccgagggcccggacgaggattcttctaacagagaaaatgccattgaggatgaagaggaggaggaggaggaagatgatgatgaggaagaagacgacttggaagttaaggaagaaaatggagtcttggtcctaaatgatgcaaactttgataattttgtggctgacaaagacacagtgctgctggagttttatgctccatggtgtggacattgcaagcagtttgctccggaatatgaaaaaattgccaacatattaaaggataaagatcctcccattcctgttgccaagatcgatgcaacctcagcgtctgtgctggccagcaggtttgatgtgagtggctaccccaccatcaagatccttaagaaggggcaggctgtagactacgagggctccagaacccaggaagaaattgttgccaaggtcagagaagtctcccagcccgactggacgcctccaccagaagtcacgcttgtgttgaccaaagagaactttgatgaagttgtgaatgatgcagatatcattctggtggagttttatgccccatggtgtggacactgcaagaaacttgcccccgagtatgagaaggccgccaaggagctcagcaagcgttctcctccaattcccctggcaaaggtcgacgccaccgcagaaacagacctggccaagaggtttgatgtctctggctatcccaccctgaaaattttccgcaaaggaaggccttatgactacaacggcccacgagaaaaatatggaatcgttgattacatgatcgagcagtccgggcctccctccaaggagattctgaccctgaagcaggtccaggagttcctgaaggatggagacgatgtcatcatcatcggggtctttaagggggagagtgacccagcctaccagcaataccaggatgccgctaacaacctgagagaagattacaaatttcaccacactttcagcacagaaatagcaaagttcttgaaagtctcccaggggcagttggttgtaatgcagcctgagaaattccagtccaagtatgagccccggagccacatgatggacgtccagggctccacccaggactcggccatcaaggacttcgtgctgaagtacgccctgcccctggttggccaccgcaaggtgtcaaacgatgctaagcgctacaccaggcgccccctggtggtcgtctactacagtgtggacttcagctttgattacagagctgcaactcagttttggcggagcaaagtcctagaggtggccaaggacttccctgagtacacctttgccattgcggacgaagaggactatgctggggaggtgaaggacctggggctcagcgagagtggggaggatgtcaatgccgccatcctggacgagagtgggaagaagttcgccatggagccagaggagtttgactctgacaccctccgcgagtttgtcactgctttcaaaaaaggaaaactgaagccagtcatcaaatcccagccagtgcccaagaacaacaagggacccgtcaaggtcgtggtgggaaagacctttgactccattgtgatggaccccaagaaggacgtcctcatcgagttctacgcgccatggtgcgggcactgcaagcagctagagcccgtgtacaacagcctggccaagaagtacaagggccaaaagggcctggtcatcgccaagatggacgccactgccaacgacgtccccagcgaccgctataaggtggagggcttccccaccatctacttcgcccccagtggggacaaaaagaacccagttaaatttgagggtggagacagagatctggagcatttgagcaagtttatagaagaacatgccacaaaactgagcaggaccaaggaagagctttga

SEQ ID NO: 70 - protein, 645 aa, Homo sapiens
  MISC_FEATURE: hPDIA4
MRPRKAFLLLLLLGLVQLLAVAGAEGPDEDSSNRENAIEDEEEEEEEDDDEEEDDLEVKEENGVLVLNDANFDNFVADKDTVLLEFYAPWCGHCKQFAPEYEKIANILKDKDPPIPVAKIDATSASVLASRFDVSGYPTIKILKKGQAVDYEGSRTQEEIVAKVREVSQPDWTPPPEVTLVLTKENFDEVVNDADIILVEFYAPWCGHCKKLAPEYEKAAKELSKRSPPIPLAKVDATAETDLAKRFDVSGYPTLKIFRKGRPYDYNGPREKYGIVDYMIEQSGPPSKEILTLKQVQEFLKDGDDVIIIGVFKGESDPAYQQYQDAANNLREDYKFHHTFSTEIAKFLKVSQGQLVVMQPEKFQSKYEPRSHMMDVQGSTQDSAIKDFVLKYALPLVGHRKVSNDAKRYTRRPLVVVYYSVDFSFDYRAATQFWRSKVLEVAKDFPEYTFAIADEEDYAGEVKDLGLSESGEDVNAAILDESGKKFAMEPEEFDSDTLREFVTAFKKGKLKPVIKSQPVPKNNKGPVKVVVGKTFDSIVMDPKKDVLIEFYAPWCGHCKQLEPVYNSLAKKYKGQKGLVIAKMDATANDVPSDRYKVEGFPTIYFAPSGDKKNPVKFEGGDRDLEHLSKFIEEHATKLSRTKEEL

SEQ ID NO: 71 - DNA, 1941 bp, Homo sapiens
  misc_feature: hHSC70 /HSPA8
atgtccaagggacctgcagttggtattgatcttggcaccacctactcttgtgtgggtgttttccagcacggaaaagtcgagataattgccaatgatcagggaaaccgaaccactccaagctatgtcgcctttacggacactgaacggttgatcggtgatgccgcaaagaatcaagttgcaatgaaccccaccaacacagtttttgatgccaaacgtctgattggacgcagatttgatgatgctgttgtccagtctgatatgaaacattggccctttatggtggtgaatgatgctggcaggcccaaggtccaagtagaatacaagggagagaccaaaagcttctatccagaggaggtgtcttctatggttctgacaaagatgaaggaaattgcagaagcctaccttgggaagactgttaccaatgctgtggtcacagtgccagcttactttaatgactctcagcgtcaggctaccaaagatgctggaactattgctggtctcaatgtacttagaattattaatgagccaactgctgctgctattgcttacggcttagacaaaaaggttggagcagaaagaaacgtgctcatctttgacctgggaggtggcacttttgatgtgtcaatcctcactattgaggatggaatctttgaggtcaagtctacagctggagacacccacttgggtggagaagattttgacaaccgaatggtcaaccattttattgctgagtttaagcgcaagcataagaaggacatcagtgagaacaagagagctgtaagacgcctccgtactgcttgtgaacgtgctaagcgtaccctctcttccagcacccaggccagtattgagatcgattctctctatgaaggaatcgacttctatacctccattacccgtgcccgatttgaagaactgaatgctgacctgttccgtggcaccctggacccagtagagaaagcccttcgagatgccaaactagacaagtcacagattcatgatattgtcctggttggtggttctactcgtatccccaagattcagaagcttctccaagacttcttcaatggaaaagaactgaataagagcatcaaccctgatgaagctgttgcttatggtgcagctgtccaggcagccatcttgtctggagacaagtctgagaatgttcaagatttgctgctcttggatgtcactcctctttcccttggtattgaaactgctggtggagtcatgactgtcctcatcaagcgtaataccaccattcctaccaagcagacacagaccttcactacctattctgacaaccagcctggtgtgcttattcaggtttatgaaggcgagcgtgccatgacaaaggataacaacctgcttggcaagtttgaactcacaggcatacctcctgcaccccgaggtgttcctcagattgaagtcacttttgacattgatgccaatggtatactcaatgtctctgctgtggacaagagtacgggaaaagagaacaagattactatcactaatgacaagggccgtttgagcaaggaagacattgaacgtatggtccaggaagctgagaagtacaaagctgaagatgagaagcagagggacaaggtgtcatccaagaattcacttgagtcctatgccttcaacatgaaagcaactgttgaagatgagaaacttcaaggcaagattaacgatgaggacaaacagaagattctggacaagtgtaatgaaattatcaactggcttgataagaatcagactgctgagaaggaagaatttgaacatcaacagaaagagctggagaaagtttgcaaccccatcatcaccaagctgtaccagagtgcaggaggcatgccaggaggaatgcctgggggatttcctggtggtggagctcctccctctggtggtgcttcctcagggcccaccattgaagaggttgattaa

SEQ ID NO: 72 - protein, 646 aa, Homo sapiens
  MISC_FEATURE: hHSC70 /HSPA8
MSKGPAVGIDLGTTYSCVGVFQHGKVEIIANDQGNRTTPSYVAFTDTERLIGDAAKNQVAMNPTNTVFDAKRLIGRRFDDAVVQSDMKHWPFMVVNDAGRPKVQVEYKGETKSFYPEEVSSMVLTKMKEIAEAYLGKTVTNAVVTVPAYFNDSQRQATKDAGTIAGLNVLRIINEPTAAAIAYGLDKKVGAERNVLIFDLGGGTFDVSILTIEDGIFEVKSTAGDTHLGGEDFDNRMVNHFIAEFKRKHKKDISENKRAVRRLRTACERAKRTLSSSTQASIEIDSLYEGIDFYTSITRARFEELNADLFRGTLDPVEKALRDAKLDKSQIHDIVLVGGSTRIPKIQKLLQDFFNGKELNKSINPDEAVAYGAAVQAAILSGDKSENVQDLLLLDVTPLSLGIETAGGVMTVLIKRNTTIPTKQTQTFTTYSDNQPGVLIQVYEGERAMTKDNNLLGKFELTGIPPAPRGVPQIEVTFDIDANGILNVSAVDKSTGKENKITITNDKGRLSKEDIERMVQEAEKYKAEDEKQRDKVSSKNSLESYAFNMKATVEDEKLQGKINDEDKQKILDKCNEIINWLDKNQTAEKEEFEHQQKELEKVCNPIITKLYQSAGGMPGGMPGGFPGGGAPPSGGASSGPTIEEVD

SEQ ID NO: 73 - DNA, 3000 bp, Homo sapiens
  misc_feature: hHYOU1
atggcagacaaagttaggaggcagaggccgaggaggcgagtctgttgggccttggtggctgtgctcttggcagacctgttggcactgagtgatacactggcagtgatgtctgtggacctgggcagtgagtccatgaaggtggccattgtcaaacctggagtgcccatggaaattgtcttgaataaggaatctcggaggaaaacaccggtgatcgtgaccctgaaagaaaatgaaagattctttggagacagtgcagcaagcatggcgattaagaatccaaaggctacgctacgttacttccagcacctcctggggaagcaggcagataacccccatgtagctctttaccaggcccgcttcccggagcacgagctgactttcgacccacagaggcagactgtgcactttcagatcagctcgcagctgcagttctcacctgaggaagtgttgggcatggttctcaattattctcgttctctagctgaagattttgcagagcagcccatcaaggatgcagtgatcaccgtgccagtcttcttcaaccaggccgagcgccgagctgtgctgcaggctgctcgtatggctggcctcaaagtgctgcagctcatcaatgacaacaccgccactgccctcagctatggtgtcttccgccggaaagatattaacaccactgcccagaatatcatgttctatgacatgggctcaggcagcaccgtatgcaccattgtgacctaccagatggtgaagactaaggaagctgggatgcagccacagctgcagatccggggagtaggatttgaccgtaccctggggggcctggagatggagctccggcttcgagaacgcctggctgggcttttcaatgagcagcgcaagggtcagagagcaaaggatgtgcgggagaacccgcgtgccatggccaagctgctgcgtgaggctaatcggctcaaaaccgtcctcagtgccaacgctgaccacatggcacagattgaaggcctgatggatgatgtggacttcaaggcaaaagtgactcgtgtggaatttgaggagttgtgtgcagacttgtttgagcgggtgcctgggcctgtacagcaggccctccagagtgccgaaatgagtctggatgagattgagcaggtgatcctggtgggtggggccactcgggtccccagagttcaggaggtgctgctgaaggccgtgggcaaggaggagctggggaagaacatcaatgcagatgaagcagccgccatgggggcagtgtaccaggcagctgcgctcagcaaagcctttaaagtgaagccatttgtcgtccgagatgcagtggtctaccccatcctggtggagttcacgagggaggtggaggaggagcctgggattcacagcctgaagcacaataaacgggtactcttctctcggatggggccctaccctcaacgcaaagtcatcacctttaaccgctacagccatgatttcaacttccacatcaactacggcgacctgggcttcctggggcctgaagatcttcgggtatttggctcccagaatctgaccacagtgaagctaaaaggggtgggtgacagcttcaagaagtatcctgactacgagtccaagggcatcaaggctcacttcaacctggatgagagtggcgtgctcagtctagacagggtggagtctgtatttgagacactggtagaggacagcgcagaagaggaatctactctcaccaaacttggcaacaccatttccagcctgtttggaggcggtaccacaccagatgccaaggagaatggtactgatactgtccaggaggaagaggagagccctgcagaggggagcaaggacgagcctggggagcaggtggagctcaaggaggaagctgaggccccagtggaggatggctctcagcccccaccccctgaacctaagggagatgcaacccctgagggagaaaaggccacagaaaaagaaaatggggacaagtctgaggcccagaaaccaagtgagaaggcagaggcagggcctgagggcgtcgctccagccccagagggagagaagaagcagaagcccgccaggaagcggcgaatggtagaggagatcggggtggagctggttgttctggacctgcctgacttgccagaggataagctggctcagtcggtgcagaaacttcaggacttgacactccgagacctggagaagcaggaacgggaaaaagctgccaacagcttggaagcattcatatttgagacccaggacaagctgtaccagcccgagtaccaggaagtgtccacagaggagcagcgtgaggagatctctgggaagctcagcgccgcatccacctggctggaggatgagggtgttggagccaccacagtgatgttgaaggagaagctggctgagctgaggaagctgtgccaagggctgttttttcgggtagaggagcgcaagaagtggcccgaacggctgtctgccctcgataatctcctcaaccattccagcatgttcctcaagggggcccggctcatcccagagatggaccagatcttcactgaggtggagatgacaacgttagagaaagtcatcaatgagacctgggcctggaagaatgcaactctggccgagcaggctaagctgcccgccacagagaagcctgtgttgctctcaaaagacattgaagctaagatgatggccctggaccgagaggtgcagtatctgctcaataaggccaagtttaccaagccccggccccggcctaaggacaagaatgggacccgggcagagccacccctcaatgccagtgccagtgaccagggggagaaggtcatccctccagcaggccagactgaagatgcagagcccatttcagaacctgagaaagtagagactggatccgagccaggagacactgagcctttggagttaggaggtcctggagcagaacctgaacagaaagaacaatcgacaggacagaagcggcctttgaagaacgacgaactataa

SEQ ID NO: 74 - protein, 999 aa, Homo sapiens
  MISC_FEATURE: hHYOU1
MADKVRRQRPRRRVCWALVAVLLADLLALSDTLAVMSVDLGSESMKVAIVKPGVPMEIVLNKESRRKTPVIVTLKENERFFGDSAASMAIKNPKATLRYFQHLLGKQADNPHVALYQARFPEHELTFDPQRQTVHFQISSQLQFSPEEVLGMVLNYSRSLAEDFAEQPIKDAVITVPVFFNQAERRAVLQAARMAGLKVLQLINDNTATALSYGVFRRKDINTTAQNIMFYDMGSGSTVCTIVTYQMVKTKEAGMQPQLQIRGVGFDRTLGGLEMELRLRERLAGLFNEQRKGQRAKDVRENPRAMAKLLREANRLKTVLSANADHMAQIEGLMDDVDFKAKVTRVEFEELCADLFERVPGPVQQALQSAEMSLDEIEQVILVGGATRVPRVQEVLLKAVGKEELGKNINADEAAAMGAVYQAAALSKAFKVKPFVVRDAVVYPILVEFTREVEEEPGIHSLKHNKRVLFSRMGPYPQRKVITFNRYSHDFNFHINYGDLGFLGPEDLRVFGSQNLTTVKLKGVGDSFKKYPDYESKGIKAHFNLDESGVLSLDRVESVFETLVEDSAEEESTLTKLGNTISSLFGGGTTPDAKENGTDTVQEEEESPAEGSKDEPGEQVELKEEAEAPVEDGSQPPPPEPKGDATPEGEKATEKENGDKSEAQKPSEKAEAGPEGVAPAPEGEKKQKPARKRRMVEEIGVELVVLDLPDLPEDKLAQSVQKLQDLTLRDLEKQEREKAANSLEAFIFETQDKLYQPEYQEVSTEEQREEISGKLSAASTWLEDEGVGATTVMLKEKLAELRKLCQGLFFRVEERKKWPERLSALDNLLNHSSMFLKGARLIPEMDQIFTEVEMTTLEKVINETWAWKNATLAEQAKLPATEKPVLLSKDIEAKMMALDREVQYLLNKAKFTKPRPRPKDKNGTRAEPPLNASASDQGEKVIPPAGQTEDAEPISEPEKVETGSEPGDTEPLELGGPGAEPEQKEQSTGQKRPLKNDEL

SEQ ID NO: 75 - DNA, 1305 bp, Homo sapiens
  misc_feature: hCMP-SAS
atggactcggtggagaagggggccgccacctccgtctccaacccgcgggggcgaccgtcccggggccggccgccgaagctgcagcgcaactctcgcggcggccagggccgaggtgtggagaagcccccgcacctggcagccctaattctggcccggggaggcagcaaaggcatccccctgaagaacattaagcacctggcgggggtcccgctcattggctgggtcctgcgtgcggccctggattcaggggccttccagagtgtatgggtttcgacagaccatgatgaaattgagaatgtggccaaacaatttggtgcacaagttcatcgaagaagttctgaagtttcaaaagacagctctacctcactagatgccatcatagaatttcttaattatcataatgaggttgacattgtaggaaatattcaagctacttctccatgtttacatcctactgatcttcaaaaagttgcagaaatgattcgagaagaaggatatgattctgttttctctgttgtgagacgccatcagtttcgatggagtgaaattcagaaaggagttcgtgaagtgaccgaacctctgaatttaaatccagctaaacggcctcgtcgacaagactgggatggagaattatatgaaaatggctcattttattttgctaaaagacatttgatagagatgggttacttgcagggtggaaaaatggcatactacgaaatgcgagctgaacatagtgtggatatagatgtggatattgattggcctattgcagagcaaagagtattaagatatggctattttggcaaagagaagcttaaggaaataaaacttttggtttgcaatattgatggatgtctcaccaatggccacatttatgtatcaggagaccaaaaagaaataatatcttatgatgtaaaagatgctattgggataagtttattaaagaaaagtggtattgaggtgaggctaatctcagaaagggcctgttcaaagcagacgctgtcttctttaaaactggattgcaaaatggaagtcagtgtatcagacaagctagcagttgtagatgaatggagaaaagaaatgggcctgtgctggaaagaagtggcatatcttggaaatgaagtgtctgatgaagagtgcttgaagagagtgggcctaagtggcgctcctgctgatgcctgttctactgcccagaaggctgttggatacatttgcaaatgtaatggtggccgtggtgccatccgagaatttgcagagcacatttgcctactaatggaaaaggttaataattcatgccaaaaatag

SEQ ID NO: 76 - protein, 434 aa, Homo sapiens
  MISC_FEATURE: hCMP-SAS
MDSVEKGAATSVSNPRGRPSRGRPPKLQRNSRGGQGRGVEKPPHLAALILARGGSKGIPLKNIKHLAGVPLIGWVLRAALDSGAFQSVWVSTDHDEIENVAKQFGAQVHRRSSEVSKDSSTSLDAIIEFLNYHNEVDIVGNIQATSPCLHPTDLQKVAEMIREEGYDSVFSVVRRHQFRWSEIQKGVREVTEPLNLNPAKRPRRQDWDGELYENGSFYFAKRHLIEMGYLQGGKMAYYEMRAEHSVDIDVDIDWPIAEQRVLRYGYFGKEKLKEIKLLVCNIDGCLTNGHIYVSGDQKEIISYDVKDAIGISLLKKSGIEVRLISERACSKQTLSSLKLDCKMEVSVSDKLAVVDEWRKEMGLCWKEVAYLGNEVSDEECLKRVGLSGAPADACSTAQKAVGYICKCNGGRGAIREFAEHICLLMEKVNNSCQK

SEQ ID NO: 77 - DNA, 1353 bp, Homo sapiens
  misc_feature: hBeclin-1
atggaagggtctaagacgtccaacaacagcaccatgcaggtgagcttcgtgtgccagcgctgcagccagcccctgaaactggacacgagtttcaagatcctggaccgtgtcaccatccaggaactcacagctccattacttaccacagcccaggcgaaaccaggagagacccaggaggaagagactaactcaggagaggagccatttattgaaactcctcgccaggatggtgtctctcgcagattcatccccccagccaggatgatgtccacagaaagtgccaacagcttcactctgattggggaggcatctgatggcggcaccatggagaacctcagccgaagactgaaggtcactggggacctttttgacatcatgtcgggccagacagatgtggatcacccactctgtgaggaatgcacagatactcttttagaccagctggacactcagctcaacgtcactgaaaatgagtgtcagaactacaaacgctgtttggagatcttagagcaaatgaatgaggatgacagtgaacagttacagatggagctaaaggagctggcactagaggaggagaggctgatccaggagctggaagacgtggaaaagaaccgcaagatagtggcagaaaatctcgagaaggtccaggctgaggctgagagactggatcaggaggaagctcagtatcagagagaatacagtgaatttaaacgacagcagctggagctggatgatgagctgaagagtgttgaaaaccagatgcgttatgcccagacgcagctggataagctgaagaaaaccaacgtctttaatgcaaccttccacatctggcacagtggacagtttggcacaatcaataacttcaggctgggtcgcctgcccagtgttcccgtggaatggaatgagattaatgctgcttggggccagactgtgttgctgctccatgctctggccaataagatgggtctgaaatttcagagataccgacttgttccttacggaaaccattcatatctggagtctctgacagacaaatctaaggagctgccgttatactgttctggggggttgcggtttttctgggacaacaagtttgaccatgcaatggtggctttcctggactgtgtgcagcagttcaaagaagaggttgagaaaggcgagacacgtttttgtcttccctacaggatggatgtggagaaaggcaagattgaagacacaggaggcagtggcggctcctattccatcaaaacccagtttaactctgaggagcagtggacaaaagctctcaagttcatgctgacgaatcttaagtggggtcttgcttgggtgtcctcacaattttataacaaatga

SEQ ID NO: 78 - protein, 450 aa, Homo sapiens
  MISC_FEATURE: hBeclin-1
MEGSKTSNNSTMQVSFVCQRCSQPLKLDTSFKILDRVTIQELTAPLLTTAQAKPGETQEEETNSGEEPFIETPRQDGVSRRFIPPARMMSTESANSFTLIGEASDGGTMENLSRRLKVTGDLFDIMSGQTDVDHPLCEECTDTLLDQLDTQLNVTENECQNYKRCLEILEQMNEDDSEQLQMELKELALEEERLIQELEDVEKNRKIVAENLEKVQAEAERLDQEEAQYQREYSEFKRQQLELDDELKSVENQMRYAQTQLDKLKKTNVFNATFHIWHSGQFGTINNFRLGRLPSVPVEWNEINAAWGQTVLLLHALANKMGLKFQRYRLVPYGNHSYLESLTDKSKELPLYCSGGLRFFWDNKFDHAMVAFLDCVQQFKEEVEKGETRFCLPYRMDVEKGKIEDTGGSGGSYSIKTQFNSEEQWTKALKFMLTNLKWGLAWVSSQFYNK

SEQ ID NO: 79 - DNA, 1077 bp, Homo sapiens
  misc_feature: hERdj3
atggctccgcagaacctgagcaccttttgcctgttgctgctatacctcatcggggcggtgattgccggacgagatttctataagatcttgggggtgcctcgaagtgcctctataaaggatattaaaaaggcctataggaaactagccctgcagcttcatcccgaccggaaccctgatgatccacaagcccaggagaaattccaggatctgggtgctgcttatgaggttctgtcagatagtgagaaacggaaacagtacgatacttatggtgaagaaggattaaaagatggtcatcagagctcccatggagacattttttcacacttctttggggattttggtttcatgtttggaggaacccctcgtcagcaagacagaaatattccaagaggaagtgatattattgtagatctagaagtcactttggaagaagtatatgcaggaaattttgtggaagtagttagaaacaaacctgtggcaaggcaggctcctggcaaacggaagtgcaattgtcggcaagagatgcggaccacccagctgggccctgggcgcttccaaatgacccaggaggtggtctgcgacgaatgccctaatgtcaaactagtgaatgaagaacgaacgctggaagtagaaatagagcctggggtgagagacggcatggagtacccctttattggagaaggtgagcctcacgtggatggggagcctggagatttacggttccgaatcaaagttgtcaagcacccaatatttgaaaggagaggagatgatttgtacacaaatgtgacaatctcattagttgagtcactggttggctttgagatggatattactcacttggatggtcacaaggtacatatttcccgggataagatcaccaggccaggagcgaagctatggaagaaaggggaagggctccccaactttgacaacaacaatatcaagggctctttgataatcacttttgatgtggattttccaaaagaacagttaacagaggaagcgagagaaggtatcaaacagctactgaaacaagggtcagtgcagaaggtatacaatggactgcaaggatattga

SEQ ID NO: 80 - protein, 358 aa, Homo sapiens
  MISC_FEATURE: hERdj3
MAPQNLSTFCLLLLYLIGAVIAGRDFYKILGVPRSASIKDIKKAYRKLALQLHPDRNPDDPQAQEKFQDLGAAYEVLSDSEKRKQYDTYGEEGLKDGHQSSHGDIFSHFFGDFGFMFGGTPRQQDRNIPRGSDIIVDLEVTLEEVYAGNFVEVVRNKPVARQAPGKRKCNCRQEMRTTQLGPGRFQMTQEVVCDECPNVKLVNEERTLEVEIEPGVRDGMEYPFIGEGEPHVDGEPGDLRFRIKVVKHPIFERRGDDLYTNVTISLVESLVGFEMDITHLDGHKVHISRDKITRPGAKLWKKGEGLPNFDNNNIKGSLIITFDVDFPKEQLTEEAREGIKQLLKQGSVQKVYNGLQGY

SEQ ID NO: 81 - DNA, 1764 bp, Cricetulus griseus
  misc_feature: CHO_AGE
atgaaaggaattctgtggggagcgttttgtgggaaagctaatgagctgaggcagcgcctggagctgaaagaaaagggcaggcacgtggtgctggaggccacagagaatgaggtggagggcaaaggcggcatgcttctgagctcaggacaggcctgttgtgaggagaagggcctggatgctgaggacggtggtggggacagcaatgacctcagcagcgtcagcgagaccacagacagcacagatgtcaaagacagctcagagacctctctgactctgcctcctagagcctcaccctgccctgcaggcttttggattcttgaaactggagctagccaaagacagtttcaggcctggtttactgcggaggagggtccgctgccaccttcgcctccttttggccctgaactgacttgcagatggagcagtctagaacagctaaaggacatcttggcgctcggagcacagcctcactgggtccacaagctccaaggcttctggtttgttgaggttatcttgtcagcaaaaagattacaggacatggagaaggagcgggcttcactgcaggcctggaaggatcgtgtggcaaaggaacttgacagcgtggtcgctttctggctgcagcactcccatgatcaggaacacgggggtttcttcacatgccttgcccgcaatgggcaggtctatgatgaccttaaatatatctggctgcaggggagacaggtatggatgtattgtcgcttgtaccgcaattttgagcgcttccgccgcgctgagcttctagatgctgcaaaagcaggtggtgagtttttgctgcgttttgcacgggtggcaccgcctgccaagaagtgtgcctttgtgttgactcgggacggccgtccagtgaaggtgcagcggaccattttcagcgagtgtttctacaccattgctatgaatgagctttggagagtaacaaaggaatcacgttaccagaatgaagctgtggagatgatggaccagattgtccactgggtacgggaagacccagctgggctaggccggcctcagctctcagggaccccggatgcagagtccatggcagtgcccatgatgctgatgaatctggtggaccagctttccgaggaagatgaggcactgacaaagaaatatgcagagctatgggactggtgtgcccagaggattcttcagcatgtgcagagggatggaaaagctatactagagaatgtatctcatgatggcaaggaactcactggttgccttggaagacatcagaacccaggccacgcaatagaggctggctggttcctgctccagtatgcccgcaagaaaggtgacgccaaacttcgtgcacacatcatcgacaagtttctcttgttgcctttccgctctggatgggacgctgagcatgggggcctcttctacttccaggatgttgatggtttctgccccacccagctggagtgggacatgaagctgtggtggccacacaatgaagccatgatttccttcctaatgggttacagggacagtggtgacccagccttgctacaaatcttcaatcaggtggctgagtacaccttcaagcattttcatgatcccgagaacggcgaatggttcggctatctgaaccgagagggcaaggtggccctcaactttaagggaggcccatttaaaggctgcttccacgtgccgcggtgcctggccatgtgcgagaagatgttgggagacctgctccaccgtgggagcgcccctgctggctcgaaataa

SEQ ID NO: 82 - protein, 587 aa, Cricetulus griseus
  MISC_FEATURE: CHO_AGE
MKGILWGAFCGKANELRQRLELKEKGRHVVLEATENEVEGKGGMLLSSGQACCEEKGLDAEDGGGDSNDLSSVSETTDSTDVKDSSETSLTLPPRASPCPAGFWILETGASQRQFQAWFTAEEGPLPPSPPFGPELTCRWSSLEQLKDILALGAQPHWVHKLQGFWFVEVILSAKRLQDMEKERASLQAWKDRVAKELDSVVAFWLQHSHDQEHGGFFTCLARNGQVYDDLKYIWLQGRQVWMYCRLYRNFERFRRAELLDAAKAGGEFLLRFARVAPPAKKCAFVLTRDGRPVKVQRTIFSECFYTIAMNELWRVTKESRYQNEAVEMMDQIVHWVREDPAGLGRPQLSGTPDAESMAVPMMLMNLVDQLSEEDEALTKKYAELWDWCAQRILQHVQRDGKAILENVSHDGKELTGCLGRHQNPGHAIEAGWFLLQYARKKGDAKLRAHIIDKFLLLPFRSGWDAEHGGLFYFQDVDGFCPTQLEWDMKLWWPHNEAMISFLMGYRDSGDPALLQIFNQVAEYTFKHFHDPENGEWFGYLNREGKVALNFKGGPFKGCFHVPRCLAMCEKMLGDLLHRGSAPAGSK

SEQ ID NO: 83 - DNA, 1818 bp, Homo sapiens
  misc_feature: hWip1
atggcggggctgtactcgctgggagtgagcgtcttctccgaccagggcgggaggaagtacatggaggacgttactcaaatcgttgtggagcccgaaccgacggctgaagaaaagccctcgccgcggcggtcgctgtctcagccgttgcctccgcggccgtcgccggccgcccttcccggcggcgaagtctcggggaaaggcccagcggtggcagcccgagaggctcgcgaccctctcccggacgccggggcctcgccggcacctagccgctgctgccgccgccgttcctccgtggcctttttcgccgtgtgcgacgggcacggcgggcgggaggcggcacagtttgcccgggagcacttgtggggtttcatcaagaagcagaagggtttcacctcgtccgagccggctaaggtttgcgctgccatccgcaaaggctttctcgcttgtcaccttgccatgtggaagaaactggcggaatggccaaagactatgacgggtcttcctagcacatcagggacaactgccagtgtggtcatcattcggggcatgaagatgtatgtagctcacgtaggtgactcaggggtggttcttggaattcaggatgacccgaaggatgactttgtcagagctgtggaggtgacacaggaccataagccagaacttcccaaggaaagagaacgaatcgaaggacttggtgggagtgtaatgaacaagtctggggtgaatcgtgtagtttggaaacgacctcgactcactcacaatggacctgttagaaggagcacagttattgaccagattccttttctggcagtagcaagagcacttggtgatttgtggagctatgatttcttcagtggtgaatttgtggtgtcacctgaaccagacacaagtgtccacactcttgaccctcagaagcacaagtatattatattggggagtgatggactttggaatatgattccaccacaagatgccatctcaatgtgccaggaccaagaggagaaaaaatacctgatgggtgagcatggacaatcttgtgccaaaatgcttgtgaatcgagcattgggccgctggaggcagcgtatgctccgagcagataacactagtgccatagtaatctgcatctctccagaagtggacaatcagggaaactttaccaatgaagatgagttatacctgaacctgactgacagcccttcctataatagtcaagaaacctgtgtgatgactccttccccatgttctacaccaccagtcaagtcactggaggaggatccatggccaagggtgaattctaaggaccatatacctgccctggttcgtagcaatgccttctcagagaattttttagaggtttcagctgagatagctcgagagaatgtccaaggtgtagtcataccctcaaaagatccagaaccacttgaagaaaattgcgctaaagccctgactttaaggatacatgattctttgaataatagccttccaattggccttgtgcctactaattcaacaaacactgtcatggaccaaaaaaatttgaagatgtcaactcctggccaaatgaaagcccaagaaattgaaagaacccctccaacaaactttaaaaggacattagaagagtccaattctggccccctgatgaagaagcatagacgaaatggcttaagtcgaagtagtggtgctcagcctgcaagtctccccacaacctcacagcgaaagaactctgttaaactcaccatgcgacgcagacttaggggccagaagaaaattggaaatcctttacttcatcaacacaggaaaactgtttgtgtttgctga

SEQ ID NO: 84 - protein, 605 aa, Homo sapiens
  MISC_FEATURE: hWip1
MAGLYSLGVSVFSDQGGRKYMEDVTQIVVEPEPTAEEKPSPRRSLSQPLPPRPSPAALPGGEVSGKGPAVAAREARDPLPDAGASPAPSRCCRRRSSVAFFAVCDGHGGREAAQFAREHLWGFIKKQKGFTSSEPAKVCAAIRKGFLACHLAMWKKLAEWPKTMTGLPSTSGTTASVVIIRGMKMYVAHVGDSGVVLGIQDDPKDDFVRAVEVTQDHKPELPKERERIEGLGGSVMNKSGVNRVVWKRPRLTHNGPVRRSTVIDQIPFLAVARALGDLWSYDFFSGEFVVSPEPDTSVHTLDPQKHKYIILGSDGLWNMIPPQDAISMCQDQEEKKYLMGEHGQSCAKMLVNRALGRWRQRMLRADNTSAIVICISPEVDNQGNFTNEDELYLNLTDSPSYNSQETCVMTPSPCSTPPVKSLEEDPWPRVNSKDHIPALVRSNAFSENFLEVSAEIARENVQGVVIPSKDPEPLEENCAKALTLRIHDSLNNSLPIGLVPTNSTNTVMDQKNLKMSTPGQMKAQEIERTPPTNFKRTLEESNSGPLMKKHRRNGLSRSSGAQPASLPTTSQRKNSVKLTMRRRLRGQKKIGNPLLHQHRKTVCVC

SEQ ID NO: 85 - DNA, 741 bp, Homo sapiens
  misc_feature: hRTP4
atggttgtagatttctggacttgggagcagacatttcaagaactaatccaagaggcaaaaccccgggccacatggacgctgaagttggatggcaaccttcagctagactgcctggctcaagggtggaagcaataccaacagagagcatttggctggttccggtgttcctcctgccagcgaagttgggcttccgcccaagtgcagattctgtgccacacgtactgggagcactggacatcccagggtcaggtgcgtatgaggctctttggccaaaggtgccagaagtgctcctggtcccaatatgagatgcctgagttctcctcggatagcaccatgaggattctgagcaacctggtgcagcatatactgaagaaatactatggaaatggcacgaggaagtctccagaaatgccagtaatcctggaagtgtccctggaaggatcccatgacacagccaattgtgaggcatgcactttgggcatctgtggacagggcttaaaaagctgcatgacaaagccgtccaaatccctactcccccacctaaagactgggaattcctcacctggaattggtgctgtgtacctcgcaaaccaagccaagaaccagtcagctgaggcaaaagaggctaaggggagtgggtatgagaaattagggcccagtcgagacccagatccactgaacatctgtgtctttattttgctgcttgtatttattgtagtcaaatgctttacatcagaatga

SEQ ID NO: 86 - protein, 246 aa, Homo sapiens
  MISC_FEATURE: hRTP4
MVVDFWTWEQTFQELIQEAKPRATWTLKLDGNLQLDCLAQGWKQYQQRAFGWFRCSSCQRSWASAQVQILCHTYWEHWTSQGQVRMRLFGQRCQKCSWSQYEMPEFSSDSTMRILSNLVQHILKKYYGNGTRKSPEMPVILEVSLEGSHDTANCEACTLGICGQGLKSCMTKPSKSLLPHLKTGNSSPGIGAVYLANQAKNQSAEAKEAKGSGYEKLGPSRDPDPLNICVFILLLVFIVVKCFTSE

SEQ ID NO: 87 - DNA, 765 bp, Homo sapiens
  misc_feature: hREEP2
atggtgtcctggatcatctctcgcctggtggtgctcatctttggcaccctgtacccagcctattcttcctacaaggccgtgaagacaaaaaacgtgaaggaatatgtgaaatggatgatgtactggatcgtctttgccttcttcaccacggccgagacgctcacggatatagtgctctcctggttccccttctactttgaactgaagatcgccttcgtgatatggctgctgtccccttacaccaagggctccagcgtgctctaccgcaagttcgtgcacccaacgctgtccaacaaggagaaggagatcgacgagtacatcacgcaggcccgagacaagagctatgagaccatgatgagggtgggcaagaggggcctgaaccttgccgccaatgctgcagtcacagctgccgccaagggccagggggtgctgtcagagaagctccgcagcttcagcatgcaggacctgaccctgatccgggacgaggacgcactgcccctgcagaggcctgacggccgcctccgacccagccctggcagcctcctggacaccatcgaggacttaggagatgaccctgccctgagtctaaggtccagcacaaacccggcagattcccggacagaggcttctgaggatgacatgggagacaaagctcccaagagggccaaacccatcaaaaaagcgcccaaagctgagccactggcttccaagacactgaagacccggcccaagaagaagacctctggcgggggcgactcagcttga

SEQ ID NO: 88 - protein, 254 aa, Homo sapiens
  MISC_FEATURE: hREEP2
MVSWIISRLVVLIFGTLYPAYSSYKAVKTKNVKEYVKWMMYWIVFAFFTTAETLTDIVLSWFPFYFELKIAFVIWLLSPYTKGSSVLYRKFVHPTLSNKEKEIDEYITQARDKSYETMMRVGKRGLNLAANAAVTAAAKGQGVLSEKLRSFSMQDLTLIRDEDALPLQRPDGRLRPSPGSLLDTIEDLGDDPALSLRSSTNPADSRTEASEDDMGDKAPKRAKPIKKAPKAEPLASKTLKTRPKKKTSGGGDSA

SEQ ID NO: 89 - DNA, 783 bp, Homo sapiens
  misc_feature: hDPM1
atggcctccttggaagtcagtcgtagtcctcgcaggtctcggcgggagctggaagtgcgcagtccacgacagaacaaatattcggtgcttttacctacctacaacgagcgcgagaacctgccgctcatcgtgtggctgctggtgaaaagcttctccgagagtggaatcaactatgaaattataatcatagatgatggaagcccagatggaacaagggatgttgctgaacagttggagaagatctatgggtcagacagaattcttctaagaccacgagagaaaaagttgggactaggaactgcatatattcatggaatgaaacatgccacaggaaactacatcattattatggatgctgatctctcacaccatccaaaatttattcctgaatttattaggaagcaaaaggagggtaattttgatattgtctctggaactcgctacaaaggaaatggaggtgtatatggctgggatttgaaaagaaaaataatcagccgtggggccaattttttaactcagatcttgctgagaccaggagcatctgatttaacaggaagtttcagattataccgaaaagaagttctagagaaattaatagaaaaatgtgtttctaaaggctacgtcttccagatggagatgattgttcgggcaagacagttgaattatactattggcgaggttccaatatcatttgtggatcgtgtttatggtgaatccaagttgggaggaaatgaaatagtatctttcttgaaaggattattgactctttttgctactacataa

SEQ ID NO: 90 - protein, 260 aa, Homo sapiens
  MISC_FEATURE: hDPM1
MASLEVSRSPRRSRRELEVRSPRQNKYSVLLPTYNERENLPLIVWLLVKSFSESGINYEIIIIDDGSPDGTRDVAEQLEKIYGSDRILLRPREKKLGLGTAYIHGMKHATGNYIIIMDADLSHHPKFIPEFIRKQKEGNFDIVSGTRYKGNGGVYGWDLKRKIISRGANFLTQILLRPGASDLTGSFRLYRKEVLEKLIEKCVSKGYVFQMEMIVRARQLNYTIGEVPISFVDRVYGESKLGGNEIVSFLKGLLTLFATT

SEQ ID NO: 91 - DNA, 2109 bp, Homo sapiens
  misc_feature: hDRiP78
atggcccagaagcaccccggagaaagagggttgtatggagcccaccacagtggtggtgcctccctcaggactttaggaccctccgtggaccctgaaataccttcattctcaggactcagggactcagcagggactgctcctaatggtacccgctgcctcacagagcactctggtcctaagcacacacagcacccaaacccagcccattggttggacccaagccatggccccccagggggtccaggaccacctagagatgcagaggaccctgatcagagtgagacgtcttcagaagaagaatcaggagtggaccaggaactctcaaaagaaaacgagactgggaaccagaaggatgggaactcttttctttccattccatctgcttgcaactgccagggaacacctggaattccagaagggccttactctgagggaggaaatggttcttctagcaacttttgccaccactgtacctctccagctttgggggaagatgagttggaagaggaatatgatgatgaagaatctctcaagttccccagtgatttttcacgtgtgtccagcggaaagaaacccccatcccggagacagcggcaccgctttccaacgaaggaggatactcgggagggtggacgtagggatcccaggtcccctggtcgacatcggctgggtcggaaacgaagtcaggcagataagcgcaaaggcctgggattgtggggagccgaggaactatgtcaacttggacaggcaggcttttggtggctgattgaactgctggtattggtgggagagtacgtagaaacttgtggccatctcatctatgcctgcaggcaactgaaaagcagtgatttggacctttttcgagtttggatgggagtgtggacagggcggttagggggctgggcccaggtcatgtttcagtttctaagccaggggttttactgtggagtaggactgtttactcgttttcttaagctgctgggtgctttgctgctcctggctctggccctctttttgggctttctacagttgggatggcggtttctggtgggactaggtgaccggttaggctggagggataaggctacctggctcttctcttggctggattctccagccttgcagcgttgcttgactctgctgagagatagcaggccatggcagcggctggtaagaatagttcagtggggctggctggagttgccttgggtcaagcagaatattaataggcaggggaatgcacctgtagctagtgggcgctactgccagcctgaagaggaagtggctcgactcttgaccatggctggggttcctgaggatgagctaaaccctttccatgtactgggggttgaggccacagcatcagatgttgaactgaagaaggcctatagacagctggcagtgatggttcatcctgacaaaaatcatcatccccgggctgaggaggccttcaaggttttgcgagcagcttgggacattgtcagcaatgctgaaaagcgaaaggagtatgagatgaaacgaatggcagagaatgagctgagccggtcagtaaatgagtttctgtccaagctgcaagatgacctcaaggaggcaatgaatactatgatgtgtagccgatgccaaggaaagcataggaggtttgaaatggaccgggaacctaagagtgccagatactgtgctgagtgtaataggctgcatcctgctgaggaaggagacttttgggcagagtcaagcatgttgggcctcaagatcacctactttgcactgatggatggaaaggtgtatgacatcacagagtgggctggatgccagcgtgtaggtatctccccagatacccacagagtcccctatcacatctcatttggttctcggattccaggcaccagagggcggcagagagccaccccagatgcccctcctgctgatcttcaggatttcttgagtcggatctttcaagtacccccagggcagatgcccaatgggaacttctttgcagctcctcagcctgcccctggagccgctgcagcctctaagcccaacagcacagtacccaagggagaagccaaacctaagcggcggaagaaagtgaggaggcccttccaacgttga

SEQ ID NO: 92 - protein, 702 aa, Homo sapiens
  MISC_FEATURE: hDRiP78
MAQKHPGERGLYGAHHSGGASLRTLGPSVDPEIPSFSGLRDSAGTAPNGTRCLTEHSGPKHTQHPNPAHWLDPSHGPPGGPGPPRDAEDPDQSETSSEEESGVDQELSKENETGNQKDGNSFLSIPSACNCQGTPGIPEGPYSEGGNGSSSNFCHHCTSPALGEDELEEEYDDEESLKFPSDFSRVSSGKKPPSRRQRHRFPTKEDTREGGRRDPRSPGRHRLGRKRSQADKRKGLGLWGAEELCQLGQAGFWWLIELLVLVGEYVETCGHLIYACRQLKSSDLDLFRVWMGVWTGRLGGWAQVMFQFLSQGFYCGVGLFTRFLKLLGALLLLALALFLGFLQLGWRFLVGLGDRLGWRDKATWLFSWLDSPALQRCLTLLRDSRPWQRLVRIVQWGWLELPWVKQNINRQGNAPVASGRYCQPEEEVARLLTMAGVPEDELNPFHVLGVEATASDVELKKAYRQLAVMVHPDKNHHPRAEEAFKVLRAAWDIVSNAEKRKEYEMKRMAENELSRSVNEFLSKLQDDLKEAMNTMMCSRCQGKHRRFEMDREPKSARYCAECNRLHPAEEGDFWAESSMLGLKITYFALMDGKVYDITEWAGCQRVGISPDTHRVPYHISFGSRIPGTRGRQRATPDAPPADLQDFLSRIFQVPPGQMPNGNFFAAPQPAPGAAAASKPNSTVPKGEAKPKRRKKVRRPFQR

SEQ ID NO: 93 - DNA, 1020 bp, Cricetulus griseus
  misc_feature: Rad51
atggctatgcagatgcagcttgaagcaaatgcagatacttcagtggaagaagaaagctttggtccacaacctatttcacggttagagcaatgtggcataagtgccaatgatgtgaagaaattagaagaagctggtttccatacggtggaggctgttgcttatgcaccaaagaaggaactcataaatattaagggaattagtgaagccaaagcagacaaaattctggctgaggccgctaaattagttccaatgggtttcaccactgcaactgaatttcaccaaaggcgttcagaaatcatacagattactactggctccaaagagcttgacaaactgcttcaaggtggaattgagactggatctatcacagagatgtttggagaattccgaactgggaagacacagatctgtcatacattggctgtaacatgccagcttcccattgatcgtggtggaggtgaaggaaaggccatgtacattgacaccgagggtacgtttaggccagaacggctgctagcagtggctgagaggtatggtctgtctggcagcgatgtcctagataatgtagcatatgctcgagggttcaacacagaccaccaaacccagctcctttatcaagcatcagccatgatggtagaatccagatatgcactgcttattgtagacagtgctactgccctctacagaacagactactcaggtcgaggagagctttcagccaggcaaatgcatttggccagatttctgaggatgctgctgcgacttgctgatgagtttggtgtagcagtggtaatcaccaaccaggtagtagcccaagtggatggagcagccatgttcactgcagatcccaaaaaacccattggaggaaacatcattgcccatgcatcaacaaccaggctgtacctgaggaaaggaagaggggagaccagaatctgcaaagtctatgactctccctgtctccctgaagctgaagccatgtttgccattaatgcagatggagtaggagatgccaaggactga

SEQ ID NO: 94 - DNA, 1053 bp, Cricetulus griseus
  misc_feature: Rad51b
atgagcaacaagaaactaagacgagtaggtttatcacaagagctgtgtgaccgtttgagcagacatcagattgttaattgtcaggactttttaggtctttccccactggaacttatgaaagtgactggcctgagttatggaggtgtccaggagcttctgtatatggtcagcagggcctgtgccccacagatgcaaacagcctatgatataaagatgcggaggtctgctgaactctccccagcgttcctgtctactaccctttctgctttggacaaagccctgcatggtggtgtggcttgtggatcgctcacagagattacaggtccgccaggttgtgggaaaactcagttttgtataatgatgagtgttttagctacattgcccaccaacatgggaggattagaagggactgtcgtgtatattgacaccgagtctgcgtttactgctgaaagactggtcgagattgcagaatcccgttttccactctattttaacacagaagaaaaactgcttttgatgagcagtaaagttcatcttcaccgggaactcagctgtgaggcagttctgcaaaggcttgaatctttggaggaagagattatttccaaaggagttaagcttgtgattgttgactctattgcttctgtggtcagaaaggagttcgatcctcagcttcagggcaacatcaaagaaaggaacaagttcttggccaaacaagcatccttgctgaagtacctggctgaggaattttcactcccagttatcttgacgaatcaaattacgacccatctgagtggagccctcccttctcaagcagacctggtgtctccggctgatgatttgtccctgtctgaaggcacttctggatccagctgtgtggtagccgcactgggaaactcatggagtcactgtgtgaacacccggctgattctccagtaccttgactcagagagaaggcagattctcattgccaagtcacctctggctgccttcacctccttcatctataccatcaagggggaaggcctagttcttcaaggccaagaaaggccatag

SEQ ID NO: 95 - DNA, 1101 bp, Cricetulus griseus
  misc_feature: Rad51c
atgcagcgggagctagtgagtttcccgctgtctcccacggtgcgagtgaagctggtggctgcgggtttccagacggccgaggacgtcctgggggtgaagccctctgagctcagcaaagaagttgggatatctaaagaggaagctttagaaactctacaaattgtaagaagagagagtctcacagacaaacccagatgtgctggtgcatctgtggcaggcaagaagtacaccgcactggaacttcttgagcaggagcacacccagggcttcataatcaccttctgctcagcgctagataacattcttgggggtggaatacccctaatgaaaacaacggaagtttgtggtgtaccaggtgttggaaaaacacagttatgtatgcagttggcagtggatgtgcagattccagagtgttttggaggagtggcaggtgaagcagtgtttattgatacggagggaagttttatggttgatagagtggtcacccttgcaaatgcctgcattcagcaccttcaccttatagcaggaacacacaaggatgaagaacaccagaaagccttggagggctttactcttgaaaatattctttctcatatttattatttccgttgtcatgattatactgagttgctggcacaagtctatctccttccagatttcctttcaaatcattcaaaggtgcagttagtgataatagatggcattgctcttccttttcgacatgaccttgatgatctatcccttcgtactcgattactaaatggccttgcccaacaaatgatcagcctggcaaataatcacagattagctgttattttaactaatcagatgacaacaaagattgataaaaatcaagcattgcttgttcctgcattaggggaaagctggggacatgctgctacaataagacttatttttcactgggagcaaaagcaaaggtttgcaacattgtacaagtcaccaagccagaaggagtccacaataccatttcagatcacaccacagggatttagagatgctgctgtcactgcttcttcatcacagacagaaggttcttcaaatctccggaaacggtcacgagaaccagaggaaggatgctga

SEQ ID NO: 96 - DNA, 1002 bp, Cricetulus griseus
  misc_feature: Rad51d
aaacatgggcgtgctcagggtggggctgtgcccgggcctcaccgaagagatcgtccagcttctgaagggccaaaggatcaagacagtggcggacctggcagctgctaacctggaggaggtagcccagaagtgtggcttgtcctacaaggccctggttgccctgaggagggtattgctggcgcagttctcggctttcccattaaacggagcagacctatatgaggaactgaagacttccactgccatcctgtccacaggcattggaagcctggacaaactacttgatgctggcctctatacaggggaggtgactgaaattgtaggaggtccaggtagcggaaaaacccaggtgtgcctgtgtgtggctgcaaatgtggcccatagcctgcagcagaatgtactgtatgttgattccagtggaggaatgacagcatcccgcctcctgcagctactacaggctagaacccaagatgaggagaaacaggcaggtgctctccagaggatacaggtggtgcatgtatttgacatcttccagatgctggatatgctacaggaccttcggggctccatggcccagcagtcgacatcttcttcaggcactgtgaaggttgtgattgtggattctgtcactgccgtgattgccccacttctgggaggtcagcagagggaaggcctggccttgatgatgcagctggcccgagagctcaagatcctggcccgggacctagctgtggcagtggtggtgaccaaccacttgacccgagacagggatggtaggaggttcaaacctgctctgggacgctcctggagctttgtgcccagtacccggattctcctggatgtcaccaaaggggctggaacattaggcagaggccaacgcacagtgtgtctgaccaagtctccccgccagccaacaggtctacaggaggtgatagacattgggacattggggactgaggagcagagcccagaattgcctgccaaacagacatgatgctgttt

SEQ ID NO: 97 - DNA, 1257 bp, Cricetulus griseus
  misc_feature: Rad52
atggctggagctgaggaaacagtccgtggaggctgtgacacccatcctccctttgctggtgggaaatctgtgctgtgctttgggcagagccagtacacagcagaggaataccaggctatccagagggctctgaggcagcggctgggcccggagtacatcagcagccgcatggctggaggaggccagaaggtgtgttatattgaaggtcatcgagtaattaacctggccaatgagatgtttggttacaatggctgggcacactccatcacccagcagaatgtggattttgttgacttcaacaatggcaaattctacgtgggagtctgtgcatttgtaagggtgcagttaaaggatggttcctatcatgaggacgtgggttatggagttagtgagggcctaaggtcaaaggccttgtcactggagaaggccaggaaggaggctgtgactgacgggctgaagcgggcactcaggagttttggaaatgcacttggaaactgcattctggacaaagactatctgaggtcactaaataagcttccacgacagctccctcttgaagtggatttaactaaagcaaagagagaagattttgaaccatctgtggaacaggcaagatataatagctgcctacagaatgaagcaccgggacccccaaaaccacaagaagcggcttccccttgcagaccaagccacccacatgattcgaacattaggctgcagggggctaaggactgcagcagctcctgcagtctggccgcccccatggagagtgatgccattcaccagcgcaagctccggaagctccggcagaaacagctgcagcagcagttccggcagcagatggaggcccacctacagggccacacacctgccgtaaaagtgaaagccgagcgtgaggcagtgcttccagaccttcctccaaaacacagtacccctgtaactgctgcctcagaactcctcagggagaaagccatttttccagataaccctgaagacaaccttgaaatgtgggacctgactccggatttagaggacatcattaagcccttgtctagaccagaaccacctcaaacctctgccaccagagtccaggtgatccaggatggtgtcctacacggcctttgccaccagatgccaccagaaaaacatgaagctggtcacctgcaggcccacagcactcaccagcatgtattaggaaactctgactctcataggaagagccaggacctgaagaaaaggaaactggatccatcctga

SEQ ID NO: 98 - DNA, 2235 bp, Cricetulus griseus
  misc_feature: Rad54
atgaggaggagcttagctcccagccagttggccaggaggaaaccagaaggcagatcatctgatgatgaagactggcagcctgggacagtaactcctaagaaacaaaaatccagtaatgagacccagtgcttcctgtctccttttcggaaacctttgactcagttaatcaaccgaccgccttgtctggatagcagtcaacatgaagcgtttattcgaagcattttgtcaaagcctttcaaggtccccattccaaattatcaaggtcctctgggctgtcgagcattgggcttgaaaaaggctggtattcgtcgtgccctccatgaccctctggaagaaggtgccttggttctgtatgagcctcccccactaagcgtccatgaccaactgaagctggacaaggagaaactccctgtccacgtggttgttgatcctattctcagtaaggtgttgcggcctcatcagagagagggagtgaagttcctatgggagtgtgtcaccagtcgtcgaatccctggaagccatggctgtatcatggctgatgagatgggcctgggaaagacactacagtgcatcacattgatgtggacacttttacgccagagcccagagtgcaagccagaaattgagaaagcagtggtagtgtcaccttccagcttggtgaagaactggtacaatgaggttggaaagtggcttggaggcaggatccaacctctggccatcgacggaggctctaaggacgagatagaccgaaaactggaaggattcatgaaccagcgtggagcgagagtgccttctcctattctcatcatttcctatgagacttttcgccttcatgtcggagtccttaaaaaaggaaatgttggactggtcatatgtgatgagggacacaggcttaaaaactctgagaatcagacttaccaggccctggacagcttgaataccagtcgtcgggtgctcatctctgggacccccatccaaaatgacttgcttgaatatttcagcttggtgcacttcgttaattcaggcattttgggaactgcccaggagttcaagaagcattttgagctgccaattttgaggagtcgagatgcagctgccagcgaggcagacaggcagctaggggaggaacgtcttcgagagctcatcagtatagtgaataggtgcctgatacggagaacatcagatatcctctctaaatatctgccagtgaagattgagcaggtggtttgttgtaggctgacaccccttcaaactgagttatataagagatttctgagacaggctaagcctgaagaagaattgcgtgaaggcaagatgagcgtgtcttccctgtcttctatcacctctctaaagaagctatgtaaccatccagccctaatctatgacaagtgtgtgtcaggggaagatggctttgaggatactttggatatcttcccacctggttatacttctaaagctgtagaaccacagctttcaggtaaaatgctggtccttgattacattctggccatgactcgaagccgcagcagtgataaagttgtgctggtgtctaattatactcaaacgttggatctctttgaaaagctgtgccgagctcgaaggtacttgtatgttcgcctggatggtacaatgtccattaagaagcgagccaaggttgtggagcgcttcaatagtccatcgagtcccgattttgtcttcatgctgagcagcaaagctgggggctgtggacttaatctcattggtgctaaccggctggtcatgtttgatcctgactggaacccagccaatgatgaacaagctatggcccgagtctggcgtgatggtcaaaagaagacctgctatatttaccgactgctatctgctggaaccatagaagagaagatctttcagcggcagagccataagaaggcactgagcagctgtgtggttgatgaggagcaagatgtagagagacatttctctcttggcgagctcaaagagctgtttaccctggatgaagctagcctcagcgacacacatgacaggctgcattgccgccgttgtgtaaacagacgccaggtctggccaccccctgacggttctgactgtacttcagatctggctcagtggaaccatagcacagataaacggggactccaggatgaggtactccaggctgcctgggatgcttcacctacagccatcaccttcgtcttccatcatcgttctcatgaggagcagcggggtctccactga

SEQ ID NO: 99 - DNA, 837 bp, Cricetulus griseus
  misc_feature: Xrcc2
atgtgcagcgactttcgtaaggccgagtccgggacggagctccttgcccggcttgaaggcagaagctccctgaaagaactagaacccaacctgtttgctgatgaagattcaccagtacatggtgatgttcttgaatttcatggtccagaaggaacaggaaaaacagaaatgctttatcatttaacagcccgatgtatacttccaaaatcagagggtggactgcaaatagaagtcttatttattgacacagattaccactttgacatgctccggcttgtgacagtgctcgagcacagactgtctcgaagctccgaggagaccatcaagctctgcctgggaagattgttcctggcctactgcagcagcagcttgcagctactgctcacgctgcactcactggaagccctgttctgtagtcacccctctctctgccttctcattgtggatagcctgtcggctttttactggacagaccgcgccagtggaggagagagtgtggccctgcaggaatccactctgaagaagtgttctcagctcctagagaggcttgtcactgagtaccgcttggtgcttttcacaacaacacaaagtctaatgcagaaagcctctgactcagcggagcagcctgcttcctccaagctcccaggtgacggagacacagactacagagcctatctctgcaaggcctggcagaaggtggtgaagcacagagtcatcttctccagagaggacgaggctaagagcagccgcttctcattagtttcacgtcatttaaaaagtaacagtttaaaaaaacatgcttttatgatcagagaaagtggggtggaattctgttga

SEQ ID NO: 100 - DNA, 1050 bp, Cricetulus griseus
  misc_feature: Xrcc3
atggacttggatcaactggacctaaatcccagaattactgctgcaattaagaaggggagactgaggtcagtgaaggaggttctgtgctactcgggaccagacctgcagaggctcaccagcctgtccacccacgatgtgcagcacctactgagagtggccgctctgcacctccagggcagccgggtcctcacagcactgcagctgttccagcagagggagagcttccccgagcagcatcaacgcctgagcctgggctgcccggtcttggatcagttcctgggtggcggcctgcccctggagggcatcactgacctggctggtcgaagctctgcagggaagacccagctggggctacagctctgcttgactgtgcagttcccacgacaatatggaggcctggaggctggggctgtctacatctgcacagaggatgccttccccagcaagcggctgtggcagctcattgaacagcaacagcagctgcggacggatgttcctggggaggtgatccagaagatcagattcagcaaccacatcttcatcgagcatgcggccgacgtggacgccttgctggagtgtgtgagcaagagggttcccattctgctgtcaagggggatggcccgcctggtagtggttgactctgttgctgccccattccgttgtgagtatgatgctcaggccttggccaccagggccaagcacctgcagtctctgggagccgcgctccgcagactgagcagtaccttccggagccctgtgctgtgcatcaaccaggtgatggaaacggtggaggagcaagagtctatgcccaggccactgggggcctgggatgagcacctctctccagcccttggcatcacctgggccaaccagatcctgatgagactgatggttgaccgggcacatgaggacgatgcctccatgggcttacccagaagcccggcacggaccatacgggtgctctctgccccgcacctgcccctctcctcctgctgctacacggtcagtgcggaaggcatcagagggataccgggaaccgagtcctgctaa

SEQ ID NO: 101 - DNA, 5373 bp, Cricetulus griseus
  misc_feature: Brca1
atggatttatctgctgttcaaatcgaagaagtacaaaatgtccttcatgctatgcagaaaatcctggagtgtccaatctgtttggaattgatcaaagaacccatttccacaaagtgtgaccacatattttgcaaattttgtatgctgaaacttcttaaccagaagaaagggccttcacaatgtcctttgtgtaagaatgagataaccaaaaggagcctgcaaggaagcacgaggtttagtcagcttgttgaagagctgttgaaaatcactgatgcttttgagcttgacacaggaatacagtatgcaaacggttacagtatttcaaaattgaaaaattcttctgaacctttgaatgaggaagcttccatcatccagagtgtgggctaccgaaaccgcggcaaaagacttagacagattgaatctggaaatgccaccttgaaggacagtctcagtgtccagctgtctaaccttggaattgtgagatcaacaaagaaaaatcatcagacacagcctcgaaataaatctgtgtacattgaattagagtctgattcttctgaagagacagttagtaaaccagatgactgcagtgtgagagaccaggaactgttacaaaccacctctctgggagctggagatgaagtcagtttggattcttcaaccagagctgcttgtgagttttctgaggacgtaacaaatattgatctgcaccagtgcagtaataaagatttggaccccattgagaatcatgcaactggaagatatccagaaaaatgtcaggatatttctgtttcaaacttacatgtggagccatgtggcacagatattcatgccagctcgttacagcatgagaacagcagcttattactcactgaagacagaatgaatgtagaaaaggctgagttctataataaaagcaaacagtctggcttagccaggagccaacagaacagatgggctgaaagtaaagaaacatgtaatgataggcagattcccagcactgagaaaaaggtagatccaaatactgattccttctgtgggagaaaaaaatggaaaaatcagaaaagtctgtgtcctgagaattctagagctacccaggatgttccttggatgacactgaatagcagcattcagaaagtcaacgagtggttttccaaaactggtgaaatgctaacttgtgatggcacatctgacaggaggcatgagtcaaatgctggagcagctgttgtgttagaagtttcagatgaagtagatggatgttccagttcttcaaaagaaatggacttagtggcctctgatccccataatgctttaaagtgtaaaagtgaaagcgacctctccaaaccagtagagaacaatatccgagataaaatatttgggaaaacgtatcagagaaagggaagtctccctcacttgaaccacgtaactgaaattataggcacatttattgcagaaccacagataacacaagaacaccccttcacaaataaattaaaacgtaaaaggagaactacatgccttcatcctgaggattttatcaagaaagcagatttaacagttactcaaaagacttctaaaaatgtaaatcaaggaactgaccaaatggagccagatggcctagtgatgggtattaccagtaatggtcaagagaatgaaacacaaggtaataatcttcagaaagagaaaaatgctaatccagtgaagtccttggaaaaggggtctgtttccacaactaaagccaaaactataagcaacagtataagtgatttggagctagaattaaatgtccacaattcacaggcacctaagaaaagtcggctgaggaggaagtcttcaaccagatgtgttcttgcactggaaccagtcagtaggaatccaagcccacctgcttgtactgaatttcaaattgatagttgtagcagcagtgaagaaacagagaaaaacaattccaacccaacaccagtcaagaacattagaaagcctcaactcacggaggacacagaacctgcagcagattccaagaagaataaagagccaaatgaacaaagaaggaagagaagggccagtgatcctttcccagaagagaaatttatgcctggcttattaactaactgtccaagttctagtaaacctcaaggacctgccaatcctagccctcagagaaaggaagtagagaaacttgaaacaagccaaatgtctgacagtaccaaagacctgagggatctgttgctggatggagaacagggtttgcccactgagaggtcggaggagagtaccagtgtttcattggtgcctgacactgattatgacactcagaacagtgtgtcattgctggaagctaatgctgtcagatatgcaaaaacagtatcaagccagtgtatgacccagtttgtagcaagtgataaccctaacgaactggtccatggttctaaagatgctggaagtggcacagagtgcttcaagcatccattgagacacgaacttagccacattcaggagaccatagaaatggaagagagtgaacttgatactcagtatttacagaatacatttcaagcttcaaagcgtcagtcatttactttattttcaaaaccaagagatccccaagaggagtgtgtaacagcttgtgcttcctctgtgtccttaagggacatgagtccaaaagtgacttctgaaggtgaacaacaagaagaaagtcggggacacgaagaggctgaaatcagtcacatacaggcagggcctgcgacagtgggcgtgcctctgcctcgtcaggaaggtgatccaggcgctgatacaatgcatgctgcagtgtgcagcctttgtccatcatctcagtacagaagcaatgaaaactcacatcctaaacaatcagcttctcccatcatgtcttctataaaaactggccatgggaaaaccctgtcagaggaacaatctgagaaacatacattgtcaaatgaaaaggcaatgggaaatgagacctttgttcaaagcacaatgcacacaattagccaaaaccacagaaaaaatggttgtcaagaagccaactcaggcagtattaatgaagtgccttccagtggtgaaaacttccaaggacagctaggccgaaacagaaggactaagttaaacactgtgcttccactaggtcttatgcaacctggagtctgtaagcatagttttcctgtcagtgattataaatatcttgaaataaaaaagcaggaaggtgagaatgttggtgcacacttctcttcgtgtctgttttcagataagctcgaacaacctgtagggagtggtaatgtttttcagatttgttctgagacacctgatgacctgttggatgatgttgaaatacaggaaaatactagctttggtgaagttgacataatggagaagtctgctgtttttaacgggagtgtccagagacgagagctcagtaggagccctagccctttaacccatgcatcgctggctcggaatctccagagacggtctaggaagttagagtcctcagaagacagcggatcttgtgaggatgaagaccttccctgcttccaacacttacttggccaagtaagcaaaacacctgaacctagcagtgttgtgacacagcctctgtcagagaaagcagaggggacccaagtgccatggaagagtagtgttggtgactctgataacgaggtgatcttgatagaggcatctcaggaacatcaccctagtgaggatgcaaaatactctggcagcatgttctcttctcagcccagtgctgtacaaggttcaactgcaaatacaagctcccaggaccccttgtttaacctttccaaacaaaagagtcaccagtctgaggatgaggaagattttctaagtgacaaggaattgatttcagatgatgaggaaatgggaacttgcctagaagaagataatgatcaagaagaggatattataatcccagattcagctgaagcggcatctggatatgagagtgaaacaaacctttctgaagattgctcacagagtgatattttaaccactcagcagagggccaccatgaaggataacctgataaagctccagcaggagatggcccacctggaggctgtgctagaacagcaaggggaccagccttctgtccactcctcgtctctcacagctgaaccttgtgcccctgaagacctaccaaacgcagaacaaaacttatcaggaacagcaattttaacttcaaagaatattaatgaaaatcctgtaagccggaatccagcatgcgtttctgctgacaagttccaaccacaacctccagacagttccagcagtgaaaataaagagtcaagggaaggaaggccttccctttttaaatctccgttggcaggcagtaggtgctctgcacacagccgctctgggagtcttcaaaacagaaactgcccatctcaagaggagctcctttggactgttgaagcagggaagtcagaaggaacgccatacctggaatctggaatcagccttttctctaatagagaccctgaatctgagtcccctaaagagccagcttatgtttgcaccacaccagcttcaacctctgcacggacaatatcccagtatcaggtttctgactctttcgagagtccggctgctactcatgctcatactgcagtgatagaaactgtgagcaagaaaaagccagaattgacatcttcaaaaggaagagccaataaaggaatatccatggtggtgtcaggcttgacccccaaagaagtaatgattgtgcaaaagtttgctgaaaaataccgcctcactttaactgatgcaattactgaggagactacccatgtcattatgaaaacagatgctgagcttgtgtgtgaacggacactgaaatattttctgggaattgcaggaggaaaatggatagttagctattcatgggtgattcagtctattcaagaaagaaaacttctgagtgtgcatgaatttgaagtcagaggagatgttgtgactggaagaaaccaccaaggtccaaagcgatccagagaatcccaggaaaagctcttcaaaggcctaacaatctgttgttgtgagcccttcaccaacatgcccaaagatgagctggagaagatgctgcagctgtgtggggcttccgtggtgaaggagctttcgtcactcacccctgacaccggtgttcatccaattgtgattgtacagccaagtgcctggacagaagagaatggctgccctgagattgaccagctgtgtggggcgcacctggtgatgtgggactgggtgttggacagtatatccgtctaccggtgtcgggatctggacgcctacctggtacagaatatcacccatggccacgacagcagcgagccacaggaccccaatgattag

SEQ ID NO: 102 - DNA, 10098 bp, Cricetulus griseus
  misc_feature: Brca2
atgtccaatgaatacaaaaggagaccaactttttttgaaatttttaaggcacgatgcagcacagcagacttaggacctataagcctgaattggtttgaagaactttcttcagaagccccaccatataattttgagcctccagaagaatatgaatataagaccaacaattatgagccacagctgtttaaaacgccacagaggaagctctcttaccatctgttggcttcaactccaataatattcaatgaacaaggtcaaactctaccagtagaccagtcgcctttcaaagaactagggaagactcttggaaatagtagacataaaaatcaccacagaaccaaggccaaaatggactccatggttgatgttgccagtccacctctgaagtcttgtctcagtgaaagccctcttactctgcgatgcacacaggttgtaccacaaagagaaaagccagtgatgtgtggaagtttattttctacaccaaaaatcgaggagggtcagacacctaaacctatttctgaaagtctgggagttgaggtggatcctgatatgtcttggtccagttcattagctacaccaccaacccttagttccactgtgctcatagcccgagatggggaagcacgaggaattgtgtttcctgaagactcccccgctgttttgaaaagctacttttccagccacaatgaaagtctgaaaaagagtggtatatcagttccctctgtgactgacagcgagaacaaaaaccagagggaagcttttagtcatggattggggaaaacgttagaggattcatctggcaaaacaaacagcttcaaagattgccttaggcagtcaataccaaatgttctagaagatggggagacagctgcagatacttctgaagaagatagtttctcattatgttttcctaagcataaaaccagaaaaatgcaaaaaatgagaatgggcaagaccaggaagaaaattttcagtgaaataagaactgatgaattaagtgaagaaactagaagtggagctgatggaaaacattcatttgcacttgaaattgacccaagagatagtgatcccttagatccagatgtgacaaaccagaaatgctttgacaatgggaatgaggaaatctgcgaggaagttgtacagtcttcagacactcgatggtctcagctaaccctttctcgtctaactggtacccagaagggaaaaatacctctacctcctatttcttcttgtaaccaaaataattcagaaaaagacttcatagatacgaaggaagaaggtattgactctgttactttagaaaattctttgcctcatatttctagttttccagaaccagaaaagatgttctgtgagaaaactctggtagataaggaacatgagggacagcatcttgaatcacatgagaactccattgcagggaagcaagtggtatctggaacttgtcaagcagcttgcctattgagagagccacttgaagagtctctgggtaatctcttctcagagagtgtgactagctcagcctttacagaagaacccagtgcctctgcaagtggattgggaatatgtgctgtgtcctcacagagagaggattctttgtgtcctagttcaggtgacactggaaactggccatcaactctcactcacacttctgcaactgtgaacaatacaggtttaatatccagtctaaaaactaaaagaagaaagtttatttactctgtcggtgacagtgcatctcatcaaggaaaaatactacaggcagacagaaagtcagagctcactaacacttctgctcagttcgaaacaagtgcttttgaagcgccattcacgtttacaaatgggaattcaggtttatcagattcttctctccaaagaagctgtttacagaatgatgctgaagagccatctttgtccttatccacctcatttgtgactgcttccaagaaagaaagtagttatagtaatgcattgatatctcaggatctccatgacaaagaagcaatagtcagtgaagaaaaactgcagccacatacagccctggaaactgattgtctgtcgtgcttgccagaaagacaatgtgaatatgatccaaagggtcccaaagtttcagatggaaaagaagaagtcttagtctcagcatgtcatcctgcaggacagcacacagcagcagcacagcccagcagcattagctttgaattacaggaagaccctgtcaatggccacaatagtacaagtcctaaagaaactcctagcttgaaggtgcttctgtcaaagccagttgtgctttctagaggaaaagtgtcatgtaaaatgccagagaaactgcagtgtgagagttataaagataatactgaattaagcaaaagcattcccttgggaggaaataaaatacacatcctaagtgaaaattctaaacctcctgagcttctgccacctggaaaatatgtaacagaagcatcccccacagtgaagtctcagttcaatcagaatacaaatctagcagtcaaaaaaaatgaccaagaagaaacgccttttatttcagaagtaacagtcaatgtgagttctggagaacttttcccagacaatgagaataatttcgcctttcaagtaactcatgaaaataataagactgccttaggaagtactgtggaactgcaggaagaagacctccgccatgctaaagggcctaatctcaacaactctcccacagcagtagatggagacataggtgatgagcaagcagctcatgcactgattatggaagactccgattcctcagctttagtccatgagtgtgcaaagaagagcagaaatactatagagcagcatctgaaaggaaccacagacaaagatttcaattcctccttggatgtgaaatcagatgggaacaatgactatacagacaaatggccaggatttttggatccagtttttaagcataaatttggaggtagcttcagaacagcttccaataaagaaataaaactttcagaacataatgttaagaaaagcaaaatgttcttcaaagatattgaagaggagtatcctactagtttaacctgtattgacatagttaatgcctcaccattagcaaaccaggagatactaagtggaccttatacatttgatttgcagtcagtcactaccatgtctgcccatccacagagtcaggcatctgtttcttgtgaagatactcacacatcacttcaggtgttaccttcaaagcaagattttcattcgaatcacaatttaacacccagccaaaaggcagaaattacagaactttctactatcttggaagaatcaggaagtcagtttgaattcacacagttcaaaaagccaagccatgtagcacagaataatatacctgaagtgcctggaaaacagacggttgccataaatactacttctgaggggtggaaaaggattggtcttcatctcacagtggatcctgcctctgtagctcagacagatgacagcaagaaatttgaaggttctgctggatttagacaaagctttccttgcctgttgaaaagcagttgtaacaaaaatacatctagttttttagcaaatgtaaatgaaatggagtttcgaggatttcgttctgctcttggcacaaagcttagtgtgtctagtgaggctctgcaaaaagctgtgaaactcttcagtgacattgaaagtggtagtgaggagacttccacaaaagtcgacccaagagctttgtcttcaggtgctcgtcatgattctggtgcttctgtgtttaagataaggaaacaaaacagtggtaaaagttttgatgagaaaactagtaagtgccaagtaacattacagaataataccgaagtgactactggtatttttgttgacagaaatcctgaaaattatgcaagaaatacaaaatgtgaagataacaactctactggttttcaaagaagtccttataaattaaaaaactcggaggatagtgaatcaagtacaagcggcacagtttctgttcatcaagatgatggtgacttaccatgtgctgctgatcactgcagcaagtaccctgagtcgtgttcccaatatgtaagggaggaaaacacacaaattaaggaatgtgtatcagatttaacatgtttggaagtcatgaaagctgaggaaacatgctatattcaaccttcagataaagaacaattaccttcaggtaagatggaacaaaatagaaaagattttaatatatcctttcagactgcaagtgggaaaaatgtcagagtctctgaggagtcattaagtaaaagtatgaatattttaaatcaagtaacagatgaatcgatcatctcttcagattctttgaattctaaatttcattgtggcacaaataacaacaagatgggtatttcacatcacaaggaaactaccagtactaaaaaggtatttgaagaacgtttcccagttgggactgtcagtcaattaccaactctccagcagcatcctagatgtgaaatagaaagtatcaaagaacctgctctgttgggttttcataccgctagtggaaaaaaagtcaaaattatgcagaaatctttagacaaagtgaaaaacctttttgatgagacacagtatgttagtcatcaagggtcaaaacccttgaaggacagagagaactgcaaagaaggacttgcattaggatgtgagacaattgaaatacctgcctccaagtgtgaagaaatgcagaagagctttctctctaaggagtctgaagtgctatctaagcaaagtgatcgtttgtataggtcgactgaaaatctcagaacatcaaatggtacctcttctaaagctaatgtacatggaaacatagaaagtgaaatagaaaaaagtcctacaacttgctgcattagtcatttatcttattcagtcactgaagattctgctttgacatgtgacacaggacacggtagaaaaacttgtgtcagtgagtcttctctatccaaagacagaaaatggcttagagaccgactgggtgataagcttcaaaaaagagatgctgccgaaattgaatgtgtaaaagaacatactgagggttatgctggagatgcctcatgtgagcatagtttagacagtatcagaaatgaagttgatataaattgtgtctctgaaaatcaaacttcagccctctttagtgaccctagcatgtgtcatagctgtccatcccattttggttgtcattgtgataacaagcataatgactcaggatatttctcaaaaaataaaatttattctgatactcagccagacacgaagaatgaagacactgccaatttttccagtgtatatgctacaaaagaagtaaatatatacccgccaactgtaaatgaagatatttgtgttcagaaacttgagactaactcttcaccacatacaaataaaaatgtagccattgacttggctatagcagattcaaggaattgtaaggtatgcccatccaagttcattacagatcactcacaagaaactgtgaaaacagtaaaagcaatatttacacataacagtgataaaacaattaagcaaaacacaaagagtaaaccagatacttgccggacaagctgtcagaaagcattggataattcagaggattttatatgtcctagctctttagaagatgactatatgaactcacataagacttctgtttatacccacgatgaacaaatattacagcataacctaagtgtgtctggactggagaaagctcaaataccacctgttcacttggaaacttgggataagtgtaaatctacaagggaacttgcacaggcagcctgttcttcacacatgccggggatttttagcacagcaagtggaaaagctgtacaggtatcagacgcttcattagaaaaggcaaggcaagtgttttctgagatggatggtggtgctaaacagttactttccacattgtctctggaaagtcatgaacaatcagaccactctgggagaagagaaaactctgtgacacataaccctgaggatgtattgtcactcccaaaaacctttgcaagcaatgccaattcatctgtattctctggatttagtacagcaggtggtaaacgggtcacagtttcagaaagtgccttacacaaagttaagggaatgttagaggaatttgatttgatcggaactgaacatactctccagtgtccacctacatctgaaggtgtatcaaaaatacttcctcaatattgtgttgaaaagagaaccccagaataccctataaactctaaattgcagaaaacctatgatgataaattcagtttaccaaacaactataaagaaagtgcttctttggggaatactcattctcttgaagcttctccccaactctctcagtttaagcaagacacacggttggtattaggaaccaaagtatcccttctggaaaaagaacaaaccttccctcaaaatataaaaacagaaagtggtgtaatggaaacttgtcctgatgtccctgtgagaacaaatgtaggagactgttctgctttcgacaaaaagccagagaactgttttgaaacagaagcggtggagattgccaaagcttttatggaagatgatgagctgacggattctgaaccaagtcacgacaaatactcattgtttacctgcccccaaaatgaggctttgttaaatttgagaactagaaagagaagaggaatggctgttgatgcagttggacaacccccaatcaaaagaagcttattaaatgagtttgacaggataatagaaaataaaggaaaatccttaaagccttcaaaaagtgctccagatggtacaataaaagacagaagattgttcacgcaccacatttctctagagccagttacctgtggacccttctgctctaccagagaaaggcaagaaatgcagagtccacatttcactgcacctgctcaaggacttctgtctaaagggcatccttctgtgcgttcggctttggaaaaatcttcaagcaattctacagtttcagtccagccgactcataaagtttctgctacaaggaatgaaaggacaggatgctcagtcacaggcaaatcccacaaagtcttcgtcccacctttcaaaatgaaatcacagtttcacagagataaacatttgaataacaagaatattaattcagaggaaaagaaccaaaagagcagagatggagacagtgaagatgtgaacgacggtgacattcgtcaatttaaaaaaggcagcttccatcaagaggccgctagaattgtcacagagtgtgaagaagagcctttagatttaatgacaagccttcagaatgccagagacctacagaatatacgaattaaaaagaaagaaaggcatcagctctgtccacagccaggcagtctgtatcttaccaagtcatccactctgcctcggatctctctgcaggccgcagtaggaggccggcttccctctgcgtgttctcataagcagctctatatgtatggcgtttctaaagagtgcataagcattaacagcaaaaatgcggaatattttcagtttgacattcaggattattttggtaaagaggacctgtgtgctggaaagggcattcagctggctgatggtggatggctgatcccctccaatgaagggaaggctggaaaagaagaattctatagggctctgtgtgacactccaggtgtggatccaaagcttatttctagcctctgggtctctaatcactaccggtggattgtgtggaaactggcagctatggaatttgcttttcctaaggaatttgctaacagatgcctaaccccagaaagagtgctgcttcaactaaaatacagatacgatgtggaaattgacaacagcagcagatcagccctaaagaagatcctggaaagggatgatactgctgcaaaaacactcgttctctgtgtttctgacgtcatgtcactaagcacaactggatcagaaacttcaggcggcaaaactagtggtgcagatcccaagagcatagacacgatcgaactcacagacggatggtatgctgtcaaggcccagctagaccctccacttgtggctcttgtaaagagcaggagactgactgtgggtcagaaaatcattacccaaggggcagaactggtgggatctcctgatgcctgcgcacctctggaagcaccagactctcttagactgaagatttctgccaacagcacacggcctgctcgctggcacagcaaactggggttctttcatgaccccaggcctttccctctgcccttgtcctcactgttcggtgatggaggaagcgttggctgtgtggacatcattgttcagagagtgtaccctttacagtgggtggagaagacggcatcaggattgtacatattccgtaatgagagagaagaggagaaggaagcagtgagatttgcagcggcccaacagaagaaactggaggccttgttcaccaaaatccaggcagagtttaaagaccatgaagaagactcagcgcagcggcgcgtgctgtcccatgcactcacaaggcagcaggtctatgctctgcaagatggtgcagagctctatgcagcggtgcagagtgcattggatccagatcaccttgagggttgtttcagtgaagagcagctgagagccttgaacaaacacagacaaatgttgaatgataagaagcaagcacagatccaatcagaattccggaaggccgtggagtccgctgagcaagaggagggcttatcaagggatgtttcaactgtgtggaagcttcgagttacaagctacgagagaaaagaaaagtcagctctgctgagtatctggcgtccatcatcagacttacactccctgttaacagaaggaaagagatacagaatctatcatctggcagtatcaaaatctaggagtacatttgaacgacctagcatccagttaacagctacgaaaagaactcagtatcagcagctaccggctgccagtgaaaccgtattccaggtttaccagccgagggagccgcttgacttcagcagactgttagagacagcctttcagcctccttgttctgaagtggacctcgtaggagctgtagtttctgttgtaagaacaacaggtcttgctcctttggtctacctatcagacgaatgccttaatttattagtggtaaagtttgggatagaccttaatgaagacataaagccacatgtgctaattgctgcaagcaacctccagtggcacccagaatccagatcaggagtgccaacgttatttgccgggaatctttccatagtttctgccagtccaaaggaggtctacttccagaagcgagtcaacagaatgaggcaaactgttgagaatatcgatacattttacaaggaggcagaaaagaagcttttacatctgcttaatggaaacagtcccaagtggtccaccccaaataaagactctactcagccggcctacacttgccctgcttcagagctccttgctacaggaggtcagctaatgaggttctcacctaatagtgagcaaagttatccaagtcctttatcacattgcacaccaaaagaaaagtctacacccctggctcggtcagcccagatggcatcaaagtcttgtaacagggagagagagactgatgaccgaaaaacctgcagaaaaagaagagccttggattttctgagtcggctgcccttacctcccccggtcagtcccatttgtacctttgtctctccggctgcacagaaggcttttcagccgccacggagttgtggcaccaaatatgcaacacctatgaagaaaaaagaacccagttcccctcagaggaggacgccatttcagaaggacagtggcatttctcttctggaacaagattcggtagctgatgaagaacttgccttcctcaatacccaagctcttgtacctggctcaccagaagaaaatcaacaagtacttcctggtgactccacaagaacctctgtgccccacaacaaaagaacccccagccagcacagaggccagaccagcatgtaggaccccgatccaggaaggggagtctatctcagggattacagaggtggcaagggcagtgatggaaaattagctgtcgagtcttag

SEQ ID NO: 103 - DNA, 888 bp, Cricetulus griseus
  misc_feature: Cyclin D1
atggaacaccagctcctgtgctgcgaagtggagaccatccgccgcgcgtaccctgacaccaacctcctgaacgaccgagtgctgcgagccatgctcaagaccgaggagacctgcgcgccctccgtgtcttacttcaagtgcgtgcagagggagattgtgccgtccatgcggaaaatcgtggccacctggatgctggaggtctgcgaggagcagaagtgcgaagaggaggtcttccctctggccatgaactacctggaccgtttcctgtctctggagcccctaaaaaagagccgcctgcagctgctaggggccacctgcatgttcgtggcctccaagatgaaggagaccattcctttgaccgccgagaagttgtgcatctacactgacaactctatccggcccgaggagctgctgcaaatggaactccttctggtgaacaaacttaagtggaacctggccgccatgactccccacgatttcatcgaacacttcctctccaaaatgccagaggcggatgagaacaagcagatcatccgcaagcatgcgcagacctttgtggccctctgtgccacagacgtgaagttcatttccaacccgccctccatggtggctgccgggagcgtggtggctgcaatgcaaggcctgaacctgggcagccccaacaactacctgtcctgctaccgcacaacgcactttctttccagagtaatcaagtgtgacccggactgcctccgcgcctgccaggaacagattgaggcccttctggagtccagcctgcgccaggcccagcagaacatcaaccccaaggccaccgaggaagagggagaagcagagggagagactgacctggcctgcacacccaccgatgtacgagatgtggacatctga

SEQ ID NO: 104 - DNA, 882 bp, Cricetulus griseus
  misc_feature: Ercc1
atggaccttgggaaagacgagggaagcctgccgcagcccaccaggaagaagtttgtgatcccactggaagacgaggcccctcctgcaggggccaagcccttattcagatcctcacggaaccccagcaccacggccccctcggtcccagcggcccctcagacgtacgccgagtatgccattgcccagcctccaggaggggctgggcccacagggcccacaggctctgaacctgtgaagggagagaaccccggccagacggtgaaaacgggagcgaaatccaatagcatccttgtgagcccccggcagaggggcaaccctgtgttgaagttcgtgcgcaacgtgccctgggaattcggcgaggtgacccctgactatgtgctgggacagagcacttgcgcccttttcctcagcctccgctaccacaatctccatccagactacatccacgaacggctgcagagcctggggaagagctttgccctgcgtgtgctgttggtccaagtggatgtgaaagatcctcagaaggccctgaaggacctggctaaaatgtgtatcttagcggactgcaccctggtcctggcctggagtgccgaggaagcaggacggtacctggagacctacaaggcatatgagcagaagcccgctgacctcctcatggagaagctggagcagaacttcctgtcccgggccaccgagtgtctgaccaccgtgaagtcagtcaacaaaaccgacagccagaccctcctggctacatttggatcccttgaacagctcttgacggcatcacgggaggacctagccttgtgccccggcctgggcccccagaaggcccgcaggctctttgacgtcctccatgaacccttcctcaaagtgccccgatga

SEQ ID NO: 105 - DNA, 4473 bp, Cricetulus griseus
  misc_feature: MDC1
atggaaaacacccaggttattgactgggatgctgaagaggaggaggagacagaaatacccagtgggtccttggggtatagcttggagcctatagggcagctgcgtctcttcagtagtactcatggaccagaaagagatttcccactctaccttggcaagaatgtaattggccgaagccccgactgctctgtggccctgccttttccatccatctctaaacagcatgcagtaattgaaatctcagcttgcaacaaagcccctatcctccaggattgtgggagcctcaatggcactcaactggtaaagcccccaaaggtcctaacccctggagtgagccatcgtctgaaggaccaggaattaattctgtttgcagactttccctgccagtaccgtcgcttggatgtccctccacctttggtctctcggggacttctaactatagagaagacccccagaatacagggagggtcccaaacctccagagttttgttggctgaggattcggaggaggaagtagattttccttctggaaggtatgtggcaaatggatcaaggaatccaacgtctccatcagcaacagtagtaccagaaagtgatgaagaggggtcttctccagcccaaagtgtccgtgggccgtctttgccctttgacttgggcagtgacacagatgaagagctatgtccacagccagcagttggggagtcctcttcagttgccagggatggtgctgctgcagaggccaagcagctggaagctaatggagtgacatctggtatccagctggtactggctcagcctgctgagcaaaagctcagagatgcaaaagtcaagagtgaggctggcaatggagcggctgtggttgggaggggctccactgtgggtaaggacagcaacacggaaatgggtgaagaacaccagccttccggctttgtggacagcgatacagacgtggaagaagacaggatccctgtgaccccccctgtagttccggggaagaagcaagtcctgcttggagttggtaaaaaggaccctggagcacctgtcgtgacccatctgcaggacagcccagctggtcgtggcacaggtgtggaagaaggcaagactccagtggctggccctccagagagaaaccacacggccatggtgatcagcagcgacacagatgaggaagatggagtctcagcagcagtcaccttggcccatctgaaagacagggggatggctctgtggagcagggagccaggcatggaagaggtcaagtcccaaccacaggtcctcgtagaacgaagccagagtgcctctgggaaagacagtgacacagacgtggaggaggaaaagagagaagtggtccctgacagccccatggacacagatgaggctcttactgtcccacattcagagagccaagctccccatagagccagtgatgatgtagaccagggtgtggatatgggctcccctggtggtcagctagagggaaaccaggcctcctctgccacagtagaagacagtagtgcacaagcagggaaggaagtcctgcctcctgaggaggcctgggaaacagctgtggaggaaggctcatcttcagcagcggcagatgtaagacaaagcaagcagccaggagtagaagatgctgggacagagtgggctgcaactgtttgtgagcaggcgagcatgcttgaggtgggggtccaaggcaggtcacctgctacactggtagagccagtggtggtgcctacagctactctgggggatcccactcagccacagagagagggagcccagacccccacaggaaaggagagaggagtacaaatgggcaggaccaagaatgccaaagactgccgtgatgcagagtctgaagatgtgtgccttccggctacccagtgctttgtagacagggagggccagagctcagaagctgtccagagtttggaagatgagcctacgcaagtctttccatgcactcttccccaagagcctgggccttcccacctcagcctgcagacgccaggtccaggtgcccaggatgtgccttgggaagtcttagctacacagccgttttgtctgagagaagctgaggcctctgaactgcagctcatggacacccaccctgcagctcatgaatcccacccatctgtgtctagtgcatcagcaggacagcagcatctggttcacacagagccgctgggaattgaaggcggagagatgcaaactgtggagaaagccatgggccaattgagttgcaagatggcatctgctggagaggactcaaggggtgatccagaaccctcggcccatcgcctgctttctccagttcctgaagcttcttctccacctcagagtctgctcacctctcagagccaaaagccgtctacaccccagtctctgttacttacctctcccccttctgagctacaccttcctgaaactcctcacaccaagcctaatgtcaggcctcggcggtcctccaggatgacctcctccccacactcctctgctgcccttaagccctatactacctgccccacaaacctgcctgctgcccctagaccaacatctcgggctactcggggcaggggcagggcaaataggtcctctaccaggaccccggaaccagttgtccctacagactctgagcttcaacctcccacctccacagaacagtctgtcatccccaaacccacatctccagtcactcagggcagcataaatggttcctttgttaaaacgcctgaaccagttgttctcacaggtcccaaaatccagcctcccacctccacagaacagcctgttaccccaaaccccacacctcaggccactcggggcaggccacataggtcttccatccagaccccagaaccacttactcccactggtcctgacctccagcctcccacctccacagaacagcctgtcatacctaaacccacatctcgggctgctcggggcaggtcacgtaagtcttctaccaggaccccagaaccagctgtccccactggtcctgacctccagcctcccacctccacagaacagcctgtcacacctaaacccacatctcgggccactcggggcaggtcacgtaagtctgtcagaaccccagaaccagctgtccccactggtcctgacctccagcttcccacctccacagctctgggcactttgggaagggcatgtaagtcctccattgaggattctgaatcagttggaccagtagcctctgattttgaacctcccatctccacagaccttgttgcccctgaggtgacaggtcagagcataacactaaagtcttcaccactaagtgcttctccagtttctgccacctctgaactccagccacctgtccccacagcccagcctgttctcctggagcccattcctcaagccaaccaccgaaggcggcggaaggctgctgggaaacggggctcccacacagttcccattggccaaaagccttactctgcaccctctgaacctggttcccaatcttcaatcaatcaaggcttggcattggaagccgctgagtctattactgttgctcctgagcctgctgtttcccaggctccagagacctccactcagaatcccgtggtgcaaaatgaagcagctgggagatcagggctcattcccaagccccagcctgaggtttctcgatcccgcaagaagccttctactaccacaacctcaccaattcaaaaacgtccccgaagacaaataccccagaagacaatagtccccaaggaagaagatcctgaggaaatgccagtgaaggaagagcctcaggagatagcaattccaacacccggcaaaagaaagagggaccgtgtagaggatgagacccagggaaacccaagtcggagccggcgggctaaacctaaccaagaagcagcagcccccaaggtactgttcacaggagttgtggattctcggggagagcgtgcagtcctggctctgggtggcagtctagccagctcagtaaatgaggcctcccacttggtcactgatcgcatccgaagaacggtcaagttcttgtgtgccctggggaagggcatccctatcctctccctgaactggctgtatcagtccagaaaggctggtcacttcctgccacctgatgactacttggtgactgaccctgaacaagagaagaactttagcttcagccttcgggactccctgagccgggctcggcaacaaaaactgctggagggctatgagatttacgtgacccctggagtgcagccacccccacctcagatgggcgagatcatcagctgctgtgggggcaccaacctgcccagcatgccccagtcctataagccttaccgagttgtcataacttgcactgaagacctacctcgctgcgctatcccatctcgactggggctgcccctcctctctcctgagttcctcctgactggagtgctaaagcaggaagtcacaccagaggcctttgtcctttcaaattag

SEQ ID NO: 106 - DNA, 2412 bp, Cricetulus griseus
  misc_feature: Bard1
atgcaactttctgagtctgtggttggactactaggtaggtacacaagccctgctcgggaacgaaacccacgaggagccccgccccttggcgttgagggcgtggccttgggccgcgctcctctcagaaattcgagcgcgctctcattgcctctcccctccctcttacttgctataaaggagcaacccaggatggtctgctgtctgcttcggctcatcatcatccagagtgtcgagttctttgaaatcatcactaatattctgaaggagccagtatgcttaggagggtgtgagcacatcttctgtagtgtgtgtataagtgattgcgttggatcaggatgtcccgtgtgttacacaccagcctggatcctagacctcaagataaacagacaattggacaacatgattcagctttataggaagcttcaaaatttgctacatgacaataaactttcagatccaaaagacaacacatctaggacaggttcatttgatgatgcagaaagcaagaagaattcaataaaaatgtggtttagtcctcgaagtaagaaggttagatgtgttgtgaataaagtatcagtgccaacccagcctcaaaagacaaaagatgacaaagcccaggaagcctccatatacgaatttgtttccacaagtccccctgaagttgtttctaagagggctaaaacagcttctagaacatctgcaaaaaagcagcagaagaaatctttagctgagatcaacaagaaggggaattcaaggccagaaacagaagatagcaggtttgattctaaagaggaactgaaagaggagagggttgtctcctgtagccaaataccagttatggaaagtccacaggtaaatggtgaaatagacttgttagctagtggttctgttgcagaatctgaatgttctggaagattgaccgaagtttctttaccattggctgagcatatagtatctccaggcactgtgagcaagagtgaagagactcctgagaagaaagtctgtgtaaaagatcttctttcagtagggcgtaatgaaaatcacaaatactgtagcaggcctcctgatcctacttctaagaattgtgagagaagcattccgagcaccagcagagatgtcattaaaccaacagtgcttgcagaaaatatactgttggttgactgttcttcactgccttcagaccagcttcaagttgatgtcacactcaggagaaagagtaacatatcagataactcccttagcctttcaccaggcacacccccaccactgctgaataattcaactcccagacaaatgatgtcaaaaccctccatagtgaagctgtcacccagcattaccgccaggaaaagaaaccacagaggagagactctgcttcatattgcttctattaagggcgatataccttctgttgaatacctcttgcaaaacggaaacgaccccaatgttaaagaccatgctggatggacaccattgcatgaagcctgcagtcatgggcacctgaaggtagtggaattgctgctccagcataacgctttggtgaataccacaggctatcagaatgacacaccactgcacgatgcagtcaagaacggccatgtggatatagtcagggtgttactgtccaatggcgcctccaggaatgctgttaacatatttggtgtacggcctgtggattatacagacaatgaaaatataagatcattattgctgctaccagagaagagtgaatcatcctcaactagccagtgtgcagttgtgactgctggacagcgaagaaatgggcctctggtgcttataggcagtgggctttcttcccaacagcagaaaatgctcagcaaacttgagacagttctcaaggctaaaagatgtgctgagtttgacagtacagtaactcatgtcattgttcctgatgatgaagctcaaagtactctgaagtgtatgcttgggattctcaatgggtgttggatcctgaagtttgactgggtgaaagcttgtttgcacagcaaagtacgtgaacaggaagaaaagtacgaagttcctggaggtccgcagaagagcaggctcaacagagagcagctgttgccaaagctatttgatggatgctacttctttttggggggaaacttcaaacatcatccaaagaatgatctccttaagctcattactgcagcaggaggcaaggtgctcagtagaaagcccaagccagacagtgacgtgactcagaccatcaacactgttgcataccatgccaaccctgactctgaccagcgcttctgtacacagtacatcgtctatgaagatctgtttaattgtcgcccagaaagggttcggcagggcaaagtctggatggctccttccacttggcttatcagctgtgtgatggcctttgaattgcttcctcttgacagctga

SEQ ID NO: 107 - DNA, 2796 bp, Cricetulus griseus
  misc_feature: Lig1 (Ligase 1)
atgagaaaaaaagaaccagagaggaaaggggagaactctgctgccaccatgcagaaaagtatcaggtcatttttccaacccatgaaagagggtaaagcacagaagccggagaaggagacagctaacagcaccaaagagaaggagccacctccaaaggtggcactgaaggagaggaatcgagcagtgcctgagagtgattctccagtgaagaggcctggaaggaaggcagcccaggtcctaagcagcgaaggggaggaggaagatgaagcccccagcacccctaaagtccagaagtctgtgtcagactccaaacaaagctctcctcccagccctgacgcatgtcctgagaacagtcctttccacagtagcccctccatggagatctccccatcaggattcccgaagcgtcgcactgctcggaagcagctcccgaaacggacaattgaggacactgtggaggagcagaatgaggacaaaggcagagcagccaagaaaaggaagaaggaagaagaagcacagactccaatggaaagcctcacagagagtgaagatgtaaaacccaaggaagaaaaggaggagggcaagcatgctgaggcttccaagtcccctgagtcgggaaccttgacaaagacagagaccatcccagtgtgtaaggccggcgtgaaacagaagcctcaggaagaggagcagagcaagcctcctgccagaggcgccaagacactcagcagcttcttcactccccggaagccagcagagaaagccatagtgaaacaagaagagccaggtactccagggaaggaagagaccaagggagccctggatccaacaaattacaatccttccaagagaaactaccaccccattgaagatgcctgctggaaacatggccagaaagtcccttttctcgctgtggcccggacctttgagaagattgaggaggtttctgctcggctcaagatggtggagacactgagcaacttgctgcgctcggtggtggccctgtcacctccagacctgcttcctgttctttacctcagcctcaaccgccttgggccacctcagcagggactagagctgggtgttggtgatggtgtcctccttaaggcagttgcccaggccacaggccgtcagctggagtccatccgggctgaggtagctgagaagggtgacgtgggactggtggccgagaacagccgcagcactcagagactcatgctgccccctcctccgctcaccacctccggggtctttaccaaattctgtgacattgcccggctcactggcagtgcttccatggccaagaagttggatgtcatcaagggcctgtttgttgcctgccgtcactcggaagcccggttcattgccaggtccctaagtggacgcctgcgcctcgggctggctgagcagtccgtcttggctgcccttgccctggctgtgagcctcacaccccctggccaagaatttcccccagctgttgtggatgctgggaagggcaagaccacagaggccagaaagacatggttggaagaacaaggcatgatcttgaagcagaccttctgtgaggtacctgacctggaccgaatcatcccggtgctgctggaacatggcctggaacgcctcccagagcactgcaggctgagcccaggggtccctcttaaaccaatgctggctcatcccactcggggtgtcagcgaggtactgaaacgctttgaggaggtggactttacctgcgagtacaaatatgacgggcagcgggcccagattcatgttctggaaggtggagaggtgaagatcttcagtaggaaccaggaagacaacacaggaaagtacccggacatcatcagccgcatccccaagattaaactcccctcggtcacctcctttatcctggacactgaggctgtggcctgggaccgggaaaagaagcagatccagccattccaagtgctcaccacacgcaagcgcaaggaggttgacgcctcggagatacaggtgcaggtgtgtctgtatgcctttgatctcatctacctcaacggagagtccctgattcgccagcccctgtctcgacgtcggcagctgctccgggagaactttgtggagacagagggtgagtttgtcttcgccacctccctggacaccaaggacatcgagcagatcgctgagttcttggagcagtccgtgaaggactcctgtgagggactgatggtgaagaccctggatgttgatgccacctatgagattgccaagaggtctcacaactggctcaagctaaagaaggactaccttgacggtgtgggcgacactctggaccttgtggtgattggcgcctacctgggccgggggaagcgtgccggccggtatgggggcttcctcttggctgcctatgatgaggagagtgaagagctgcaggccatatgcaagctgggaactggattcagtgatgaagagctggaggagcatcaccagagcctaaaggccctagtgttgccgaccccacgcccctatgtgaggatcgatggggcagttgccccagaccactggctggacccaaaggtcgtatgggaggtgaagtgtgcggatctctccctgtcccctatctaccctgctgcgcggggcctggtggacaaagagaaagggatctcccttcgtttccctcggttcattcgtgtccgtgaagacaagcagccagagcaggccaccaccagtgaccaggtggcctgtttgtaccggaagcagagtcagatacagaaccagcacaactcagacttggactccgactttgaggactgctattaa

SEQ ID NO: 108 - DNA, 2121 bp, Cricetulus griseus
  misc_feature: Mre11
atgagccctgcagatccacttgatgatgaagacacttttaaaatcctggttgccactgatattcaccttggatttatggagaaagatgcagttcgaggaaatgatacatttgtgacacttaatgaaattttaaaacttgccctggaaaatgaagtggattttattttgttaggtggtgatcttttccatgaaaacaagccctcaaggaaaactcttcatagttgcttggagttgcttaggaagtactgtatgggtgatcgccctgtgcagtttgagatcatcagtgaccagtcagtcaactttggttttagtaggtttccatgggtgaactatcaggatggcaatctcaacatttccattccagtgtttagtatccatggcaaccatgacgatcccacaggggcagatgccctctgtgccctggatattttaagctgtgctgggtttgtgaatcactttggacggtcaatgtctgtggagaagattgacattagtccagttctgctgcagaaaggaagcacaaaacttgctctgtacggcctagggtccattcctgatgaaaggctctatcggatgtttgtcaataaaaaagtaacaatgctgagaccaaaggaagatgagaactcatggtttaacttatttgtgattcatcagaacaggagtaaacatggaagtaccaacttcatcccagaacagtttttggatgacttcattgacctcgttatctggggccatgaacacgagtgtaaaattggcccaaccaaaaatgagcagcagctcttctatgtgtctcagcctggaagctcagtggtgacttctctttcccctggagaagctgttaagaaacacgtgggcttgctgcgcgttaaagggaggaagatgaacctgcagaagctgcctctccgcacagtgcggcagttcttcatggaggatgtggttctcgctaaccacccaaacctgttcaaccctgacaatcctaaggtgacccaggccatccagagcttctgcttggagaagattgaagaaatgcttgaaaatgccgagcgcgaacggctagggaattctcttcaaccagagaagcctcttatccgactacgggtggactacagtggaggctttgaaccttttagtgttcttcgctttagccagaaatttgtggatcgggtcgctaaccccaaagatatcatccactttttcaggcatagggagcaaaagggaaaaacaggtgaagagatcaactttgggaagcttgtttcaaaatctccttcggaaggaacgacactcagagtagaagacctggtgaagcagtatttccagactgcggagaagaatgttcagctctcactgctgacagaaagagggatgggtgaagccgttcaagaatttgtggacaaggaagaaaaagatgccatcgaggaattagtgaagtaccagctggagaaaacacagcggtttcttaaggagcgccatatcgatgctctggaagacaagattgacgaagaggtccggcgtttcagagaaagcagacagagaaataccaacgaagaagacgatgaagtgcgagaggccatgagcagggcccgggcgctcagatcgcagtcagagaactctgcctcagccttcagtgctgacgacctgagtttcgatatagcagaacagacagcaaatgactctgatgacagcctgtcagcagtgcccagcagaggccggggccgaggccgaggtcgaagaggaggcagagggcagagcaccgcatcaagaggaggatctcagagaggccgagacactgggcaggagacggctactcgaggcagatgctcaaaggccactacatcgacctctagaaatatgtccattctagacgctttcagatctactcgacagcagccttccagaaacactgccactaaaaattactcagagactattgaagtggatgaatctgatgaagatgacatttttcctaccagttccaaggctgatcaaaggtggccaggcacaacatctagcaaacggatgtcccagagccagatagccaagggggttgactttgaatcagatgaggacgatgacgatgaccctttcatgagcagtagttctctaagaagccgaagataataa

SEQ ID NO: 109 - DNA, 5973 bp, Cricetulus griseus
  misc_feature: 53BP1
atgccaggggagcagatggaccctactggaagtcagttggattcagatttctctcagcaagatactccttgcctgataattgaagattctcagcctgaaagccaggttctggaagaagatgcgggctctcacttcagtgtgctgtctcgacaccttcccaatctgcagatacacaaagagaaccctgtgttggatattgtgtccaatccggaacaagcagctgcagaagagcaaggagacaataatagctccttcaatgaacatctgaaagagaacaaagctgctgcagatcctgtggattccactcatttgggcacatgtgattccatcagtcaggtcatagaacagttgcctcagccaaacaggacaagcagtgttctgggagtgacagtggaagctgcttctcttccagaagaggagaaggaggaagagctggaagaggagaatgaagaggtgggagcagatgctgctgatgccgctccgtgctcccttggtgctgaagattctgcttcatcacagttgggctttggggttctggaactgtcccagagccaggatgttgaagaacatacagtgccatatgatgtcaaccaagaacatatgcagttggttaccaccaactcgggttcttcccagctgtctgacatggatgcaaataatgttaaatgtgaagaacagtccactgaagatacctccatggcagaacaacctaacaaagacatccctgttacagtcgagcacagtaaaggtatccctgtggtagatgagcaaaatctaccaccggcaaggccagaggatctgccttccagtcctcaagcctctgctgcagctgtggaaacaaaggaagaggtacctgcccaagagttgccagaaggggcgctggaggttcagatgtcctcggagcctgaggtctcgtccactcaggaggacttgtttgagcagagtagtaaaacagcttctgatggttgttctactccttcaagggaggaaggtgggtgttctccggtttccacacccgccaccaccctgcaactcctgcagctgtctggtcagaggccccttgtccaggacagtctttccacgaattcctcagatcttgttgctccttcccctgatgctttccgacctaccccttttatcgttcctagcagtcccacagagcaaggagggagaaaagttgagcccttggatatgtcagtgatgcctgaagaaggaggggagactttgcagaagcttcaggatgacgaagcagtggagatagaaaagccccatctcccatctcagccggctgtttccccacaagtgtcaacaccagtgtctcagagcacacctgtcttcactccaggctctcttcccatcccgtcccagcctgaattttctcatgacattttcattccatcaccaagtttggaagaaccatcaagtgatgggaagaaaggtggcgatttgcacagctcatctttgactgtggagtgttctaagacttcagagagtgaaccaaagaatttcactgctgatcttgggctctccttgacaggggagtcttgcaaactgatgctttcttcaagtgagtatagtcaatcctcaaagatggagagcttggcttctcccaggagtgagggagatggagagaatacccagattgaggacactgaaccgttgtctccagtcaccaattctaaacttcctgctgaaagtgatgatgtcctgatgaatccagcaccagatgaccaagtagaaatgaatcagaatgatgacaaagtaaaagagggtgacacagagaacacaggtgaccatggtgttttagctgctggtagtaaaggcagagaagaaaccgttgctgaagatgtttgcattgatctcacttgtgattctgggagtcaggcagttccgtctcccgctactcggtccgaggcactttctagtgtcttagatcaggaggaagctatggaaattaaagaacagcatccagaggaggggttttcgggatctgaggtagaagaagtccccgagactccctgtgaaagtcacagagaggagcccaaggaagaaacgatggagagtatcccactgcacctttctcttactgaaacacagtcccaggcattgtgtcttcagaaggaaatgcccaaagaagaatgcccagaggccatggaagtggaaccctctgtgattagtgttgactctccccagaagctgccggtactcgaccaggagtcagagcataaggagccagaggcctgggaagaagccgcgtcggaggactcaagtgtggaggactcaagtgtggttatcgttgatgtgaaggagccctcgccaagagttgtcccctgcgaacctttggagggagcagagaaatgctcagattcccactcctgggaggatgtggtgcccgaggtggaaccgtgtgctgcaaatagagtagacactccggaggaaaagattgtagaatgtgacggagatgtgaaagcagagaccacaagaaaggactctgtagaggaagactccccacagcctcctttgccttcagtgaaagacgagcctcccagagacgagcctcccagacccgaccaggagatgcagcagtcccagcttcaagagaaagagagcccagtgaccatagatgcaaaagtggctgatgccaagcagctggagtcagagggagcatcccagcagctttcgaaagcccctgcccgcgactcacaaagtttctgtgaaagttctagtgaaaccccatttcatttcactttgcctaaagaaggtgatattatcccaccattgactggtgcaaccccacctcacattgggcacctaaaattggatcgcaacagacatagtactccaattgggattggcaactatccagaaagcaccatagcaaccagtgatgtcatgtctgaaagcatggtggagatcaatgatcctctacttgggagtgaaaaaggagattctgagtctgccccagaaatggacggaaaactgtatctgaaaatgaaactggttagtcctgagacagaggccagtgaagaatctttgcagtttagcctggaaaagcctgctactgctgagagaaaaaatggatcaactgctgttgctgagcctgttgcaaaaaatggatcaactgctgttgctgagcctgttgccagtccccagaagaccgtgcctgtgtttagctgcaggcaagaggaggtttggagtgaggaccctccctctgtacccatcagggcaaacttgctccattttccaagtgttgaagaagaggacaaagaaaaactggatggtaccccaaagcttaggcagagtgaacagcctgtgaggcccgttgggctggtcaaggatgctgctacttctgaggactctgcttcttctgttccccagcagagagcaacacaggggtcattcagccctcaaggagaagtgatggaaacagacctgctagaaggactgagtgctaaccaggaaaaaccgtgtaaggtcttgatggaaaggcccacccagagtaacataggaatccagaccatggaccattccctgtgtgctccagaaactgtttcagcagcaacccagactgtgaagagtgtatgtgaacaagggaccagtacagtggaccagaactctgggaaacaagatgccactgtgcagaccgagagggggggtgtcgagaaacaggcccctgtggacgatacagaatccctccacagccagggagaagaagaatttgaaatgccccagcctccacatggccatgtcttgcatcgtcacatgagaaccatccgtgaagtccggacacttgtcacccgtgtcatcacagatgtttactatgtggatgggacagaagtggaaaggaaagtaactgaggagactgaagaaccaattgtagaatgtcaggaatgtgaaacagaggtttccccttcccagactggaggctcttctggagacctgggagacatcagttccttctcctccaaagcatccagctcacaccatacatcaagtgggacaagtctctcagccatgcatagcagtggcagctcaggacgaggagccgggccactcaaagggaaaaccagcgggacagaacctgcagattttgctttacccagttcccgaggaggcccaggaaaactgagtcctagaaaagggatcaatcagacaggggcaccagtgtgtgaggaagatggtgatgcaggccttggcatcagacagggagggaaggctcctgtcacacctcgtggtcgtggtcgaaggggccgcccaccttctcggaccactggaacaagagatgcagttgtgtctggtccgttgggcatagaagacatttcacctagcatgtcaccagatgacaagtccttcacccgaattgtgccccgtgtaccagactctaccaaacgaattgataccagttctactgttttgaggcggagtgattccccagagattccttttcaggctgctactgggtcttctgatggcttggatgcctcatctccaggaaatagctttgtcgggctccgtgttgtagccaagtggtcatccaatggctatttttactctgggaaaatcacacgggatgttggagctgggaagtataagctgctcttcgatgatgggtatgaatgtgatgtgctgggcaaagacattctcctgtgtgaccctatacccctggacactgaagtgacagccctctcagaagatgagtatttcagtgcaggagtggtcaaaggacacagaaaggagtctggggagctgtactacagcattgaaaaagaaggccaaaggaagtggtataagcggatggcagtcatcctgtccttggaacaaggaaacaggttaagagagcaatatgggcttggcccatatgaagctgttacacccctcacaaaggcagcagacatcagcctagataatttggtggaaggaaagcggaaacgtcgcagtaacatcagctccccagccacccccactgcctccagcagcagcagcagcagcagcacaacacccacccgtaaaaccacagagagtccccgtgcttccacgggagttccatcaggcaaaaggaaactcatcacttctgaagaggaacggtccccagctaagcgaggccgcaagtctgtcaccgtgaaacctggtacagtgggggcaggagaatttgtgagcccctgcgagagtggagacaacacaggtgaaccttctgtcctggaagagccaagagggcctttgcccctcaacaagaccttgtttctgggctatgcctttctccttaccatggccacaaccaatgacaagctggccagccgctctaaactgctagatggtcctacaggaagcagtgaagaagaggaggaatttttagaaattcctcctttcaacaagcagtatacagaatgccagcttcgagcaggagctgggtatatccttgaagacttcaatgaagcccagtgtaacacagcctaccagtgtctcctaattgctgatcagcattgtcgaacccggaagtacttcctgtgccttgccagtggaattccttgtgtgtctcatgtctgggtccatgacagctgccatgccaaccagctccaaaactaccgtaattatctgctgcctgctgggtatagccttgaggagcagcgaattctggattggcaacctcgtgaaaaccctttccagaatctgaaggtactcttggtgtcagatcaacaacagaacttcctggagctctggtctgagatcctcatgactggaggggcagcctctgtgaagcagcaccattcaagtgcccataacaaagacattgctttaggggtatttgatgtggtggtgacagacccctcatgcccagcctcggtgctcaagtgtgctgaagccttgcagctgcctgtggtgtcacaagagtgggtgatccagtgcctcattgttggggagagaattggattcaagcagcatccaaaatataaacatgattatgtttctcactaa

SEQ ID NO: 110 - DNA, 384 bp, Human cytomegalovirus
  misc_feature: CMV IE enhancer
gttgacattgattattgactagttattaatagtaatcaattacggggtcattagttcatagcccatatatggagttccgcgttacataacttacggtaaatggcccgcctggctgaccgcccaacgacccccgcccattgacgtcaataatgacgtatgttcccatagtaacgccaatagggactttccattgacgtcaatgggtggagtatttacggtaaactgcccacttggcagtacatcaagtgtatcatatgccaagtacgccccctattgacgtcaatgacggtaaatggcccgcctggcattatgcccagtacatgaccttatgggactttcctacttggcagtacatctacgtattagtcatcgctattaccatgg

SEQ ID NO: 111 - DNA, 799 bp, Homo sapiens
  misc_feature: Human GAPDH promoter
gagaagttccccaactttcccgcctctcagcctttgaaagaaagaaaggggagggggcaggccgcgtgcagccgcgagcggtgctgggctccggctccaattccccatctcagtcgttcccaaagtcctcctgtttcatccaagcgtgtaagggtccccgtccttgactccctagtgtcctgctgcccacagtccagtcctgggaaccagcaccgatcacctcccatcgggccaatctcagtcccttcccccctacgtcggggcccacacgctcggtgcgtgcccagttgaaccaggcggctgcggaaaaaaaaaagcggggagaaagtagggcccggctactagcggttttacgggcgcacgtagctcaggcctcaagaccttgggctgggactggctgagcctggcgggaggcggggtccgagtcaccgcctgccgccgcgcccccggtttctataaattgagcccgcagcctcccgcttcgctctctgctcctcctgttcgacagtcagccgcatcttcttttgcgtcgccaggtgaagacgggcggagagaaacccgggaggctagggacggcctgaaggcggcaggggcgggcgcaggccggatgtgttcgcgccgctgcggggtgggcccgggcggcctccgcattgcaggggcgggcggaggacgtgatgcggcgcgggctgggcatggaggcctggtgggggaggggaggggaggcgtgtgtgtcggccggggccactaggcgctcactgttctctccctccgcgcagccgagccacatcgctcagacacc

SEQ ID NO: 112 - DNA, 1188 bp, Homo sapiens
  misc_feature: Human Ef1 alpha promoter
catgggtgaggctccggtgcccgtcagtgggcagagcgcacatcgcccacagtccccgagaagttggggggaggggtcggcaattgaaccggtgcctagagaaggtggcgcggggtaaactgggaaagtgatgtcgtgtactggctccgcctttttcccgagggtgggggagaaccgtatataagtgcagtagtcgccgtgaacgttctttttcgcaacgggtttgccgccagaacacaggtaagtgccgtgtgtggttcccgcgggcctggcctctttacgggttatggcccttgcgtgccttgaattacttccacctggctgcagtacgtgattcttgatcccgagcttcgggttggaagtgggtgggagagttcgaggccttgcgcttaaggagccccttcgcctcgtgcttgagttgaggcctggcctgggcgctggggccgccgcgtgcgaatctggtggcaccttcgcgcctgtctcgctgctttcgataagtctctagccatttaaaatttttgatgacctgctgcgacgctttttttctggcaagatagtcttgtaaatgcgggccaagatctgcacactggtatttcggtttttggggccgcgggcggcgacggggcccgtgcgtcccagcgcacatgttcggcgaggcggggcctgcgagcgcggccaccgagaatcggacgggggtagtctcaagctggccggcctgctctggtgcctggcctcgcgccgccgtgtatcgccccgccctgggcggcaaggctggcccggtcggcaccagttgcgtgagcggaaagatggccgcttcccggccctgctgcagggagctcaaaatggaggacgcggcgctcgggagagcgggcgggtgagtcacccacacaaaggaaaagggcctttccgtcctcagccgtcgcttcatgtgactccacggagtaccgggcgccgtccaggcacctcgattagttctcgagcttttggagtacgtcgtctttaggttggggggaggggttttatgcgatggagtttccccacactgagtgggtggagactgaagttaggccagcttggcacttgatgtaattctccttggaatttgccctttttgagtttggatcttggttcattctcaagcctcagacagtggttcaaagtttttttcttccatttcaggtgtcgtga

SEQ ID NO: 113 - DNA, 985 bp, Simian cytomegalovirus
  misc_feature: CMV promoter
gaccatagccaattcaatatggcgtatatggactcatgccaattcaatatggtggatctggacctgtgccaattcaatatggcgtatatggactcgtgccaattcaatatggtggatctggaccccagccaattcaatatggcggacttggcaccatgccaattcaatatggcggacttggcactgtgccaactggggaggggtctacttggcacggtgccaagtttgaggaggggtcttggccctgtgccaagtccgccatattgaattggcatggtgccaataatggcggccatattggctatatgccaggatcaatatataggcaatatccaatatggccctatgccaatatggctattggccaggttcaatactatgtattggccctatgccatatagtattccatatatgggttttcctattgacgtagatagcccctcccaatgggcggtcccatataccatatatggggcttcctaataccgcccatagccactcccccattgacgtcaatggtctctatatatggtctttcctattgacgtcatatgggcggtcctattgacgtatatggcgcctcccccattgacgtcaattacggtaaatggcccgcctggctcaatgcccattgacgtcaataggaccacccaccattgacgtcaatgggatggctcattgcccattcatatccgttctcacgccccctattgacgtcaatgacggtaaatggcccacttggcagtacatcaatatctattaatagtaacttggcaagtacattactattggaaggacgccagggtacattggcagtactcccattgacgtcaatggcggtaaatggcccgcgatggctgccaagtacatccccattgacgtcaatggggaggggcaatgacgcaaatgggcgttccattgacgtaaatgggcggtaggcgtgcctaatgggaggtctatataagcaatgctcgtttagggaac

SEQ ID NO: 114 - DNA, 197 bp, Simian virus 40
  misc_feature: SV40 promoter
tgcatctcaattagtcagcaaccatagtcccgcccctaactccgcccatcccgcccctaactccgcccagttccgcccattctccgccccatcgctgactaattttttttatttatgcagaggccgaggccgcctcggcctctgagctattccagaagtagtgaggaggcttttttggaggcctaggcttttgcaaa

SEQ ID NO: 115 - DNA, 999 bp, Cricetulus griseus
  misc_feature: CHO Actb promoter
gggcggaggccagtcatgcatgttcgggcctatggggccagcacccaacgccaaaactctccatcctcttcctcaatctcgctttctctctctctctctttttttttttttttttttttttttttttttttttgcaaaaggaggggagagggggtaaaaaaatgctgcactgtgcggctaggccggtgagtgagcggcgcggagccaatcagcgctcgccgttccgaaagttgccttttatggctcgagtggccgctgtggcgtcctataaaacccggcggcgcaacgcgcagccactgtcgagtccgcgtccacccgcgagcacaggcctttcgcagctctttcttcgccgctccacacccgccaccaggtaagcagggacaacaggcccagccggccacagccctcccgtgggcagtgaccgcgctgcagggtcgcgggggacactcggcgcggacaccggggaaggctggagggtggtgccgggccgcggagcggacactttcagatccaactttcagtccagggtgtagaccctttacagccgcattgccacggtgtagacaccggtggacccgctctggctcagagcacgcggcttgggggaacccattagggtcgcagtgtgggcgctatgagagccgatgcagctttcgggtgttgaaccgtatctgcccaccttggggggaggacacaaggtcgggagccaaacgccacgatcatgccttggtggcccatgggtctttgtctaaaccggtttgcccatttggcttgccgggcgggcgggcgcggcgggcccggctcggccgggtgggggctgggttgccactgcgcttgcgcgctctatggctgggtattggggcgcgtgcacgctggggagggagcccttcctcttccccctctcccaagttaaacttgcgcgtgcgtattgagacttggagcgcggccaccggggttgggcgagggcggggccgttgtccggaaggggcggggtcgcag

SEQ ID NO: 116 - DNA, 683 bp, Cricetulus griseus
  misc_feature: CHO Hspa5 promoter
acccgaggggacttaggaggagaaaaggccgcatactgcttcggggtaagggacagaccggggaaggacccaagtcccaccgcccagagggaactgacacgcagaccccgcagcagtccccgggggccgggtgacgggaggacctggacggttaccggcggaaacggtctcgggttgagaggtcacctgagggacaggcagctgctgaaccaataggaccggcgcacagggcggatgctgcctctcattggcggccgttgagagtaaccagtagccaatgagtcagcccggggggcgtagcggtgacgtaagttgcggaggaggccgcttcgaatcggcagcggccagcttggtggcatggaccaatcagcgtcctccaacgagaagcgccttcaccaatcggaggcctccacgacggggctggggggagggtatataagccaagtcggcggcggcgcgctccacactggccaagacaacagtgaccggaggacctgcctttgcggctccgagaggtaagcgccgcggcctgctcttgccagacctcctttgagcctgtctcgtggctcctcctgacccggggggcttctgtcgccctcagatcggaacgccgccgcgctccgggactacagcctgttgctggacttcgagactgcagacggaccgaccgctgagcactggcc